European Patent Application EP 4 748 856 A2, published May 27, 2026. Title: COMPOSITIONS AND METHODS FOR TREATING CANCER WITH SELF-DRIVING CHIMERIC ANTIGEN RECEPTORS. Applicant: Lentigen Technology, Inc. Application EP Divisional application of EP20716630.7, filed March 6, 2020. The sequence listing filed with the application follows.

SEQUENCE LISTING (189 sequences)

SEQ ID NO: 1-3 - skipped (3 entries)

SEQ ID NO: 4 - DNA, 10 bp, synthetic construct
  misc_feature 1..10: note = source = /note="Description of Artificial Sequence: Synthetic oligonucleotide"
  source 1..10: mol_type = other DNA
gggaatttcc

SEQ ID NO: 5 - DNA, 10 bp, synthetic construct
  misc_feature 1..10: note = source = /note="Description of Artificial Sequence: Synthetic oligonucleotide"
  source 1..10: mol_type = other DNA
gggactttcc

SEQ ID NO: 6 - skipped

SEQ ID NO: 7 - DNA, 1494 bp, synthetic construct
  misc_feature 1..1494: note = source = /note="Description of Artificial Sequence: Synthetic polynucleotide"
  source 1..1494: mol_type = other DNA
atgctgctgctggtgaccagcctgctgctgtgcgaactgccgcatccggcgtttctgctgattccggaagtgcaattggtgcagagcggtggaggacttgtgaaacctggtggatccctgagactttcctgtgccgcttcgggcttcaccttctcggactactacatgtcctggattcgccaggcccctggaaagggactggaatgggtgtcatacatcagctcctccggttccaccatctactatgccgattccgtgaagggcagattcaccatctcgcgcgacaacgccaagaacactctctatctgcaaatgaactcactgcgggctgaggacaccgcggtctactactgcgcccgggacctcagcggaaagtccagcggatggtcccattacttcgattactggggacagggaaccctggtcaccgtgtccagcggcggggggggctcgggtggcggcggctccggcggcggcgggagcaacttcatgctgactcagccccactccgtgtccgagagcccgggaaagaccgtgactatttcgtgcacacggtcctccgggagcattgcgaacaactacgtgcagtggtaccagcagcggcccgatagggccccaaccactgtgatctacgaagatgaccagcggccgtctggagtcccggaccgcttctcggggtccatcgactcatcatccaattccgcatcgctgacgatcagcggactgaagatcgaggacgaagccgattactactgccagtcctacgacggcaccaactgggtctttgggggtggaaccaagctgactgtgctcggagcggccgcaactaccacccctgcccctcggccgccgactccggccccaaccatcgcaagccaacccctctccttgcgccccgaagcttgccgcccggccgcgggtggagccgtgcatacccgggggctggactttgcctgcgatatctacatttgggccccgctggccggcacttgcggcgtgctcctgctgtcgctggtcatcaccctttactgcaagaggggccggaagaagctgctttacatcttcaagcagccgttcatgcggcccgtgcagacgactcaggaagaggacggatgctcgtgcagattccctgaggaggaagaggggggatgcgaactgcgcgtcaagttctcacggtccgccgacgcccccgcatatcaacagggccagaatcagctctacaacgagctgaacctgggaaggagagaggagtacgacgtgctggacaagcgacgcggacgcgacccggagatgggggggaaaccacggcggaaaaaccctcaggaaggactgtacaacgaactccagaaagacaagatggcggaagcctactcagaaatcgggatgaagggagagcggaggaggggaaagggtcacgacgggctgtaccagggactgagcaccgccactaaggatacctacgatgccttgcatatgcaagcactcccaccccgg

SEQ ID NO: 8 - protein, 498 aa, synthetic construct
  REGION 1..498: note = source = /note="Description of Artificial Sequence: Synthetic polypeptide"
MLLLVTSLLLCELPHPAFLLIPEVQLVQSGGGLVKPGGSLRLSCAASGFTFSDYYMSWIRQAPGKGLEWVSYISSSGSTIYYADSVKGRFTISRDNAKNTLYLQMNSLRAEDTAVYYCARDLSGKSSGWSHYFDYWGQGTLVTVSSGGGGSGGGGSGGGGSNFMLTQPHSVSESPGKTVTISCTRSSGSIANNYVQWYQQRPDRAPTTVIYEDDQRPSGVPDRFSGSIDSSSNSASLTISGLKIEDEADYYCQSYDGTNWVFGGGTKLTVLGAAATTTPAPRPPTPAPTIASQPLSLRPEACRPAAGGAVHTRGLDFACDIYIWAPLAGTCGVLLLSLVITLYCKRGRKKLLYIFKQPFMRPVQTTQEEDGCSCRFPEEEEGGCELRVKFSRSADAPAYQQGQNQLYNELNLGRREEYDVLDKRRGRDPEMGGKPRRKNPQEGLYNELQKDKMAEAYSEIGMKGERRRGKGHDGLYQGLSTATKDTYDALHMQALPPR

SEQ ID NO: 9 - DNA, 1473 bp, synthetic construct
  misc_feature 1..1473: note = source = /note="Description of Artificial Sequence: Synthetic polynucleotide"
  source 1..1473: mol_type = other DNA
atgctgctgctggtgaccagcctgctgctgtgcgaactgccgcatccggcgtttctgctgattccggaagtgcaacttgtcgaaagcggtggaggtcttgtccaacctggtcgctccctgaggctctcgtgtgccgcgagcggattcaccttctcatcgtacgctatgtcctgggtcagacaggctcctggaaagggcctggaatgggtggccgtgatctcctacgacggcagcaacaagtattacgccgactcagtgaagggccggttcaccatttcccgggacaacagcaagaacaccctgtacttgcaaatgaactccctgcgggccgaggataccgcggtgtactactgcgcccacctccgctttggatacggaatggatgtctggggacagggaactaccgtgaccgtgtcgtccgggggggggggaagcggcggcgggggatcgggtggcggcggatcccagactgtggtcacccaagagccttcactgaccgtgtccccgggtggcaccgtgacgctgacttgcgcgtcatctaccggggccgtgacctcggaccactacccctgctggttccagcagaaacccggacatccaccgagagccctggtgtactccactgacaccatccactcctggactccggcccggttctccggaagcctcctgggcgggaaggccgcactgacagtgtccggagtgcagcccgaggatgaagccgactactactgtctgctctactatgggggagcacgcgtgttcggtggcggcactcagctgaccgtgctgggagcggccgcaactaccacccctgcccctcggccgccgactccggccccaaccatcgcaagccaacccctctccttgcgccccgaagcttgccgcccggccgcgggtggagccgtgcatacccgggggctggactttgcctgcgatatctacatttgggccccgctggccggcacttgcggcgtgctcctgctgtcgctggtcatcaccctttactgcaagaggggccggaagaagctgctttacatcttcaagcagccgttcatgcggcccgtgcagacgactcaggaagaggacggatgctcgtgcagattccctgaggaggaagaggggggatgcgaactgcgcgtcaagttctcacggtccgccgacgcccccgcatatcaacagggccagaatcagctctacaacgagctgaacctgggaaggagagaggagtacgacgtgctggacaagcgacgcggacgcgacccggagatgggggggaaaccacggcggaaaaaccctcaggaaggactgtacaacgaactccagaaagacaagatggcggaagcctactcagaaatcgggatgaagggagagcggaggaggggaaagggtcacgacgggctgtaccagggactgagcaccgccactaaggatacctacgatgccttgcatatgcaagcactcccaccccgg

SEQ ID NO: 10 - protein, 491 aa, synthetic construct
  REGION 1..491: note = source = /note="Description of Artificial Sequence: Synthetic polypeptide"
MLLLVTSLLLCELPHPAFLLIPEVQLVESGGGLVQPGRSLRLSCAASGFTFSSYAMSWVRQAPGKGLEWVAVISYDGSNKYYADSVKGRFTISRDNSKNTLYLQMNSLRAEDTAVYYCAHLRFGYGMDVWGQGTTVTVSSGGGGSGGGGSGGGGSQTVVTQEPSLTVSPGGTVTLTCASSTGAVTSDHYPCWFQQKPGHPPRALVYSTDTIHSWTPARFSGSLLGGKAALTVSGVQPEDEADYYCLLYYGGARVFGGGTQLTVLGAAATTTPAPRPPTPAPTIASQPLSLRPEACRPAAGGAVHTRGLDFACDIYIWAPLAGTCGVLLLSLVITLYCKRGRKKLLYIFKQPFMRPVQTTQEEDGCSCRFPEEEEGGCELRVKFSRSADAPAYQQGQNQLYNELNLGRREEYDVLDKRRGRDPEMGGKPRRKNPQEGLYNELQKDKMAEAYSEIGMKGERRRGKGHDGLYQGLSTATKDTYDALHMQALPPR

SEQ ID NO: 11 - DNA, 1467 bp, synthetic construct
  misc_feature 1..1467: note = source = /note="Description of Artificial Sequence: Synthetic polynucleotide"
  source 1..1467: mol_type = other DNA
atgctgctgctggtgaccagcctgctgctgtgcgaactgccgcatccggcgtttctgctgattccgcaagtccaactcgtccagtccggtgccgaagtcaagaagcctggctcatccgtgaaagtgtcctgcaaagcatcgggcggaaccttctcctcctatgccatttcctgggtccgccaggcaccgggccagggtctggagtggatgggcgggattatccctatcttcggaactgccaaccacgcccaaaagttccagggacgcgtgaccattaccgccgatgaatcaacctcaaccgcctacatggaactgtccagcttgaggtccgaggacaccgccgtgtactactgcgcgttcatgatggtgccggagtactactttgactactggggccagggaacccttgtgaccgtgtcgtccggtggtggcggatccgggggggggggatctgggggcggcggaagcgatatccagatgacccagtcgccatcgagcctgtccgcttccgtgggcgacagagtgacgatcacttgccgggcttcacaaggcatcagaaatgacctgggctggtatcagcagaagcccggagaagcgcccaagcggctgatctacgcggccagcaccctgcaaaacggagtgccttcgcggttctccgggagcggctccggaactgacttcactctgactattaacagcctccagcccgaggatttcgccacatactactgtcagcagtacaacagctacccgtacaccttcggacagggaactaagctcgaaatcaaggcggccgcaactaccacccctgcccctcggccgccgactccggccccaaccatcgcaagccaacccctctccttgcgccccgaagcttgccgcccggccgcgggtggagccgtgcatacccgggggctggactttgcctgcgatatctacatttgggccccgctggccggcacttgcggcgtgctcctgctgtcgctggtcatcaccctttactgcaagaggggccggaagaagctgctttacatcttcaagcagccgttcatgcggcccgtgcagacgactcaggaagaggacggatgctcgtgcagattccctgaggaggaagaggggggatgcgaactgcgcgtcaagttctcacggtccgccgacgcccccgcatatcaacagggccagaatcagctctacaacgagctgaacctgggaaggagagaggagtacgacgtgctggacaagcgacgcggacgcgacccggagatgggggggaaaccacggcggaaaaaccctcaggaaggactgtacaacgaactccagaaagacaagatggcggaagcctactcagaaatcgggatgaagggagagcggaggaggggaaagggtcacgacgggctgtaccagggactgagcaccgccactaaggatacctacgatgccttgcatatgcaagcactcccaccccgg

SEQ ID NO: 12 - protein, 489 aa, synthetic construct
  REGION 1..489: note = source = /note="Description of Artificial Sequence: Synthetic polypeptide"
MLLLVTSLLLCELPHPAFLLIPQVQLVQSGAEVKKPGSSVKVSCKASGGTFSSYAISWVRQAPGQGLEWMGGIIPIFGTANHAQKFQGRVTITADESTSTAYMELSSLRSEDTAVYYCAFMMVPEYYFDYWGQGTLVTVSSGGGGSGGGGSGGGGSDIQMTQSPSSLSASVGDRVTITCRASQGIRNDLGWYQQKPGEAPKRLIYAASTLQNGVPSRFSGSGSGTDFTLTINSLQPEDFATYYCQQYNSYPYTFGQGTKLEIKAAATTTPAPRPPTPAPTIASQPLSLRPEACRPAAGGAVHTRGLDFACDIYIWAPLAGTCGVLLLSLVITLYCKRGRKKLLYIFKQPFMRPVQTTQEEDGCSCRFPEEEEGGCELRVKFSRSADAPAYQQGQNQLYNELNLGRREEYDVLDKRRGRDPEMGGKPRRKNPQEGLYNELQKDKMAEAYSEIGMKGERRRGKGHDGLYQGLSTATKDTYDALHMQALPPR

SEQ ID NO: 13 - DNA, 66 bp, synthetic construct
  misc_feature 1..66: note = source = /note="Description of Artificial Sequence: Synthetic oligonucleotide"
  source 1..66: mol_type = other DNA
atgctgctgctggtgaccagcctgctgctgtgcgaactgccgcatccggcgtttctgctgattccg

SEQ ID NO: 14 - protein, 22 aa, synthetic construct
  REGION 1..22: note = source = /note="Description of Artificial Sequence: Synthetic peptide"
MLLLVTSLLLCELPHPAFLLIP

SEQ ID NO: 15 - DNA, 1500 bp, synthetic construct
  misc_feature 1..1500: note = source = /note="Description of Artificial Sequence: Synthetic polynucleotide"
  source 1..1500: mol_type = other DNA
atgctgctgctggtgaccagcctgctgctgtgcgaactgccgcatccggcgtttctgctgattccgcaactccaactccaagaatctggaccaggcctcgtgaagccctcccaaactctgtccctgacctgtaccgtgtcgggtggaagcatttcgagcggtggatactactggtcctggatcaggcagcatcctggaaagggactggagtggattgggtacatctactactccggctcaacctactacaacccgtccttgaaatcgcgcgtgacgatctccgtggacacttcaaagaaccagttcagcctgaagctttcctccgtgaccgcggccgatacagcggtgtactactgcgctcgggatcagagcgtggccgaccctggtggcggctactactactacggaatggatgtctggggacagggaaccaccgtgactgtgtccagcgggggcggcggatccgggggggggggatcgggcggcggcggttcgcagtccgtgctgacccagccacctagcgtgtcagtggcaccgggacagaccgcctccatttcctgcgggggaaatgacttcggtagccgctccgtgtcatggtatcaccagaagccgggacaggccccggtgctggtcatctatgacgacaacgacagaccctcgggcatccccgaacggttttcgggaagcacctccggagacactgccaccctgaccatctcccgggtcgaggtcggcgatgaagccgattactactgccaagtctgggacgacgactccgaccactgggtgttcggcggcggaactaagctgactgtgctgggggcggccgcaactaccacccctgcccctcggccgccgactccggccccaaccatcgcaagccaacccctctccttgcgccccgaagcttgccgcccggccgcgggtggagccgtgcatacccgggggctggactttgcctgcgatatctacatttgggccccgctggccggcacttgcggcgtgctcctgctgtcgctggtcatcaccctttactgcaagaggggccggaagaagctgctttacatcttcaagcagccgttcatgcggcccgtgcagacgactcaggaagaggacggatgctcgtgcagattccctgaggaggaagaggggggatgcgaactgcgcgtcaagttctcacggtccgccgacgcccccgcatatcaacagggccagaatcagctctacaacgagctgaacctgggaaggagagaggagtacgacgtgctggacaagcgacgcggacgcgacccggagatgggggggaaaccacggcggaaaaaccctcaggaaggactgtacaacgaactccagaaagacaagatggcggaagcctactcagaaatcgggatgaagggagagcggaggaggggaaagggtcacgacgggctgtaccagggactgagcaccgccactaaggatacctacgatgccttgcatatgcaagcactcccaccccgg

SEQ ID NO: 16 - protein, 500 aa, synthetic construct
  REGION 1..500: note = source = /note="Description of Artificial Sequence: Synthetic polypeptide"
MLLLVTSLLLCELPHPAFLLIPQLQLQESGPGLVKPSQTLSLTCTVSGGSISSGGYYWSWIRQHPGKGLEWIGYIYYSGSTYYNPSLKSRVTISVDTSKNQFSLKLSSVTAADTAVYYCARDQSVADPGGGYYYYGMDVWGQGTTVTVSSGGGGSGGGGSGGGGSQSVLTQPPSVSVAPGQTASISCGGNDFGSRSVSWYHQKPGQAPVLVIYDDNDRPSGIPERFSGSTSGDTATLTISRVEVGDEADYYCQVWDDDSDHWVFGGGTKLTVLGAAATTTPAPRPPTPAPTIASQPLSLRPEACRPAAGGAVHTRGLDFACDIYIWAPLAGTCGVLLLSLVITLYCKRGRKKLLYIFKQPFMRPVQTTQEEDGCSCRFPEEEEGGCELRVKFSRSADAPAYQQGQNQLYNELNLGRREEYDVLDKRRGRDPEMGGKPRRKNPQEGLYNELQKDKMAEAYSEIGMKGERRRGKGHDGLYQGLSTATKDTYDALHMQALPPR

SEQ ID NO: 17 - DNA, 1467 bp, synthetic construct
  misc_feature 1..1467: note = source = /note="Description of Artificial Sequence: Synthetic polynucleotide"
  source 1..1467: mol_type = other DNA
atgctgctgctggtgaccagcctgctgctgtgcgaactgccgcatccggcgtttctgctgattccgcaagttcagctgcaagaatcaggacctgggcttgtcaaaccatctgaaaccctcagcttgacttgtaccgtatcaggagggtcaatttcaagctcatcctactattggggatggatcagacaaccacccgggaaagggctcgagtggatagggtccatatattacagcggatctacatactacaacccgtcattgaagtccagggtaacgattccggtggacactagcaagaatcagtttagcctcaagttgagcagtgtaactgctgcggacacggcggtatattattgtgctcgacacctcggtggagatgcttttgacatatggggtcaagggacaacagtcaccgttagctcaggtggagggggtagcggggggggcggatctgggggaggcggttcattgcccgtacttacacagccaccctctgtcagcgtcgcacctggacaaaccgctcgcatcacctgtggcggaaataatataggttccaagtctgttcattggtatcagcagaaaccgggacaggcccccgtccttgtggtgtatgatgattctgataggccatctggtatcccagaacggttttcaggtagcaattcagggaatactgccactctcactattagcggtactcaagctatggatgaggccgactatttttgccagagctacgactctagtaacccagtcgtgttcgggggagggacccagttgaccgtgctggcggccgcaactaccacccctgcccctcggccgccgactccggccccaaccatcgcaagccaacccctctccttgcgccccgaagcttgccgcccggccgcgggtggagccgtgcatacccgggggctggactttgcctgcgatatctacatttgggccccgctggccggcacttgcggcgtgctcctgctgtcgctggtcatcaccctttactgcaagaggggccggaagaagctgctttacatcttcaagcagccgttcatgcggcccgtgcagacgactcaggaagaggacggatgctcgtgcagattccctgaggaggaagaggggggatgcgaactgcgcgtcaagttctcacggtccgccgacgcccccgcatatcaacagggccagaatcagctctacaacgagctgaacctgggaaggagagaggagtacgacgtgctggacaagcgacgcggacgcgacccggagatgggggggaaaccacggcggaaaaaccctcaggaaggactgtacaacgaactccagaaagacaagatggcggaagcctactcagaaatcgggatgaagggagagcggaggaggggaaagggtcacgacgggctgtaccagggactgagcaccgccactaaggatacctacgatgccttgcatatgcaagcactcccaccccgg

SEQ ID NO: 18 - protein, 489 aa, synthetic construct
  REGION 1..489: note = source = /note="Description of Artificial Sequence: Synthetic polypeptide"
MLLLVTSLLLCELPHPAFLLIPQVQLQESGPGLVKPSETLSLTCTVSGGSISSSSYYWGWIRQPPGKGLEWIGSIYYSGSTYYNPSLKSRVTIPVDTSKNQFSLKLSSVTAADTAVYYCARHLGGDAFDIWGQGTTVTVSSGGGGSGGGGSGGGGSLPVLTQPPSVSVAPGQTARITCGGNNIGSKSVHWYQQKPGQAPVLVVYDDSDRPSGIPERFSGSNSGNTATLTISGTQAMDEADYFCQSYDSSNPVVFGGGTQLTVLAAATTTPAPRPPTPAPTIASQPLSLRPEACRPAAGGAVHTRGLDFACDIYIWAPLAGTCGVLLLSLVITLYCKRGRKKLLYIFKQPFMRPVQTTQEEDGCSCRFPEEEEGGCELRVKFSRSADAPAYQQGQNQLYNELNLGRREEYDVLDKRRGRDPEMGGKPRRKNPQEGLYNELQKDKMAEAYSEIGMKGERRRGKGHDGLYQGLSTATKDTYDALHMQALPPR

SEQ ID NO: 19 - DNA, 1476 bp, synthetic construct
  misc_feature 1..1476: note = source = /note="Description of Artificial Sequence: Synthetic polynucleotide"
  source 1..1476: mol_type = other DNA
atgctgctgctggtgaccagcctgctgctgtgcgaactgccgcatccggcgtttctgctgattccgcaggcggcccaggtacagctgcagcagtcaggggctgaggtgaagaagcctgggtcctcggtgaaggtctcctgcaaggcttctggaggcaccttcagcagctatgctatcagctgggtgcgacaggcccctggacaagggcttgagtggatgggatggatcaaccctaacagtggtggcacaaactatgcacagaggtttcagggcagggtcaccatgaccagggacacgtccatcagcacagcctacatggagctgagcaggctgagatctgacgacacggccgtgtattactgtgcgagttataatgatgcttttgatatctggggccaaggcaccctggtcaccgtctcctcaggaggtggcgggtctggtggtggcggtagcggtggtggcggatccaattttatgctgactcagccccactctgtgtcggagtctccggggaagacggtaaccatctcctgcacccgcagcagtggcagcattgccagcaactatgtgcagtggtaccagcagcgcccgggcagtgcccccaccattgtgatctatgaggatgatcaaagaccctctggggtccctgatcggttctctggctccatcgacacctcctccaactctgcctccctcaccatctctggactgcagagtgaggacgaggctgactactactgtcagtcttatgagcccggcaatggggtattcggcggagggaccaaggtcaccgtcctagcggccgcaactaccacccctgcccctcggccgccgactccggccccaaccatcgcaagccaacccctctccttgcgccccgaagcttgccgcccggccgcgggtggagccgtgcatacccgggggctggactttgcctgcgatatctacatttgggccccgctggccggcacttgcggcgtgctcctgctgtcgctggtcatcaccctttactgcaagaggggccggaagaagctgctttacatcttcaagcagccgttcatgcggcccgtgcagacgactcaggaagaggacggatgctcgtgcagattccctgaggaggaagaggggggatgcgaactgcgcgtcaagttctcacggtccgccgacgcccccgcatatcaacagggccagaatcagctctacaacgagctgaacctgggaaggagagaggagtacgacgtgctggacaagcgacgcggacgcgacccggagatgggggggaaaccacggcggaaaaaccctcaggaaggactgtacaacgaactccagaaagacaagatggcggaagcctactcagaaatcgggatgaagggagagcggaggaggggaaagggtcacgacgggctgtaccagggactgagcaccgccactaaggatacctacgatgccttgcatatgcaagcactcccaccccgg

SEQ ID NO: 20 - protein, 492 aa, synthetic construct
  REGION 1..492: note = source = /note="Description of Artificial Sequence: Synthetic polypeptide"
MLLLVTSLLLCELPHPAFLLIPQAAQVQLQQSGAEVKKPGSSVKVSCKASGGTFSSYAISWVRQAPGQGLEWMGWINPNSGGTNYAQRFQGRVTMTRDTSISTAYMELSRLRSDDTAVYYCASYNDAFDIWGQGTLVTVSSGGGGSGGGGSGGGGSNFMLTQPHSVSESPGKTVTISCTRSSGSIASNYVQWYQQRPGSAPTIVIYEDDQRPSGVPDRFSGSIDTSSNSASLTISGLQSEDEADYYCQSYEPGNGVFGGGTKVTVLAAATTTPAPRPPTPAPTIASQPLSLRPEACRPAAGGAVHTRGLDFACDIYIWAPLAGTCGVLLLSLVITLYCKRGRKKLLYIFKQPFMRPVQTTQEEDGCSCRFPEEEEGGCELRVKFSRSADAPAYQQGQNQLYNELNLGRREEYDVLDKRRGRDPEMGGKPRRKNPQEGLYNELQKDKMAEAYSEIGMKGERRRGKGHDGLYQGLSTATKDTYDALHMQALPPR

SEQ ID NO: 21 - DNA, 1488 bp, synthetic construct
  misc_feature 1..1488: note = source = /note="Description of Artificial Sequence: Synthetic polynucleotide"
  source 1..1488: mol_type = other DNA
atgctgctgctggtgaccagcctgctgctgtgcgaactgccgcatccggcgtttctgctgattccgcaagaacagcttgtagagtccggcggtagattggtgacaccgggggggagccttaccctgtcttgtaaggcatctgggttcgatttcagtgcgtattatatgagctgggttcggcaggcgcccgggaaggggctggaatggatagccactatatacccgtcatccggcaagacttactacgcgacttgggtaaacgggaggtttacgataagctcagataacgcccaaaacacggttgatctccaaatgaatagcttgaccgccgctgatagggcgacctatttctgtgcgcgggactcttacgctgatgacggggccctcttcaatatatggggaccgggaacgctcgtaaccatatcatctggaggaggtgggagcggaggcggagggtcaggtgggggcgggagcgaactcgtacttacacaatctccaagcgtaagcgcagcgttggggagtccagcaaagatcacctgcactttgtcaagcgcccacaaaacggatacgatagattggtatcagcaactccaaggtgaagcgccacgatatctcatgcaggtacagagcgacgggagttatactaagaggcccggggtcccagacagattcagtggcagcagttcaggtgccgacagatacctgataataccctcagttcaagccgatgatgaagccgattactactgtggggctgactacataggtgggtatgttttcgggggcggcactcaattgacagttacaggggcggccgcaactaccacccctgcccctcggccgccgactccggccccaaccatcgcaagccaacccctctccttgcgccccgaagcttgccgcccggccgcgggtggagccgtgcatacccgggggctggactttgcctgcgatatctacatttgggccccgctggccggcacttgcggcgtgctcctgctgtcgctggtcatcaccctttactgcaagaggggccggaagaagctgctttacatcttcaagcagccgttcatgcggcccgtgcagacgactcaggaagaggacggatgctcgtgcagattccctgaggaggaagaggggggatgcgaactgcgcgtcaagttctcacggtccgccgacgcccccgcatatcaacagggccagaatcagctctacaacgagctgaacctgggaaggagagaggagtacgacgtgctggacaagcgacgcggacgcgacccggagatgggggggaaaccacggcggaaaaaccctcaggaaggactgtacaacgaactccagaaagacaagatggcggaagcctactcagaaatcgggatgaagggagagcggaggaggggaaagggtcacgacgggctgtaccagggactgagcaccgccactaaggatacctacgatgccttgcatatgcaagcactcccaccccgg

SEQ ID NO: 22 - protein, 496 aa, synthetic construct
  REGION 1..496: note = source = /note="Description of Artificial Sequence: Synthetic polypeptide"
MLLLVTSLLLCELPHPAFLLIPQEQLVESGGRLVTPGGSLTLSCKASGFDFSAYYMSWVRQAPGKGLEWIATIYPSSGKTYYATWVNGRFTISSDNAQNTVDLQMNSLTAADRATYFCARDSYADDGALFNIWGPGTLVTISSGGGGSGGGGSGGGGSELVLTQSPSVSAALGSPAKITCTLSSAHKTDTIDWYQQLQGEAPRYLMQVQSDGSYTKRPGVPDRFSGSSSGADRYLIIPSVQADDEADYYCGADYIGGYVFGGGTQLTVTGAAATTTPAPRPPTPAPTIASQPLSLRPEACRPAAGGAVHTRGLDFACDIYIWAPLAGTCGVLLLSLVITLYCKRGRKKLLYIFKQPFMRPVQTTQEEDGCSCRFPEEEEGGCELRVKFSRSADAPAYQQGQNQLYNELNLGRREEYDVLDKRRGRDPEMGGKPRRKNPQEGLYNELQKDKMAEAYSEIGMKGERRRGKGHDGLYQGLSTATKDTYDALHMQALPPR

SEQ ID NO: 23 - DNA, 1464 bp, synthetic construct
  misc_feature 1..1464: note = source = /note="Description of Artificial Sequence: Synthetic polynucleotide"
  source 1..1464: mol_type = other DNA
atgctgctgctggtgaccagcctgctgctgtgcgaactgccgcatccggcgtttctgctgattccggaagtgcaactcgtcgaaactggagccgaagtgaaaaagcctggagcgtccgtcaaagtgtcgtgcaaggcctccggctacaccttcacgacctactacgtgcactgggtcagacaggctccgggtcaagggctggagtggatgggcatcattaacccctccggtggaagcacctcctatgcgcaaaagttccagggtcgcgtcaccatgactcgcgatacctccacttccactgtgtacatggaactgagctccctgaggtccgaggacaccgccgtgtactactgcgcacgggatggaggcttgggcggctacgaggcttggggacagggcaccctcgtgactgtgtcaagcggagggggtggatccggagggggaggatcaggcggtggtggaagcgatatccagcttacccagtcgccttccgcgctgtctgcatcggccggcgacagagtgacaattacctgtcaagccagccaggacatctccaactatctgaactggtaccagcagaagcccggaaaggctccgaagctgctgatctacgacgccagcaacctggaacggggcgtgccatcacggttctcgggatcagggtcgggcactgagttcaccttcaccatctcctccctccaacccgaggacattgccacctactactgccagcagtacgacaacctcccgatcacctttggacaggggactcgcctggaaatcaaggcggccgcaactaccacccctgcccctcggccgccgactccggccccaaccatcgcaagccaacccctctccttgcgccccgaagcttgccgcccggccgcgggtggagccgtgcatacccgggggctggactttgcctgcgatatctacatttgggccccgctggccggcacttgcggcgtgctcctgctgtcgctggtcatcaccctttactgcaagaggggccggaagaagctgctttacatcttcaagcagccgttcatgcggcccgtgcagacgactcaggaagaggacggatgctcgtgcagattccctgaggaggaagaggggggatgcgaactgcgcgtcaagttctcacggtccgccgacgcccccgcatatcaacagggccagaatcagctctacaacgagctgaacctgggaaggagagaggagtacgacgtgctggacaagcgacgcggacgcgacccggagatgggggggaaaccacggcggaaaaaccctcaggaaggactgtacaacgaactccagaaagacaagatggcggaagcctactcagaaatcgggatgaagggagagcggaggaggggaaagggtcacgacgggctgtaccagggactgagcaccgccactaaggatacctacgatgccttgcatatgcaagcactcccaccccgg

SEQ ID NO: 24 - protein, 488 aa, synthetic construct
  REGION 1..488: note = source = /note="Description of Artificial Sequence: Synthetic polypeptide"
MLLLVTSLLLCELPHPAFLLIPEVQLVETGAEVKKPGASVKVSCKASGYTFTTYYVHWVRQAPGQGLEWMGIINPSGGSTSYAQKFQGRVTMTRDTSTSTVYMELSSLRSEDTAVYYCARDGGLGGYEAWGQGTLVTVSSGGGGSGGGGSGGGGSDIQLTQSPSALSASAGDRVTITCQASQDISNYLNWYQQKPGKAPKLLIYDASNLERGVPSRFSGSGSGTEFTFTISSLQPEDIATYYCQQYDNLPITFGQGTRLEIKAAATTTPAPRPPTPAPTIASQPLSLRPEACRPAAGGAVHTRGLDFACDIYIWAPLAGTCGVLLLSLVITLYCKRGRKKLLYIFKQPFMRPVQTTQEEDGCSCRFPEEEEGGCELRVKFSRSADAPAYQQGQNQLYNELNLGRREEYDVLDKRRGRDPEMGGKPRRKNPQEGLYNELQKDKMAEAYSEIGMKGERRRGKGHDGLYQGLSTATKDTYDALHMQALPPR

SEQ ID NO: 25 - DNA, 1503 bp, synthetic construct
  misc_feature 1..1503: note = source = /note="Description of Artificial Sequence: Synthetic polynucleotide"
  source 1..1503: mol_type = other DNA
atgctgctgctggtgaccagcctgctgctgtgcgaactgccgcatccggcgtttctgctgattccggaagtgcaattggtccagagcggaggaggacttgtgaagccaggcggatccctgagattgtcatgcgccgcatcggggttcaccttttcctcctactccatgaactgggtcagacaggcgcccggaaagggacttgaatgggtgtcgtccatttcctcctcctcgtcctacatctactacgccgactccgtgaagggccgcttcaccatctcccgggacaacgccaagaacagcctgtatctccaaatgaactccctgcgggccgaagatactgctgtgtattactgcgctcgggacttcccgtacgactcatcgggctattactcggacgcgttcgatatctggggccagggaactatggtcaccgtcagctctggtggcggtggttccggagggggtggatccggtggcggaggatcagagattgtgctgacccagtccccgctgtcactgcccgtgactccgggagagcctgcctcgatctcgtgtcggtccagccagtccctgctgcactcgaatgggtacaactacctcgattggtacctccaaaagcctgggcagtcaccccaactgctgatctacctcgggagcaacagagccagcggagtgcctgaccgctttagcggttccggatccggcaccgacttcaccctgaaaatcagccgggtggaagccgaggatgtcggcgtgtactactgcatgcaggcactgcagactctggggtacaccttcggccagggcacgaagctcgagatcaaggcggccgcaactaccacccctgcccctcggccgccgactccggccccaaccatcgcaagccaacccctctccttgcgccccgaagcttgccgcccggccgcgggtggagccgtgcatacccgggggctggactttgcctgcgatatctacatttgggccccgctggccggcacttgcggcgtgctcctgctgtcgctggtcatcaccctttactgcaagaggggccggaagaagctgctttacatcttcaagcagccgttcatgcggcccgtgcagacgactcaggaagaggacggatgctcgtgcagattccctgaggaggaagaggggggatgcgaactgcgcgtcaagttctcacggtccgccgacgcccccgcatatcaacagggccagaatcagctctacaacgagctgaacctgggaaggagagaggagtacgacgtgctggacaagcgacgcggacgcgacccggagatgggggggaaaccacggcggaaaaaccctcaggaaggactgtacaacgaactccagaaagacaagatggcggaagcctactcagaaatcgggatgaagggagagcggaggaggggaaagggtcacgacgggctgtaccagggactgagcaccgccactaaggatacctacgatgccttgcatatgcaagcactcccaccccgg

SEQ ID NO: 26 - protein, 501 aa, synthetic construct
  REGION 1..501: note = source = /note="Description of Artificial Sequence: Synthetic polypeptide"
MLLLVTSLLLCELPHPAFLLIPEVQLVQSGGGLVKPGGSLRLSCAASGFTFSSYSMNWVRQAPGKGLEWVSSISSSSSYIYYADSVKGRFTISRDNAKNSLYLQMNSLRAEDTAVYYCARDFPYDSSGYYSDAFDIWGQGTMVTVSSGGGGSGGGGSGGGGSEIVLTQSPLSLPVTPGEPASISCRSSQSLLHSNGYNYLDWYLQKPGQSPQLLIYLGSNRASGVPDRFSGSGSGTDFTLKISRVEAEDVGVYYCMQALQTLGYTFGQGTKLEIKAAATTTPAPRPPTPAPTIASQPLSLRPEACRPAAGGAVHTRGLDFACDIYIWAPLAGTCGVLLLSLVITLYCKRGRKKLLYIFKQPFMRPVQTTQEEDGCSCRFPEEEEGGCELRVKFSRSADAPAYQQGQNQLYNELNLGRREEYDVLDKRRGRDPEMGGKPRRKNPQEGLYNELQKDKMAEAYSEIGMKGERRRGKGHDGLYQGLSTATKDTYDALHMQALPPR

SEQ ID NO: 27 - DNA, 72 bp, synthetic construct
  misc_feature 1..72: note = source = /note="Description of Artificial Sequence: Synthetic oligonucleotide"
  source 1..72: mol_type = other DNA
atctacatctgggcgcccttggccgggacttgtggggtccttctcctgtcactggttatcaccctttactgc

SEQ ID NO: 28 - protein, 22 aa, synthetic construct
  REGION 1..22: note = source = /note="Description of Artificial Sequence: Synthetic peptide"
IWAPLAGTCGVLLLSLVITLYC

SEQ ID NO: 29 - DNA, 135 bp, synthetic construct
  misc_feature 1..135: note = source = /note="Description of Artificial Sequence: Synthetic polynucleotide"
  source 1..135: mol_type = other DNA
accacgacgccagcgccgcgaccaccaacaccggcgcccaccatcgcgtcgcagcccctgtccctgcgcccagaggcgtgccggccagcggcggggggcgcagtgcacacgagggggctggacttcgcctgtgat

SEQ ID NO: 30 - protein, 47 aa, synthetic construct
  REGION 1..47: note = source = /note="Description of Artificial Sequence: Synthetic polypeptide"
TTTPAPRPPTPAPTIASQPLSLRPEACRPAAGGAVHTRGLDFACDIY

SEQ ID NO: 31 - protein, 42 aa, Homo sapiens
KRGRKKLLYIFKQPFMRPVQTTQEEDGCSCRFPEEEEGGCEL

SEQ ID NO: 32 - protein, 106 aa, Homo sapiens
GQPKAAPSVTLFPPSSEELQANKATLVCLISDFYPGAVTVAWKADSSPVKAGVETTTPSKQSNNKYAASSYLSLTPEQWKSHRSYSCQVTHEGSTVEKTVAPTECS

SEQ ID NO: 33 - DNA, 126 bp, synthetic construct
  misc_feature 1..126: note = source = /note="Description of Artificial Sequence: Synthetic polynucleotide"
  source 1..126: mol_type = other DNA
aaacggggcagaaagaaactcctgtatatattcaaacaaccatttatgagaccagtacaaactactcaagaggaagatggctgtagctgccgatttccagaagaagaagaaggaggatgtgaactg

SEQ ID NO: 34 - protein, 42 aa, synthetic construct; identical to SEQ ID NO: 31
  REGION 1..42: note = source = /note="Description of Artificial Sequence: Synthetic polypeptide"

SEQ ID NO: 35 - DNA, 336 bp, synthetic construct
  misc_feature 1..336: note = source = /note="Description of Artificial Sequence: Synthetic polynucleotide"
  source 1..336: mol_type = other DNA
agagtgaagttcagcaggagcgcagacgcccccgcgtacaagcagggccagaaccagctctataacgagctcaatctaggacgaagagaggagtacgatgttttggacaagagacgtggccgggaccctgagatggggggaaagccgagaaggaagaaccctcaggaaggcctgtacaatgaactgcagaaagataagatggcggaggcctacagtgagattgggatgaaaggcgagcgccggaggggcaaggggcacgatggcctttaccagggtctcagtacagccaccaaggacacctacgacgcccttcacatgcaggccctgccccctcgc

SEQ ID NO: 36 - protein, 112 aa, synthetic construct
  REGION 1..112: note = source = /note="Description of Artificial Sequence: Synthetic polypeptide"
RVKFSRSADAPAYKQGQNQLYNELNLGRREEYDVLDKRRGRDPEMGGKPRRKNPQEGLYNELQKDKMAEAYSEIGMKGERRRGKGHDGLYQGLSTATKDTYDALHMQALPPR

SEQ ID NO: 37 - DNA, 726 bp, synthetic construct
  misc_feature 1..726: note = source = /note="Description of Artificial Sequence: Synthetic polynucleotide"
  source 1..726: mol_type = other DNA
gacatccagatgacacagactacatcctccctgtctgcctctctgggagacagagtcaccatcagttgcagggcaagtcaggacattagtaaatatttaaattggtatcagcagaaaccagatggaactgttaaactcctgatctaccatacatcaagattacactcaggagtcccatcaaggttcagtggcagtgggtctggaacagattattctctcaccattagcaacctggagcaagaagatattgccacttacttttgccaacagggtaatacgcttccgtacacgttcggaggggggaccaagctggagatcacaggtggcggtggctcgggcggtggtgggtcgggtggcggcggatctgaggtgaaactgcaggagtcaggacctggcctggtggcgccctcacagagcctgtccgtcacatgcactgtctcaggggtctcattacccgactatggtgtaagctggattcgccagcctccacgaaagggtctggagtggctgggagtaatatggggtagtgaaaccacatactataattcagctctcaaatccagactgaccatcatcaaggacaactccaagagccaagttttcttaaaaatgaacagtctgcaaactgatgacacagccatttactactgtgccaaacattattactacggtggtagctatgctatggactactggggccaaggaacctcagtcaccgtctcctca

SEQ ID NO: 38 - protein, 242 aa, synthetic construct
  REGION 1..242: note = source = /note="Description of Artificial Sequence: Synthetic polypeptide"
DIQMTQTTSSLSASLGDRVTISCRASQDISKYLNWYQQKPDGTVKLLIYHTSRLHSGVPSRFSGSGSGTDYSLTISNLEQEDIATYFCQQGNTLPYTFGGGTKLEITGGGGSGGGGSGGGGSEVKLQESGPGLVAPSQSLSVTCTVSGVSLPDYGVSWIRQPPRKGLEWLGVIWGSETTYYNSALKSRLTIIKDNSKSQVFLKMNSLQTDDTAIYYCAKHYYYGGSYAMDYWGQGTSVTVSS

SEQ ID NO: 39 - DNA, 66 bp, synthetic construct; identical to SEQ ID NO: 13
  misc_feature 1..66: note = source = /note="Description of Artificial Sequence: Synthetic oligonucleotide"
  source 1..66: mol_type = other DNA

SEQ ID NO: 40 - protein, 22 aa, synthetic construct
  REGION 1..22: note = source = /note="Description of Artificial Sequence: Synthetic peptide"
MLLLVTSLLLCELPHPAFLLIP

SEQ ID NO: 41 - DNA, 85 bp, synthetic construct
  misc_feature 1..85: note = source = /note="Description of Artificial Sequence: Synthetic oligonucleotide"
  source 1..85: mol_type = other DNA
ggctctgaaagtgctgttggaacaagaaaagaccttcttcaccttgctcgtgttgctggggtacctgtcctgcaaagtcacctgt

SEQ ID NO: 42 - protein, 29 aa, synthetic construct
  REGION 1..29: note = source = /note="Description of Artificial Sequence: Synthetic peptide"
MALKVLLEQEKTFFTLLVLLGYLSCKVTC

SEQ ID NO: 43 - DNA, 63 bp, synthetic construct
  misc_feature 1..63: note = source = /note="Description of Artificial Sequence: Synthetic oligonucleotide"
  source 1..63: mol_type = other DNA
atggcgctgccggtgaccgcgctgctgctgccgctggcgctgctgctgcatgcggcgcgcccg

SEQ ID NO: 44 - protein, 21 aa, synthetic construct
  REGION 1..21: note = source = /note="Description of Artificial Sequence: Synthetic peptide"
MALPVTALLLPLALLLHAARP

SEQ ID NO: 45 - DNA, 123 bp, synthetic construct
  misc_feature 1..123: note = source = /note="Description of Artificial Sequence: Synthetic polynucleotide"
  source 1..123: mol_type = other DNA
cggtcgaagaggtccagactcttgcactccgactacatgaacatgactcctagaaggcccggacccactagaaagcactaccagccgtacgcccctcctcgggatttcgccgcataccggtcc

SEQ ID NO: 46 - protein, 41 aa, synthetic construct
  REGION 1..41: note = source = /note="Description of Artificial Sequence: Synthetic polypeptide"
RSKRSRLLHSDYMNMTPRRPGPTRKHYQPYAPPRDFAAYRS

SEQ ID NO: 47 - DNA, 336 bp, synthetic construct
  misc_feature 1..336: note = source = /note="Description of Artificial Sequence: Synthetic polynucleotide"
  source 1..336: mol_type = other DNA
agagtgaagttcagccgctcagccgatgcaccggcctaccagcagggacagaaccagctctacaacgagctcaacctgggtcggcgggaagaatatgacgtgctggacaaacggcgcggcagagatccggagatggggggaaagccgaggaggaagaaccctcaagagggcctgtacaacgaactgcagaaggacaagatggcggaagcctactccgagatcggcatgaagggagaacgccggagagggaagggtcatgacggactgtaccagggcctgtcaactgccactaaggacacttacgatgcgctccatatgcaagctttgcccccgcgg

SEQ ID NO: 48 - protein, 112 aa, synthetic construct
  REGION 1..112: note = source = /note="Description of Artificial Sequence: Synthetic polypeptide"
RVKFSRSADAPAYQQGQNQLYNELNLGRREEYDVLDKRRGRDPEMGGKPRRKNPQEGLYNELQKDKMAEAYSEIGMKGERRRGKGHDGLYQGLSTATKDTYDALHMQALPPR

SEQ ID NO: 49 - DNA, 201 bp, synthetic construct
  misc_feature 1..201: note = source = /note="Description of Artificial Sequence: Synthetic polynucleotide"
  source 1..201: mol_type = other DNA
gcggccgcggtcggattccaagacatggaatgcgtgccctgcggcgacccgccacctccttacgagccgcactgcgcatcgaaggtcaacctcgtgaagatcgcgagcaccgcgtcctcaccccgggatactgctctggccgccgtgatttgttccgccttggccaccgtgcttctggccctgctgatcctctgtgtgatc

SEQ ID NO: 50 - protein, 67 aa, synthetic construct
  REGION 1..67: note = source = /note="Description of Artificial Sequence: Synthetic polypeptide"
AAAVGFQDMECVPCGDPPPPYEPHCASKVNLVKIASTASSPRDTALAAVICSALATVLLALLILCVI

SEQ ID NO: 51 - DNA, 63 bp, synthetic construct
  misc_feature 1..63: note = source = /note="Description of Artificial Sequence: Synthetic oligonucleotide"
  source 1..63: mol_type = other DNA
gccgccgtgatttgttccgccttggccaccgtgcttctggccctgctgatcctctgtgtgatc

SEQ ID NO: 52 - protein, 21 aa, synthetic construct
  REGION 1..21: note = source = /note="Description of Artificial Sequence: Synthetic peptide"
AAVICSALATVLLALLILCVI

SEQ ID NO: 53 - DNA, 138 bp, synthetic construct
  misc_feature 1..138: note = source = /note="Description of Artificial Sequence: Synthetic polynucleotide"
  source 1..138: mol_type = other DNA
gcggccgcggtcggattccaagacatggaatgcgtgccctgcggcgacccgccacctccttacgagccgcactgcgcatcgaaggtcaacctcgtgaagatcgcgagcaccgcgtcctcaccccgggatactgctctg

SEQ ID NO: 54 - protein, 46 aa, synthetic construct
  REGION 1..46: note = source = /note="Description of Artificial Sequence: Synthetic polypeptide"
AAAVGFQDMECVPCGDPPPPYEPHCASKVNLVKIASTASSPRDTAL

SEQ ID NO: 55 - DNA, 80 bp, synthetic construct
  misc_feature 1..80: note = source = /note="Description of Artificial Sequence: Synthetic oligonucleotide"
  source 1..80: mol_type = other DNA
tacgagcctcactgcgccagcaaagtcaacttggtgaagatcgcgagcactgcctcgtcccctcgggacactgctctggc

SEQ ID NO: 56 - protein, 26 aa, synthetic construct
  REGION 1..26: note = source = /note="Description of Artificial Sequence: Synthetic peptide"
YEPHCASKVNLVKIASTASSPRDTAL

SEQ ID NO: 57 - DNA, 222 bp, synthetic construct
  misc_feature 1..222: note = source = /note="Description of Artificial Sequence: Synthetic polynucleotide"
  source 1..222: mol_type = other DNA
gcggccgcgcccgcccctcggcccccgactcctgccccgacgatcgcttcccaacctctctcgctgcgcccggaagcatgccggcccgccgccggtggcgctgtccacactcgcggactggactttgataccgcactggcggccgtgatctgtagcgccctggccaccgtgctgctggcgctgctcatcctttgcgtgatctactgcaagcggcagcctagg

SEQ ID NO: 58 - protein, 74 aa, synthetic construct
  REGION 1..74: note = source = /note="Description of Artificial Sequence: Synthetic polypeptide"
AAAPAPRPPTPAPTIASQPLSLRPEACRPAAGGAVHTRGLDFDTALAAVICSALATVLLALLILCVIYCKRQPR

SEQ ID NO: 59 - DNA, 123 bp, synthetic construct; identical to SEQ ID NO: 45
  misc_feature 1..123: note = source = /note="Description of Artificial Sequence: Synthetic polynucleotide"
  source 1..123: mol_type = other DNA

SEQ ID NO: 60 - protein, 41 aa, synthetic construct; identical to SEQ ID NO: 46
  REGION 1..41: note = source = /note="Description of Artificial Sequence: Synthetic polypeptide"

SEQ ID NO: 61 - DNA, 336 bp, synthetic construct
  misc_feature 1..336: note = source = /note="Description of Artificial Sequence: Synthetic polynucleotide"
  source 1..336: mol_type = other DNA
cgcgtgaaatttagccgcagcgcggatgcgccggcgtatcagcagggccagaaccagctgtataacgaactgaacctgggccgccgcgaagaatatgatgtgctggataaacgccgcggccgcgatccggaaatgggcggcaaaccgcgccgcaaaaacccgcaggaaggcctgtataacgaactgcagaaagataaaatggcggaagcgtatagcgaaattggcatgaaaggcgaacgccgccgcggcaaaggccatgatggcctgtatcagggcctgagcaccgcgaccaaagatacctatgatgcgctgcatatgcaggcgctgccgccgcgc

SEQ ID NO: 62 - protein, 112 aa, synthetic construct; identical to SEQ ID NO: 48
  REGION 1..112: note = source = /note="Description of Artificial Sequence: Synthetic polypeptide"

SEQ ID NO: 63 - DNA, 93 bp, synthetic construct
  misc_feature 1..93: note = source = /note="Description of Artificial Sequence: Synthetic oligonucleotide"
  source 1..93: mol_type = other DNA
cgcgcgaaacgcagcggcagcggcgcgaccaactttagcctgctgaaacaggcgggcgatgtggaagaaaacccgggcccgcgagcaaagagg

SEQ ID NO: 64 - protein, 31 aa, synthetic construct
  REGION 1..31: note = source = /note="Description of Artificial Sequence: Synthetic polypeptide"
RAKRSGSGATNFSLLKQAGDVEENPGPRAKR

SEQ ID NO: 65 - DNA, 78 bp, synthetic construct
  misc_feature 1..78: note = source = /note="Description of Artificial Sequence: Synthetic oligonucleotide"
  source 1..78: mol_type = other DNA
agagctaaacgctctgggtctggtgaaggacgaggtagccttcttacgtgcggagacgtggaggaaaacccaggaccc

SEQ ID NO: 66 - protein, 26 aa, synthetic construct
  REGION 1..26: note = source = /note="Description of Artificial Sequence: Synthetic peptide"
RAKRSGSGEGRGSLLTCGDVEENPGP

SEQ ID NO: 67 - DNA, 1005 bp, synthetic construct
  misc_feature 1..1005: note = source = /note="Description of Artificial Sequence: Synthetic polynucleotide"
  source 1..1005: mol_type = other DNA
aggaaggtttgcaatggaatcggtataggggagtttaaggattcacttagcataaacgctactaatattaaacacttcaaaaactgtacgagtataagtggagatcttcacattttgccggttgcattccgaggcgattcattcacccacacgccaccgcttgacccacaagaattggatattcttaaaaccgttaaagaaataacggggtttttgctcattcaagcgtggccagaaaatcgcactgacctccatgctttcgagaacctggagattataagaggacgaactaagcagcatggtcaattctcccttgctgtggtcagcctgaacatcaccagtcttggtttgcggtccctcaaggaaatttcagatggagatgtcatcataagcggcaacaagaatttgtgctatgcaaataccataaactggaaaaaactgtttggcacttccggccagaaaaccaagattatttcaaatcggggtgagaacagctgcaaagccaccggccaggtttgtcatgccttgtgctctccggaaggctgttgggggccagaacccagggactgcgtcagttgcagaaacgtctcaagaggccgcgaatgcgttgacaagtgtaacctccttgagggtgagccacgagagtttgttgagaacagcgagtgtatacaatgtcaccctgaatgtttgccccaggctatgaatataacctgcacaggccgcgggcctgataactgcatccagtgtgctcattacatagatggacctcactgtgtgaaaacctgcccggccggagttatgggagaaaacaacactctggtgtggaaatacgctgatgcaggccacgtgtgccacctttgtcacccgaattgtacatatgggtgtaccggtcctggacttgaaggttgccctaccaatggccctaaaatacccagtatcgcaactggcatggtaggcgctcttctcttgctcttggtagttgctctcggcataggtctttttatg

SEQ ID NO: 68 - protein, 335 aa, synthetic construct
  REGION 1..335: note = source = /note="Description of Artificial Sequence: Synthetic polypeptide"
RKVCNGIGIGEFKDSLSINATNIKHFKNCTSISGDLHILPVAFRGDSFTHTPPLDPQELDILKTVKEITGFLLIQAWPENRTDLHAFENLEIIRGRTKQHGQFSLAVVSLNITSLGLRSLKEISDGDVIISGNKNLCYANTINWKKLFGTSGQKTKIISNRGENSCKATGQVCHALCSPEGCWGPEPRDCVSCRNVSRGRECVDKCNLLEGEPREFVENSECIQCHPECLPQAMNITCTGRGPDNCIQCAHYIDGPHCVKTCPAGVMGENNTLVWKYADAGHVCHLCHPNCTYGCTGPGLEGCPTNGPKIPSIATGMVGALLLLLVVALGIGLFM

SEQ ID NO: 69 - DNA, 1482 bp, synthetic construct
  misc_feature 1..1482: note = source = /note="Description of Artificial Sequence: Synthetic polynucleotide"
  source 1..1482: mol_type = other DNA
atgcttcttttggtgacttcccttttgctgtgcgagttgccacaccccgccttcctgcttattccccaggtacagctccagcagagtggcccagggctcgtgaagccaagccagacgctgtccctgacttgtgcaatttcaggggattcagtttcatcaaatagcgcggcgtggaattggattcgacaatctccttcccgagggttggaatggcttggacgaacatattacagatccaaatggtataacgactatgcggtatcagtaaagtcaagaataaccattaaccccgacacaagcaagaaccaattctctttgcagcttaactctgtcacgccagaagacacggcagtctattattgcgctcgcgaggtaacgggtgacctggaagacgcttttgacatttgggggcagggtacgatggtgacagtcagttcagggggcggtgggagtgggggagggggtagcggggggggagggtcagacattcagatgacccagtccccttcatccttgtctgcctccgtcggtgacagggtgacaataacatgcagagcaagccaaacaatctggagctatctcaactggtaccagcagcgaccaggaaaagcgccaaacctgctgatttacgctgcttcctccctccaatcaggcgtgcctagtagatttagcggtaggggctccggcaccgattttacgctcactataagctctcttcaagcagaagattttgcgacttattactgccagcagtcctatagtatacctcagactttcggacagggtaccaagttggagattaaggcggccgcaactaccacccctgcccctcggccgccgactccggccccaaccatcgcaagccaacccctctccttgcgccccgaagcttgccgcccggccgcgggtggagccgtgcatacccgggggctggactttgcctgcgatatctacatttgggccccgctggccggcacttgcggcgtgctcctgctgtcgctggtcatcaccctttactgcaagaggggccggaagaagctgctttacatcttcaagcagccgttcatgcggcccgtgcagacgactcaggaagaggacggatgctcgtgcagattccctgaggaggaagaggggggatgcgaactgcgcgtcaagttctcacggtccgccgacgcccccgcatatcaacagggccagaatcagctctacaacgagctgaacctgggaaggagagaggagtacgacgtgctggacaagcgacgcggacgcgacccggagatgggggggaaaccacggcggaaaaaccctcaggaaggactgtacaacgaactccagaaagacaagatggcggaagcctactcagaaatcgggatgaagggagagcggaggaggggaaagggtcacgacgggctgtaccagggactgagcaccgccactaaggatacctacgatgccttgcatatgcaagcactcccaccccgg

SEQ ID NO: 70 - protein, 494 aa, synthetic construct
  REGION 1..494: note = source = /note="Description of Artificial Sequence: Synthetic polypeptide"
MLLLVTSLLLCELPHPAFLLIPQVQLQQSGPGLVKPSQTLSLTCAISGDSVSSNSAAWNWIRQSPSRGLEWLGRTYYRSKWYNDYAVSVKSRITINPDTSKNQFSLQLNSVTPEDTAVYYCAREVTGDLEDAFDIWGQGTMVTVSSGGGGSGGGGSGGGGSDIQMTQSPSSLSASVGDRVTITCRASQTIWSYLNWYQQRPGKAPNLLIYAASSLQSGVPSRFSGRGSGTDFTLTISSLQAEDFATYYCQQSYSIPQTFGQGTKLEIKAAATTTPAPRPPTPAPTIASQPLSLRPEACRPAAGGAVHTRGLDFACDIYIWAPLAGTCGVLLLSLVITLYCKRGRKKLLYIFKQPFMRPVQTTQEEDGCSCRFPEEEEGGCELRVKFSRSADAPAYQQGQNQLYNELNLGRREEYDVLDKRRGRDPEMGGKPRRKNPQEGLYNELQKDKMAEAYSEIGMKGERRRGKGHDGLYQGLSTATKDTYDALHMQALPPR

SEQ ID NO: 71 - DNA, 1485 bp, synthetic construct
  misc_feature 1..1485: note = source = /note="Description of Artificial Sequence: Synthetic polynucleotide"
  source 1..1485: mol_type = other DNA
atgcttctcctggtcacctccctgctcctctgcgaactgcctcaccctgccttccttctgattcctgacactgacattcagatgactcagaccacctcttccttgtccgcgtcactgggagacagagtgaccatctcgtgtcgcgcaagccaggatatctccaagtacctgaactggtaccaacagaagcccgacgggactgtgaagctgctgatctaccacacctcacgcctgcacagcggagtgccaagcagattctccggctccggctcgggaaccgattactcgcttaccattagcaacctcgagcaggaggacatcgctacctacttctgccagcaaggaaataccctgccctacaccttcggcggaggaaccaaattggaaatcaccggctccacgagcggctccgggaagcctggttccggggaaggctccactaagggtgaagtgaagctccaggagtccggccccggcctggtggcgccgtcgcaatcactctctgtgacctgtaccgtgtcgggagtgtccctgcctgattacggcgtgagctggattcggcagccgccgcggaagggcctggaatggctgggtgtcatctggggatccgagactacctactacaactcggccctgaagtcccgcctgactatcatcaaagacaactcgaagtcccaggtctttctgaagatgaactccctgcaaactgacgacaccgccatctattactgtgctaagcactactactacggtggaagctatgctatggactactggggccaggggacatccgtgacagtcagctccgcggccgcaactaccacccctgcccctcggccgccgactccggccccaaccatcgcaagccaacccctctccttgcgccccgaagcttgccgcccggccgcgggtggagccgtgcatacccgggggctggactttgcctgcgatatctacatttgggccccgctggccggcacttgcggcgtgctcctgctgtcgctggtcatcaccctttactgcaagaggggccggaagaagctgctttacatcttcaagcagccgttcatgcggcccgtgcagacgactcaggaagaggacggatgctcgtgcagattccctgaggaggaagaggggggatgcgaactgcgcgtcaagttctcacggtccgccgacgcccccgcatatcaacagggccagaatcagctctacaacgagctgaacctgggaaggagagaggagtacgacgtgctggacaagcgacgcggacgcgacccggagatgggggggaaaccacggcggaaaaaccctcaggaaggactgtacaacgaactccagaaagacaagatggcggaagcctactcagaaatcgggatgaagggagagcggaggaggggaaagggtcacgacgggctgtaccagggactgagcaccgccactaaggatacctacgatgccttgcatatgcaagcactcccaccccgg

SEQ ID NO: 72 - protein, 495 aa, synthetic construct
  REGION 1..495: note = source = /note="Description of Artificial Sequence: Synthetic polypeptide"
MLLLVTSLLLCELPHPAFLLIPDTDIQMTQTTSSLSASLGDRVTISCRASQDISKYLNWYQQKPDGTVKLLIYHTSRLHSGVPSRFSGSGSGTDYSLTISNLEQEDIATYFCQQGNTLPYTFGGGTKLEITGSTSGSGKPGSGEGSTKGEVKLQESGPGLVAPSQSLSVTCTVSGVSLPDYGVSWIRQPPRKGLEWLGVIWGSETTYYNSALKSRLTIIKDNSKSQVFLKMNSLQTDDTAIYYCAKHYYYGGSYAMDYWGQGTSVTVSSAAATTTPAPRPPTPAPTIASQPLSLRPEACRPAAGGAVHTRGLDFACDIYIWAPLAGTCGVLLLSLVITLYCKRGRKKLLYIFKQPFMRPVQTTQEEDGCSCRFPEEEEGGCELRVKFSRSADAPAYQQGQNQLYNELNLGRREEYDVLDKRRGRDPEMGGKPRRKNPQEGLYNELQKDKMAEAYSEIGMKGERRRGKGHDGLYQGLSTATKDTYDALHMQALPPR

SEQ ID NO: 73 - DNA, 1470 bp, synthetic construct
  misc_feature 1..1470: note = source = /note="Description of Artificial Sequence: Synthetic polynucleotide"
  source 1..1470: mol_type = other DNA
atgcttctcctggtcacctccctgctcctctgcgaactgcctcaccctgccttccttctgattcctgacattcagatgactcagaccacctcttccttgtccgcgtcactgggagacagagtgaccatctcgtgtcgcgcaagccaggatatctccaagtacctgaactggtaccaacagaagcccgacgggactgtgaagctgctgatctaccacacctcacgcctgcacagcggagtgccaagcagattctccggctccggctcgggaaccgattactcgcttaccattagcaacctcgagcaggaggacatcgctacctacttctgccagcaaggaaataccctgccctacaccttcggcggaggaaccaaattggaaatcaccggcggaggaggctccgggggaggaggttccgggggcgggggttccgaagtgaagctccaggagtccggccccggcctggtggcgccgtcgcaatcactctctgtgacctgtaccgtgtcgggagtgtccctgcctgattacggcgtgagctggattcggcagccgccgcggaagggcctggaatggctgggtgtcatctggggatccgagactacctactacaactcggccctgaagtcccgcctgactatcatcaaagacaactcgaagtcccaggtctttctgaagatgaactccctgcaaactgacgacaccgccatctattactgtgctaagcactactactacggtggaagctatgctatggactactgggggcaaggcacttcggtgactgtgtcaagcgcggccgcaactaccacccctgcccctcggccgccgactccggccccaaccatcgcaagccaacccctctccttgcgccccgaagcttgccgcccggccgcgggtggagccgtgcatacccgggggctggactttgcctgcgatatctacatttgggccccgctggccggcacttgcggcgtgctcctgctgtcgctggtcatcaccctttactgcaagaggggccggaagaagctgctttacatcttcaagcagccgttcatgcggcccgtgcagacgactcaggaagaggacggatgctcgtgcagattccctgaggaggaagaggggggatgcgaactgcgcgtcaagttctcacggtccgccgacgcccccgcatatcaacagggccagaatcagctctacaacgagctgaacctgggaaggagagaggagtacgacgtgctggacaagcgacgcggacgcgacccggagatgggggggaaaccacggcggaaaaaccctcaggaaggactgtacaacgaactccagaaagacaagatggcggaagcctactcagaaatcgggatgaagggagagcggaggaggggaaagggtcacgacgggctgtaccagggactgagcaccgccactaaggatacctacgatgccttgcatatgcaagcactcccaccccgg

SEQ ID NO: 74 - protein, 490 aa, synthetic construct
  REGION 1..490: note = source = /note="Description of Artificial Sequence: Synthetic polypeptide"
MLLLVTSLLLCELPHPAFLLIPDIQMTQTTSSLSASLGDRVTISCRASQDISKYLNWYQQKPDGTVKLLIYHTSRLHSGVPSRFSGSGSGTDYSLTISNLEQEDIATYFCQQGNTLPYTFGGGTKLEITGGGGSGGGGSGGGGSEVKLQESGPGLVAPSQSLSVTCTVSGVSLPDYGVSWIRQPPRKGLEWLGVIWGSETTYYNSALKSRLTIIKDNSKSQVFLKMNSLQTDDTAIYYCAKHYYYGGSYAMDYWGQGTSVTVSSAAATTTPAPRPPTPAPTIASQPLSLRPEACRPAAGGAVHTRGLDFACDIYIWAPLAGTCGVLLLSLVITLYCKRGRKKLLYIFKQPFMRPVQTTQEEDGCSCRFPEEEEGGCELRVKFSRSADAPAYQQGQNQLYNELNLGRREEYDVLDKRRGRDPEMGGKPRRKNPQEGLYNELQKDKMAEAYSEIGMKGERRRGKGHDGLYQGLSTATKDTYDALHMQALPPR

SEQ ID NO: 75 - DNA, 1467 bp, synthetic construct
  misc_feature 1..1467: note = source = /note="Description of Artificial Sequence: Synthetic polynucleotide"
  source 1..1467: mol_type = other DNA
atgctgctgctggtgaccagcctgctgctgtgcgaactgccgcatccggcgtttctgctgattccggatattcagatgacccagaccaccagcagcctgagcgcgagcctgggcgatcgcgtgaccattagctgccgcgcgagccaggatattagcaaatatctgaactggtatcagcagaaaccggatggcaccgtgaaactgctgatttatcataccagccgcctgcatagcggcgtgccgagccgctttagcggcagcggcagcggcaccgattatagcctgaccattagcaacctggaacaggaagatattgcgacctatttttgccagcagggcaacaccctgccgtatacctttggcggcggcaccaaactggaaattaccggcggcggcggcagcggcggcggcggcagcggcggcggcggcagcgaagtgaaactgcaggaaagcggcccgggcctggtggcgccgagccagagcctgagcgtgacctgcaccgtgagcggcgtgagcctgccggattatggcgtgagctggattcgccagccgccgcgcaaaggcctggaatggctgggcgtgatttggggcagcgaaaccacctattataacagcgcgctgaaaagccgcctgaccattattaaagataacagcaaaagccaggtgtttctgaaaatgaacagcctgcagaccgatgataccgcgatttattattgcgcgaaacattattattatggcggcagctatgcgatggattattggggccagggcaccagcgtgaccgtgagcagcgcggcggcgccggcgccgcgcccgccgaccccggcgccgaccattgcgagccagccgctgagcctgcgcccggaagcgtgccgcccggcggcgggcggcgcggtgcatacccgcggcctggattttgtgcagccgatggcgctgattgtgctgggcggcgtggcgggcctgctgctgtttattggcctgggcatttttttttgcgtgcgctgccgcccgcgccgcaaaaaactgctgtatatttttaaacagccgtttatgcgcccggtgcagaccacccaggaagaagatggctgcagctgccgctttccggaagaagaagaaggcggctgcgaactgcgcgtgaaatttagccgcagcgcggatgcgccggcgtatcagcagggccagaaccagctgtataacgaactgaacctgggccgccgcgaagaatatgatgtgctggataaacgccgcggccgcgatccggaaatgggcggcaaaccgcgccgcaaaaacccgcaggaaggcctgtataacgaactgcagaaagataaaatggcggaagcgtatagcgaaattggcatgaaaggcgaacgccgccgcggcaaaggccatgatggcctgtatcagggcctgagcaccgcgaccaaagatacctatgatgcgctgcatatgcaggcgctgccgccgcgc

SEQ ID NO: 76 - protein, 489 aa, synthetic construct
  REGION 1..489: note = source = /note="Description of Artificial Sequence: Synthetic polypeptide"
MLLLVTSLLLCELPHPAFLLIPDIQMTQTTSSLSASLGDRVTISCRASQDISKYLNWYQQKPDGTVKLLIYHTSRLHSGVPSRFSGSGSGTDYSLTISNLEQEDIATYFCQQGNTLPYTFGGGTKLEITGGGGSGGGGSGGGGSEVKLQESGPGLVAPSQSLSVTCTVSGVSLPDYGVSWIRQPPRKGLEWLGVIWGSETTYYNSALKSRLTIIKDNSKSQVFLKMNSLQTDDTAIYYCAKHYYYGGSYAMDYWGQGTSVTVSSAAAPAPRPPTPAPTIASQPLSLRPEACRPAAGGAVHTRGLDFVQPMALIVLGGVAGLLLFIGLGIFFCVRCRPRRKKLLYIFKQPFMRPVQTTQEEDGCSCRFPEEEEGGCELRVKFSRSADAPAYQQGQNQLYNELNLGRREEYDVLDKRRGRDPEMGGKPRRKNPQEGLYNELQKDKMAEAYSEIGMKGERRRGKGHDGLYQGLSTATKDTYDALHMQALPPR

SEQ ID NO: 77 - DNA, 1467 bp, synthetic construct
  misc_feature 1..1467: note = source = /note="Description of Artificial Sequence: Synthetic polynucleotide"
  source 1..1467: mol_type = other DNA
atgctgctgctggtcaccagcctgctgctgtgcgagctccctcaccccgcctttctgcttatcccggacattcagatgacacagaccacctcgagcttgtccgcgtcgctgggcgatcgcgtgaccatctcctgccgggcctcccaagacatttcaaagtatctcaactggtaccagcagaagccggacggaaccgtgaaactgctgatctaccataccagccgcctgcactccggcgtgccgtcccgcttctccggatcgggttccggaactgactactcactgactatctccaacttggaacaagaggacatcgccacttacttctgtcaacaaggaaatacccttccctacaccttcggggggggtaccaagctggagatcactgggggcggaggctccggtggaggcggatccggcggtggagggagcgaagtcaagctgcaggaatcaggaccaggactcgtggcgccatcccagtccctgtcggtgacctgtactgtctccggagtcagcctccccgattacggagtgtcatggattaggcaacccccaagaaaagggctggaatggctcggagtgatctggggctccgaaaccacctactacaactcggcgctgaagtcccggctgaccatcatcaaggacaactccaagagccaagtgttcttgaagatgaacagcttgcagaccgacgataccgcaatctactactgtgccaagcactattactacggggggtcttacgccatggactactggggacagggcacctccgtgactgtgtcgtccgcggccgcgcccgcccctcggcccccgactcctgccccgacgatcgcttcccaacctctctcgctgcgcccggaagcatgccggcccgccgccggtggcgctgtccacactcgcggactggactttgataccgcactggcggccgtgatctgtagcgccctggccaccgtgctgctggcgctgctcatcctttgcgtgatctactgcaagcggcagcctaggcgaaagaagctcctctacattttcaagcaacccttcatgcgccccgtgcaaaccacccaggaggaggatggatgctcatgccggttccctgaggaagaagagggcggttgcgagctcagagtgaaattcagccggtcggctgacgccccggcgtaccagcagggccagaaccagctgtacaatgagctcaacctggggcgccgcgaagagtacgacgtgctggacaagaggagaggcagagatccggaaatgggcggaaagccaaggcggaagaacccgcaggaaggtctttacaacgaactgcagaaggacaagatggccgaggcctactccgagattgggatgaagggagaaagacggaggggaaagggacatgacggactttaccagggcctgagcactgccacgaaggacacctatgatgccctgcacatgcaggcgctgccgcctcgg

SEQ ID NO: 78 - protein, 489 aa, synthetic construct
  REGION 1..489: note = source = /note="Description of Artificial Sequence: Synthetic polypeptide"
MLLLVTSLLLCELPHPAFLLIPDIQMTQTTSSLSASLGDRVTISCRASQDISKYLNWYQQKPDGTVKLLIYHTSRLHSGVPSRFSGSGSGTDYSLTISNLEQEDIATYFCQQGNTLPYTFGGGTKLEITGGGGSGGGGSGGGGSEVKLQESGPGLVAPSQSLSVTCTVSGVSLPDYGVSWIRQPPRKGLEWLGVIWGSETTYYNSALKSRLTIIKDNSKSQVFLKMNSLQTDDTAIYYCAKHYYYGGSYAMDYWGQGTSVTVSSAAAPAPRPPTPAPTIASQPLSLRPEACRPAAGGAVHTRGLDFDTALAAVICSALATVLLALLILCVIYCKRQPRRKKLLYIFKQPFMRPVQTTQEEDGCSCRFPEEEEGGCELRVKFSRSADAPAYQQGQNQLYNELNLGRREEYDVLDKRRGRDPEMGGKPRRKNPQEGLYNELQKDKMAEAYSEIGMKGERRRGKGHDGLYQGLSTATKDTYDALHMQALPPR

SEQ ID NO: 79 - DNA, 36 bp, Homo sapiens
  source 1..36: mol_type = other DNA
gagagcaaatacgggccgccatgtcccccgtgtccg

SEQ ID NO: 80 - protein, 12 aa, Homo sapiens
ESKYGPPCPPCP

SEQ ID NO: 81 - DNA, 327 bp, Homo sapiens
  source 1..327: mol_type = other DNA
gcaccaccagttgctggccctagtgtcttcttgttccctcccaagcccaaagacaccttgatgatttccagaactcctgaggttacctgcgttgtcgtagatgtttctcaggaggacccagaggtccaatttaactggtacgttgatggggtggaagttcacaatgcgaagacaaagccgcgggaagaacaatttcagtccacttaccgggttgtcagcgttctgacggtattgcatcaagactggcttaatggaaaggaatataagtgtaaggtgtccaacaaaggtttgccgagcagtattgagaagaccatatcaaaggcgaag

SEQ ID NO: 82 - protein, 109 aa, Homo sapiens
APPVAGPSVFLFPPKPKDTLMISRTPEVTCVVVDVSQEDPEVQFNWYVDGVEVHNAKTKPREEQFQSTYRVVSVLTVLHQDWLNGKEYKCKVSNKGLPSSIEKTISKAK

SEQ ID NO: 83 - DNA, 321 bp, Homo sapiens
  source 1..321: mol_type = other DNA
gggcagccgcgcgagccacaagtttacactttgccgccatctcaagaggaaatgactaaaaaccaggtatccttgacatgcctcgtaaaaggattttatccatctgatattgctgtggaatgggagtctaacgggcagccggaaaataattacaaaactacaccacctgtgctcgattcagatggaagtttcttcctttacagtagacttacggtggacaaatctaggtggcaggaagggaatgtgtttagttgtagtgtaatgcacgaggcacttcataaccactatacacagaagtcactgagtttgagtcttggcaaa

SEQ ID NO: 84 - protein, 107 aa, Homo sapiens
GQPREPQVYTLPPSQEEMTKNQVSLTCLVKGFYPSDIAVEWESNGQPENNYKTTPPVLDSDGSFFLYSRLTVDKSRWQEGNVFSCSVMHEALHNHYTQKSLSLSLGK

SEQ ID NO: 85 - DNA, 684 bp, Homo sapiens
  source 1..684: mol_type = other DNA
gagagcaaatacgggccgccatgtcccccgtgtccggcaccaccagttgctggccctagtgtcttcttgttccctcccaagcccaaagacaccttgatgatttccagaactcctgaggttacctgcgttgtcgtagatgtttctcaggaggacccagaggtccaatttaactggtacgttgatggggtggaagttcacaatgcgaagacaaagccgcgggaagaacaatttcagtccacttaccgggttgtcagcgttctgacggtattgcatcaagactggcttaatggaaaggaatataagtgtaaggtgtccaacaaaggtttgccgagcagtattgagaagaccatatcaaaggcgaaggggcagccgcgcgagccacaagtttacactttgccgccatctcaagaggaaatgactaaaaaccaggtatccttgacatgcctcgtaaaaggattttatccatctgatattgctgtggaatgggagtctaacgggcagccggaaaataattacaaaactacaccacctgtgctcgattcagatggaagtttcttcctttacagtagacttacggtggacaaatctaggtggcaggaagggaatgtgtttagttgtagtgtaatgcacgaggcacttcataaccactatacacagaagtcactgagtttgagtcttggcaaa

SEQ ID NO: 86 - protein, 228 aa, Homo sapiens
ESKYGPPCPPCPAPPVAGPSVFLFPPKPKDTLMISRTPEVTCVVVDVSQEDPEVQFNWYVDGVEVHNAKTKPREEQFQSTYRVVSVLTVLHQDWLNGKEYKCKVSNKGLPSSIEKTISKAKGQPREPQVYTLPPSQEEMTKNQVSLTCLVKGFYPSDIAVEWESNGQPENNYKTTPPVLDSDGSFFLYSRLTVDKSRWQEGNVFSCSVMHEALHNHYTQKSLSLSLGK

SEQ ID NO: 87 - DNA, 732 bp, synthetic construct
  misc_feature 1..732: note = source = /note="Description of Artificial Sequence: Synthetic polynucleotide"
  source 1..732: mol_type = other DNA
gaggtccagctggtacagtctgggggaggcttggtacagcctggggggtccctgagactctcctgtgcagcctctggattcacctttgatgattatgccatgcactgggtccggcaagctccagggaagggcctggagtgggtctcaggtattagttggaatagtggtagcataggctatgcggactctgtgaagggccgattcaccatctccagagacaacgccaagaactccctgtatctgcaaatgaacagtctgagagctgaggacacggccttgtattactgtgcaaaagatttatcgtcagtggctggaccctttaactactggggccagggcaccctggtcaccgtctcctcaggaggtggcgggtctggtggaggcggtagcggcggtggcggatcctcttctgagctgactcaggaccctgctgtgtctgtggccttgggacagacagtcaggatcacatgccaaggagacagcctcagaagctattatgcaagctggtaccagcagaagccaggacaggcccctgtacttgtcatctatggtaaaaacaaccggccctcagggatcccagaccgattctctggctccagctcaggaaacacagcttccttgaccatcactggggctcaggcggaggatgaggctgactattactgtaactcccgggacagcagtggtaaccatctggtattcggcggaggcacccagctgaccgtcctcggt

SEQ ID NO: 88 - protein, 244 aa, synthetic construct
  REGION 1..244: note = source = /note="Description of Artificial Sequence: Synthetic polypeptide"
EVQLVQSGGGLVQPGGSLRLSCAASGFTFDDYAMHWVRQAPGKGLEWVSGISWNSGSIGYADSVKGRFTISRDNAKNSLYLQMNSLRAEDTALYYCAKDLSSVAGPFNYWGQGTLVTVSSGGGGSGGGGSGGGGSSSELTQDPAVSVALGQTVRITCQGDSLRSYYASWYQQKPGQAPVLVIYGKNNRPSGIPDRFSGSSSGNTASLTITGAQAEDEADYYCNSRDSSGNHLVFGGGTQLTVLG

SEQ ID NO: 89 - DNA, 1476 bp, synthetic construct
  misc_feature 1..1476: note = source = /note="Description of Artificial Sequence: Synthetic polynucleotide"
  source 1..1476: mol_type = other DNA
atgctgctgctggtgaccagcctgctgctgtgcgaactgccgcatccggcgtttctgctgattccggaggtccagctggtacagtctgggggaggcttggtacagcctggggggtccctgagactctcctgtgcagcctctggattcacctttgatgattatgccatgcactgggtccggcaagctccagggaagggcctggagtgggtctcaggtattagttggaatagtggtagcataggctatgcggactctgtgaagggccgattcaccatctccagagacaacgccaagaactccctgtatctgcaaatgaacagtctgagagctgaggacacggccttgtattactgtgcaaaagatttatcgtcagtggctggaccctttaactactggggccagggcaccctggtcaccgtctcctcaggaggtggcgggtctggtggaggcggtagcggcggtggcggatcctcttctgagctgactcaggaccctgctgtgtctgtggccttgggacagacagtcaggatcacatgccaaggagacagcctcagaagctattatgcaagctggtaccagcagaagccaggacaggcccctgtacttgtcatctatggtaaaaacaaccggccctcagggatcccagaccgattctctggctccagctcaggaaacacagcttccttgaccatcactggggctcaggcggaggatgaggctgactattactgtaactcccgggacagcagtggtaaccatctggtattcggcggaggcacccagctgaccgtcctcggtgcggccgcaactaccacccctgcccctcggccgccgactccggccccaaccatcgcaagccaacccctctccttgcgccccgaagcttgccgcccggccgcgggtggagccgtgcatacccgggggctggactttgcctgcgatatctacatttgggccccgctggccggcacttgcggcgtgctcctgctgtcgctggtcatcaccctttactgcaagaggggccggaagaagctgctttacatcttcaagcagccgttcatgcggcccgtgcagacgactcaggaagaggacggatgctcgtgcagattccctgaggaggaagaggggggatgcgaactgcgcgtcaagttctcacggtccgccgacgcccccgcatatcaacagggccagaatcagctctacaacgagctgaacctgggaaggagagaggagtacgacgtgctggacaagcgacgcggacgcgacccggagatgggggggaaaccacggcggaaaaaccctcaggaaggactgtacaacgaactccagaaagacaagatggcggaagcctactcagaaatcgggatgaagggagagcggaggaggggaaagggtcacgacgggctgtaccagggactgagcaccgccactaaggatacctacgatgccttgcatatgcaagcactcccaccccgg

SEQ ID NO: 90 - protein, 492 aa, synthetic construct
  REGION 1..492: note = source = /note="Description of Artificial Sequence: Synthetic polypeptide"
MLLLVTSLLLCELPHPAFLLIPEVQLVQSGGGLVQPGGSLRLSCAASGFTFDDYAMHWVRQAPGKGLEWVSGISWNSGSIGYADSVKGRFTISRDNAKNSLYLQMNSLRAEDTALYYCAKDLSSVAGPFNYWGQGTLVTVSSGGGGSGGGGSGGGGSSSELTQDPAVSVALGQTVRITCQGDSLRSYYASWYQQKPGQAPVLVIYGKNNRPSGIPDRFSGSSSGNTASLTITGAQAEDEADYYCNSRDSSGNHLVFGGGTQLTVLGAAATTTPAPRPPTPAPTIASQPLSLRPEACRPAAGGAVHTRGLDFACDIYIWAPLAGTCGVLLLSLVITLYCKRGRKKLLYIFKQPFMRPVQTTQEEDGCSCRFPEEEEGGCELRVKFSRSADAPAYQQGQNQLYNELNLGRREEYDVLDKRRGRDPEMGGKPRRKNPQEGLYNELQKDKMAEAYSEIGMKGERRRGKGHDGLYQGLSTATKDTYDALHMQALPPR

SEQ ID NO: 91 - DNA, 339 bp, synthetic construct
  misc_feature 1..339: note = source = /note="Description of Artificial Sequence: Synthetic polynucleotide"
  source 1..339: mol_type = other DNA
gaggtgcagctggtggagtctgggggaggcttggtacagcctggagggtccctgagactctcctgtgcagcctctggattcaccttcagtagctatggcatgagctgggtccgccaggctccaagacaagggcttgagtgggtggccaacataaagcaagatggaagtgagaaatactatgcggactcagtgaagggccgattcaccatctccagagacaattccaagaacacgctgtatctgcaaatgaacagcctgagagccgaggacacagccacgtattactgtgcgaaagaaaatgtggactggggccagggcaccctggtcaccgtctcctca

SEQ ID NO: 92 - protein, 113 aa, synthetic construct
  REGION 1..113: note = source = /note="Description of Artificial Sequence: Synthetic polypeptide"
EVQLVESGGGLVQPGGSLRLSCAASGFTFSSYGMSWVRQAPRQGLEWVANIKQDGSEKYYADSVKGRFTISRDNSKNTLYLQMNSLRAEDTATYYCAKENVDWGQGTLVTVSS

SEQ ID NO: 93 - DNA, 1083 bp, synthetic construct
  misc_feature 1..1083: note = source = /note="Description of Artificial Sequence: Synthetic polynucleotide"
  source 1..1083: mol_type = other DNA
atgctgctgctggtgaccagcctgctgctgtgcgaactgccgcatccggcgtttctgctgattccggaggtgcagctggtggagtctgggggaggcttggtacagcctggagggtccctgagactctcctgtgcagcctctggattcaccttcagtagctatggcatgagctgggtccgccaggctccaagacaagggcttgagtgggtggccaacataaagcaagatggaagtgagaaatactatgcggactcagtgaagggccgattcaccatctccagagacaattccaagaacacgctgtatctgcaaatgaacagcctgagagccgaggacacagccacgtattactgtgcgaaagaaaatgtggactggggccagggcaccctggtcaccgtctcctcagcggccgcaactaccacccctgcccctcggccgccgactccggccccaaccatcgcaagccaacccctctccttgcgccccgaagcttgccgcccggccgcgggtggagccgtgcatacccgggggctggactttgcctgcgatatctacatttgggccccgctggccggcacttgcggcgtgctcctgctgtcgctggtcatcaccctttactgcaagaggggccggaagaagctgctttacatcttcaagcagccgttcatgcggcccgtgcagacgactcaggaagaggacggatgctcgtgcagattccctgaggaggaagaggggggatgcgaactgcgcgtcaagttctcacggtccgccgacgcccccgcatatcaacagggccagaatcagctctacaacgagctgaacctgggaaggagagaggagtacgacgtgctggacaagcgacgcggacgcgacccggagatgggggggaaaccacggcggaaaaaccctcaggaaggactgtacaacgaactccagaaagacaagatggcggaagcctactcagaaatcgggatgaagggagagcggaggaggggaaagggtcacgacgggctgtaccagggactgagcaccgccactaaggatacctacgatgccttgcatatgcaagcactcccaccccgg

SEQ ID NO: 94 - protein, 361 aa, synthetic construct
  REGION 1..361: note = source = /note="Description of Artificial Sequence: Synthetic polypeptide"
MLLLVTSLLLCELPHPAFLLIPEVQLVESGGGLVQPGGSLRLSCAASGFTFSSYGMSWVRQAPRQGLEWVANIKQDGSEKYYADSVKGRFTISRDNSKNTLYLQMNSLRAEDTATYYCAKENVDWGQGTLVTVSSAAATTTPAPRPPTPAPTIASQPLSLRPEACRPAAGGAVHTRGLDFACDIYIWAPLAGTCGVLLLSLVITLYCKRGRKKLLYIFKQPFMRPVQTTQEEDGCSCRFPEEEEGGCELRVKFSRSADAPAYQQGQNQLYNELNLGRREEYDVLDKRRGRDPEMGGKPRRKNPQEGLYNELQKDKMAEAYSEIGMKGERRRGKGHDGLYQGLSTATKDTYDALHMQALPPR

SEQ ID NO: 95 - DNA, 2283 bp, synthetic construct
  misc_feature 1..2283: note = source = /note="Description of Artificial Sequence: Synthetic polynucleotide"
  source 1..2283: mol_type = other DNA
atgctccttctcgtgacctccctgcttctctgcgaactgccccatcctgccttcctgctgattcccgacattcagatgactcagaccacctcctccctgtccgcctccctgggcgaccgcgtgaccatctcatgccgcgccagccaggacatctcgaagtacctcaactggtaccagcagaagcccgacggaaccgtgaagctcctgatctaccacacctcccggctgcacagcggagtgccgtctagattctcgggttcggggtcgggaactgactactcccttactatttccaacctggagcaggaggatattgccacctacttctgccaacaaggaaacaccctgccgtacacttttggcgggggaaccaagctggaaatcactggcagcacatccggttccgggaagcccggctccggagagggcagcaccaagggggaagtcaagctgcaggaatcaggacctggcctggtggccccgagccagtcactgtccgtgacttgtactgtgtccggagtgtcgctcccggattacggagtgtcctggatcaggcagccacctcggaaaggattggaatggctcggagtcatctggggttccgaaaccacctattacaactcggcactgaaatccaggctcaccattatcaaggataactccaagtcacaagtgttcctgaagatgaatagcctgcagactgacgacacggcgatctactattgcgccaagcactactactacggcggatcctacgctatggactactggggccaggggaccagcgtgaccgtgtcatccggaggcggcggcagcggcgggggagggtccggagggggtggttctggtggaggaggatcgggaggcggtggcagcgaggtgcagttgcaacagtcaggagctgaactggtcaagccaggagccagcgtgaagatgagctgcaaggcctccggttacaccttcacctcctacaacatgcactgggtgaaacagaccccgggacaagggctcgaatggattggcgccatctaccccgggaatggcgatacttcgtacaaccagaagttcaagggaaaggccaccctgaccgccgacaagagctcctccaccgcgtatatgcagttgagctccctgacctccgaggactccgccgactactactgcgcacggtccaactactatggaagctcgtactggttcttcgatgtctggggggccggcaccactgtgaccgtcagctccgggggcggaggatccggtggaggcggaagcgggggtggaggatccgacattgtgctgactcagtccccggcaatcctgtcggcctcaccgggcgaaaaggtcacgatgacttgtagagcgtcgtccagcgtgaactacatggattggtaccaaaagaagcctggatcgtcacccaagccttggatctacgctacatctaacctggcctccggcgtgccagcgcggttcagcgggtccggctcgggcacctcatactcgctgaccatctcccgcgtggaggctgaggacgccgcgacctactactgccagcagtggtccttcaacccgccgacttttggaggcggtactaagctggagatcaaagcggccgcaactaccacccctgcccctcggccgccgactccggccccaaccatcgcaagccaacccctctccttgcgccccgaagcttgccgcccggccgcgggtggagccgtgcatacccgggggctggactttgcctgcgatatctacatttgggccccgctggccggcacttgcggcgtgctcctgctgtcgctggtcatcaccctttactgcaagaggggccggaagaagctgctttacatcttcaagcagccgttcatgcggcccgtgcagacgactcaggaagaggacggatgctcgtgcagattccctgaggaggaagaggggggatgcgaactgcgcgtcaagttctcacggtccgccgacgcccccgcatatcaacagggccagaatcagctctacaacgagctgaacctgggaaggagagaggagtacgacgtgctggacaagcgacgcggacgcgacccggagatgggggggaaaccacggcggaaaaaccctcaggaaggactgtacaacgaactccagaaagacaagatggcggaagcctactcagaaatcgggatgaagggagagcggaggaggggaaagggtcacgacgggctgtaccagggactgagcaccgccactaaggatacctacgatgccttgcatatgcaagcactcccaccccgg

SEQ ID NO: 96 - protein, 761 aa, synthetic construct
  REGION 1..761: note = source = /note="Description of Artificial Sequence: Synthetic polypeptide"
MLLLVTSLLLCELPHPAFLLIPDIQMTQTTSSLSASLGDRVTISCRASQDISKYLNWYQQKPDGTVKLLIYHTSRLHSGVPSRFSGSGSGTDYSLTISNLEQEDIATYFCQQGNTLPYTFGGGTKLEITGSTSGSGKPGSGEGSTKGEVKLQESGPGLVAPSQSLSVTCTVSGVSLPDYGVSWIRQPPRKGLEWLGVIWGSETTYYNSALKSRLTIIKDNSKSQVFLKMNSLQTDDTAIYYCAKHYYYGGSYAMDYWGQGTSVTVSSGGGGSGGGGSGGGGSGGGGSGGGGSEVQLQQSGAELVKPGASVKMSCKASGYTFTSYNMHWVKQTPGQGLEWIGAIYPGNGDTSYNQKFKGKATLTADKSSSTAYMQLSSLTSEDSADYYCARSNYYGSSYWFFDVWGAGTTVTVSSGGGGSGGGGSGGGGSDIVLTQSPAILSASPGEKVTMTCRASSSVNYMDWYQKKPGSSPKPWIYATSNLASGVPARFSGSGSGTSYSLTISRVEAEDAATYYCQQWSFNPPTFGGGTKLEIKAAATTTPAPRPPTPAPTIASQPLSLRPEACRPAAGGAVHTRGLDFACDIYIWAPLAGTCGVLLLSLVITLYCKRGRKKLLYIFKQPFMRPVQTTQEEDGCSCRFPEEEEGGCELRVKFSRSADAPAYQQGQNQLYNELNLGRREEYDVLDKRRGRDPEMGGKPRRKNPQEGLYNELQKDKMAEAYSEIGMKGERRRGKGHDGLYQGLSTATKDTYDALHMQALPPR

SEQ ID NO: 97 - DNA, 2283 bp, synthetic construct
  misc_feature 1..2283: note = source = /note="Description of Artificial Sequence: Synthetic polynucleotide"
  source 1..2283: mol_type = other DNA
atgctccttctcgtgacctccctgcttctctgcgaactgccccatcctgccttcctgctgattcccgaggtgcagttgcaacagtcaggagctgaactggtcaagccaggagccagcgtgaagatgagctgcaaggcctccggttacaccttcacctcctacaacatgcactgggtgaaacagaccccgggacaagggctcgaatggattggcgccatctaccccgggaatggcgatacttcgtacaaccagaagttcaagggaaaggccaccctgaccgccgacaagagctcctccaccgcgtatatgcagttgagctccctgacctccgaggactccgccgactactactgcgcacggtccaactactatggaagctcgtactggttcttcgatgtctggggggccggcaccactgtgaccgtcagctccgggggcggaggatccggtggaggcggaagcgggggtggaggatccgacattgtgctgactcagtccccggcaatcctgtcggcctcaccgggcgaaaaggtcacgatgacttgtagagcgtcgtccagcgtgaactacatggattggtaccaaaagaagcctggatcgtcacccaagccttggatctacgctacatctaacctggcctccggcgtgccagcgcggttcagcgggtccggctcgggcacctcatactcgctgaccatctcccgcgtggaggctgaggacgccgcgacctactactgccagcagtggtccttcaacccgccgacttttggaggcggtactaagctggagatcaaaggaggcggcggcagcggcgggggagggtccggagggggtggttctggtggaggaggatcgggaggcggtggcagcgacattcagatgactcagaccacctcctccctgtccgcctccctgggcgaccgcgtgaccatctcatgccgcgccagccaggacatctcgaagtacctcaactggtaccagcagaagcccgacggaaccgtgaagctcctgatctaccacacctcccggctgcacagcggagtgccgtctagattctcgggttcggggtcgggaactgactactcccttactatttccaacctggagcaggaggatattgccacctacttctgccaacaaggaaacaccctgccgtacacttttggcgggggaaccaagctggaaatcactggcagcacatccggttccgggaagcccggctccggagagggcagcaccaagggggaagtcaagctgcaggaatcaggacctggcctggtggccccgagccagtcactgtccgtgacttgtactgtgtccggagtgtcgctcccggattacggagtgtcctggatcaggcagccacctcggaaaggattggaatggctcggagtcatctggggttccgaaaccacctattacaactcggcactgaaatccaggctcaccattatcaaggataactccaagtcacaagtgttcctgaagatgaatagcctgcagactgacgacacggcgatctactattgcgccaagcactactactacggcggatcctacgctatggactactggggccaggggaccagcgtgaccgtgtcatccgcggccgcaactaccacccctgcccctcggccgccgactccggccccaaccatcgcaagccaacccctctccttgcgccccgaagcttgccgcccggccgcgggtggagccgtgcatacccgggggctggactttgcctgcgatatctacatttgggccccgctggccggcacttgcggcgtgctcctgctgtcgctggtcatcaccctttactgcaagaggggccggaagaagctgctttacatcttcaagcagccgttcatgcggcccgtgcagacgactcaggaagaggacggatgctcgtgcagattccctgaggaggaagaggggggatgcgaactgcgcgtcaagttctcacggtccgccgacgcccccgcatatcaacagggccagaatcagctctacaacgagctgaacctgggaaggagagaggagtacgacgtgctggacaagcgacgcggacgcgacccggagatgggggggaaaccacggcggaaaaaccctcaggaaggactgtacaacgaactccagaaagacaagatggcggaagcctactcagaaatcgggatgaagggagagcggaggaggggaaagggtcacgacgggctgtaccagggactgagcaccgccactaaggatacctacgatgccttgcatatgcaagcactcccaccccgg

SEQ ID NO: 98 - protein, 761 aa, synthetic construct
  REGION 1..761: note = source = /note="Description of Artificial Sequence: Synthetic polypeptide"
MLLLVTSLLLCELPHPAFLLIPEVQLQQSGAELVKPGASVKMSCKASGYTFTSYNMHWVKQTPGQGLEWIGAIYPGNGDTSYNQKFKGKATLTADKSSSTAYMQLSSLTSEDSADYYCARSNYYGSSYWFFDVWGAGTTVTVSSGGGGSGGGGSGGGGSDIVLTQSPAILSASPGEKVTMTCRASSSVNYMDWYQKKPGSSPKPWIYATSNLASGVPARFSGSGSGTSYSLTISRVEAEDAATYYCQQWSFNPPTFGGGTKLEIKGGGGSGGGGSGGGGSGGGGSGGGGSDIQMTQTTSSLSASLGDRVTISCRASQDISKYLNWYQQKPDGTVKLLIYHTSRLHSGVPSRFSGSGSGTDYSLTISNLEQEDIATYFCQQGNTLPYTFGGGTKLEITGSTSGSGKPGSGEGSTKGEVKLQESGPGLVAPSQSLSVTCTVSGVSLPDYGVSWIRQPPRKGLEWLGVIWGSETTYYNSALKSRLTIIKDNSKSQVFLKMNSLQTDDTAIYYCAKHYYYGGSYAMDYWGQGTSVTVSSAAATTTPAPRPPTPAPTIASQPLSLRPEACRPAAGGAVHTRGLDFACDIYIWAPLAGTCGVLLLSLVITLYCKRGRKKLLYIFKQPFMRPVQTTQEEDGCSCRFPEEEEGGCELRVKFSRSADAPAYQQGQNQLYNELNLGRREEYDVLDKRRGRDPEMGGKPRRKNPQEGLYNELQKDKMAEAYSEIGMKGERRRGKGHDGLYQGLSTATKDTYDALHMQALPPR

SEQ ID NO: 99 - DNA, 797 bp, synthetic construct
  misc_feature 1..797: note = source = /note="Description of Artificial Sequence: Synthetic polynucleotide"
  source 1..797: mol_type = other DNA
atggcactgcccgtgaccgccctgcttctgccgcttgcacttctgctgcacgccgctaggccccaagtcaccctcaaagagtcagggccaggaatcctcaagccctcacagactctgtctcttacttgctcattcagcggattcagcctttccacctctggtatgggcgtggggtggattaggcaacctagcggaaaggggcttgaatggctggcccacatctggtgggacgacgacaagtactacaacccctcactgaagtcccagctcactatttccaaagatacttcccggaatcaggtgttcctcaagattacctctgtcgacaccgctgataccgccacttactattgttcacgcagaccgagaggtaccatggacgcaatggactactggggacagggcaccagcgtgaccgtgtcatctggcggtggagggtcaggaggtggaggtagcggaggcggtgggtccgacattgtcatgacccaggccgccagcagcctgagcgcttcactgggcgacagggtgaccatcagctgtcgcgcatcacaagatatctctaagtatcttaattggtaccagcaaaagccggatggaaccgtgaagctgctgatctactacacctcacggctgcattctggagtgcctagccgctttagcggatctgggtccggtactgactacagcctcaccattagaaaccttgaacaggaggacatcgcaacttatttctgccaacaggtctatactctgccgtggaccttcggcggaggtaccaaactggagattaagtccgg

SEQ ID NO: 100 - protein, 265 aa, synthetic construct
  REGION 1..265: note = source = /note="Description of Artificial Sequence: Synthetic polypeptide"
MALPVTALLLPLALLLHAARPQVTLKESGPGILKPSQTLSLTCSFSGFSLSTSGMGVGWIRQPSGKGLEWLAHIWWDDDKYYNPSLKSQLTISKDTSRNQVFLKITSVDTADTATYYCSRRPRGTMDAMDYWGQGTSVTVSSGGGGSGGGGSGGGGSDIVMTQAASSLSASLGDRVTISCRASQDISKYLNWYQQKPDGTVKLLIYYTSRLHSGVPSRFSGSGSGTDYSLTIRNLEQEDIATYFCQQVYTLPWTFGGGTKLEIKS

SEQ ID NO: 101 - DNA, 1170 bp, synthetic construct
  misc_feature 1..1170: note = source = /note="Description of Artificial Sequence: Synthetic polynucleotide"
  source 1..1170: mol_type = other DNA
atggcactgcccgtgaccgccctgcttctgccgcttgcacttctgctgcacgccgctaggccccaagtcaccctcaaagagtcagggccaggaatcctcaagccctcacagactctgtctcttacttgctcattcagcggattcagcctttccacctctggtatgggcgtggggtggattaggcaacctagcggaaaggggcttgaatggctggcccacatctggtgggacgacgacaagtactacaacccctcactgaagtcccagctcactatttccaaagatacttcccggaatcaggtgttcctcaagattacctctgtcgacaccgctgataccgccacttactattgttcacgcagaccgagaggtaccatggacgcaatggactactggggacagggcaccagcgtgaccgtgtcatctggcggtggagggtcaggaggtggaggtagcggaggcggtgggtccgacattgtcatgacccaggccgccagcagcctgagcgcttcactgggcgacagggtgaccatcagctgtcgcgcatcacaagatatctctaagtatcttaattggtaccagcaaaagccggatggaaccgtgaagctgctgatctactacacctcacggctgcattctggagtgcctagccgctttagcggcacttgcggcgtgctcctgctgtcgctggtcatcaccctttactgcaagaggggccggaagaagctgctttacatcttcaagcagccgttcatgcggcccgtgcagacgactcaggaagaggacggatgctcgtgcagattccctgaggaggaagaggggggatgcgaactgcgcgtcaagttctcacggtccgccgacgcccccgcatatcaacagggccagaatcagctctacaacgagctgaacctgggaaggagagaggagtacgacgtgctggacaagcgacgcggacgcgacccggagatgggggggaaaccacggcggaaaaaccctcaggaaggactgtacaacgaactccagaaagacaagatggcggaagcctactcagaaatcgggatgaagggagagcggaggaggggaaagggtcacgacgggctgtaccagggactgagcaccgccactaaggatacctacgatgccttgcatatgcaagcactcccaccccgg

SEQ ID NO: 102 - protein, 490 aa, synthetic construct
  REGION 1..490: note = source = /note="Description of Artificial Sequence: Synthetic polypeptide"
MALPVTALLLPLALLLHAARPQVTLKESGPGILKPSQTLSLTCSFSGFSLSTSGMGVGWIRQPSGKGLEWLAHIWWDDDKYYNPSLKSQLTISKDTSRNQVFLKITSVDTADTATYYCSRRPRGTMDAMDYWGQGTSVTVSSGGGGSGGGGSGGGGSDIVMTQAASSLSASLGDRVTISCRASQDISKYLNWYQQKPDGTVKLLIYYTSRLHSGVPSRFSGSGSGTDYSLTIRNLEQEDIATYFCQQVYTLPWTFGGGTKLEIKAAATTTPAPRPPTPAPTIASQPLSLRPEACRPAAGGAVHTRGLDFACDIYIWAPLAGTCGVLLLSLVITLYCKRGRKKLLYIFKQPFMRPVQTTQEEDGCSCRFPEEEEGGCELRVKFSRSADAPAYQQGQNQLYNELNLGRREEYDVLDKRRGRDPEMGGKPRRKNPQEGLYNELQKDKMAEAYSEIGMKGERRRGKGHDGLYQGLSTATKDTYDALHMQALPPR

SEQ ID NO: 103 - DNA, 2366 bp, synthetic construct
  misc_feature 1..2366: note = source = /note="Description of Artificial Sequence: Synthetic polynucleotide"
  source 1..2366: mol_type = other DNA
tgagctctgagtcagtgactcagtgagtcagtgactcagtgagtcagtgactcagctcgaggatctcgctagcgggaatttccggggactttccgggaatttccggggactttccgggaatttccagatctggcctcggcggccaagcttagacactagagggtatataatggaagctcgacttccagcttggcaatccggtactgttggtaaaggcgcgccccaccatgctgctgctggtcaccagcctgctgctgtgcgagctccctcaccccgcctttctgcttatcccggacattcagatgacacagaccacctcgagcttgtccgcgtcgctgggcgatcgcgtgaccatctcctgccgggcctcccaagacatttcaaagtatctcaactggtaccagcagaagccggacggaaccgtgaaactgctgatctaccataccagccgcctgcactccggcgtgccgtcccgcttctccggatcgggttccggaactgactactcactgactatctccaacttggaacaagaggacatcgccacttacttctgtcaacaaggaaatacccttccctacaccttcggggggggtaccaagctggagatcactgggggcggaggctccggtggaggcggatccggcggtggagggagcgaagtcaagctgcaggaatcaggaccaggactcgtggcgccatcccagtccctgtcggtgacctgtactgtctccggagtcagcctccccgattacggagtgtcatggattaggcaacccccaagaaaagggctggaatggctcggagtgatctggggctccgaaaccacctactacaactcggcgctgaagtcccggctgaccatcatcaaggacaactccaagagccaagtgttcttgaagatgaacagcttgcagaccgacgataccgcaatctactactgtgccaagcactattactacggggggtcttacgccatggactactggggacagggcacctccgtgactgtgtcgtccgcggccgctaccacaacccctgcgccccggcctcctacccccgcacccacgattgcttctcaacctctttcactccgacctgaggcttgtagacctgcagccgggggtgccgtccacacacggggactcgacttcgcttgtgatatatatatttgggcgcccctggccggcacttgtggagttcttttgctctctcttgttatcacattgtactgcaagcgaggtaggaagaaattgctttacatttttaagcagccgttcatgcgaccagtacagactactcaagaagaagatgggtgctcttgtcggttcccggaagaagaagagggtggttgcgagttgagggtgaagttctcccgctctgccgacgcaccggcatatcagcagggacaaaaccagctctacaacgaattgaacctgggtcggcgggaagaatatgacgtgctcgataagcggcggggtcgcgacccagaaatgggaggcaaaccgcgcaggaaaaatccacaggagggactttataacgaacttcaaaaggataagatggcagaggcatacagcgaaatcgggatgaaaggcgagagaagaagggggaaagggcacgatggtctttaccaggggctttctaccgcgacgaaggatacctacgatgctctccatatgcaagcacttcctcctagacgggcaaagcggggctcaggggcgactaacttttcactgttgaagcaggccggggatgtggaggagaatcctggtcctagagctaagcgagtagacatgggaagagggctgctccgaggcttgtggccgttgcatattgtattgtggacgcggatagcgagtacaatcccgcctcacgtgcaaaaatcagttaataacgacatgatcgttactgacaacaatggcgcagttaaatttccgcagctttgtaaattctgtgatgtaagattttcaacgtgcgataaccagaaaagctgtatgtccaactgcagcatcacatcaatctgtgaaaaaccccaagaggtatgtgtggccgtctggcgaaagaatgacgaaaatatcacactggagaccgtttgtcacgatcctaaactcccttatcatgactttattctggaagacgcagcgtcaccgaagtgtataatgaaagagaagaagaagcctggagagacgtttttcatgtgcagttgctcctcagatgagtgtaatgacaacatcattttttccgaggagtacaatacgagtaacccagacctcctgctggttattttccaggtaaccggcatcagtttgttgcccccactgggtgttgcaatcagtgtaataatcatattttattgttaccgggtg

SEQ ID NO: 104 - protein, 713 aa, synthetic construct
  REGION 1..713: note = source = /note="Description of Artificial Sequence: Synthetic polypeptide"
MLLLVTSLLLCELPHPAFLLIPDIQMTQTTSSLSASLGDRVTISCRASQDISKYLNWYQQKPDGTVKLLIYHTSRLHSGVPSRFSGSGSGTDYSLTISNLEQEDIATYFCQQGNTLPYTFGGGTKLEITGGGGSGGGGSGGGGSEVKLQESGPGLVAPSQSLSVTCTVSGVSLPDYGVSWIRQPPRKGLEWLGVIWGSETTYYNSALKSRLTIIKDNSKSQVFLKMNSLQTDDTAIYYCAKHYYYGGSYAMDYWGQGTSVTVSSAAATTTPAPRPPTPAPTIASQPLSLRPEACRPAAGGAVHTRGLDFACDIYIWAPLAGTCGVLLLSLVITLYCKRGRKKLLYIFKQPFMRPVQTTQEEDGCSCRFPEEEEGGCELRVKFSRSADAPAYQQGQNQLYNELNLGRREEYDVLDKRRGRDPEMGGKPRRKNPQEGLYNELQKDKMAEAYSEIGMKGERRRGKGHDGLYQGLSTATKDTYDALHMQALPPRRAKRGSGATNFSLLKQAGDVEENPGPRAKRVDMGRGLLRGLWPLHIVLWTRIASTIPPHVQKSVNNDMIVTDNNGAVKFPQLCKFCDVRFSTCDNQKSCMSNCSITSICEKPQEVCVAVWRKNDENITLETVCHDPKLPYHDFILEDAASPKCIMKEKKKPGETFFMCSCSSDECNDNIIFSEEYNTSNPDLLLVIFQVTGISLLPPLGVAISVIIIFYCYRV

SEQ ID NO: 105 - DNA, 2390 bp, synthetic construct
  misc_feature 1..2390: note = source = /note="Description of Artificial Sequence: Synthetic polynucleotide"
  source 1..2390: mol_type = other DNA
tgagctctgagtcagtgactcagtgagtcagtgactcagtgagtcagtgactcagctcgaggatctcgctagcgggaatttccggggactttccgggaatttccggggactttccgggaatttccagatctggcctcggcggccaagcttagacactagagggtatataatggaagctcgacttccagcttggcaatccggtactgttggtaaaggcgcgccccaccatgctgctgctggtcaccagcctgctgctgtgcgagctccctcaccccgcctttctgcttatcccggacattcagatgacacagaccacctcgagcttgtccgcgtcgctgggcgatcgcgtgaccatctcctgccgggcctcccaagacatttcaaagtatctcaactggtaccagcagaagccggacggaaccgtgaaactgctgatctaccataccagccgcctgcactccggcgtgccgtcccgcttctccggatcgggttccggaactgactactcactgactatctccaacttggaacaagaggacatcgccacttacttctgtcaacaaggaaatacccttccctacaccttcggggggggtaccaagctggagatcactgggggcggaggctccggtggaggcggatccggcggtggagggagcgaagtcaagctgcaggaatcaggaccaggactcgtggcgccatcccagtccctgtcggtgacctgtactgtctccggagtcagcctccccgattacggagtgtcatggattaggcaacccccaagaaaagggctggaatggctcggagtgatctggggctccgaaaccacctactacaactcggcgctgaagtcccggctgaccatcatcaaggacaactccaagagccaagtgttcttgaagatgaacagcttgcagaccgacgataccgcaatctactactgtgccaagcactattactacggggggtcttacgccatggactactggggacagggcacctccgtgactgtgtcgtccgcggccgctaccacaacccctgcgccccggcctcctacccccgcacccacgattgcttctcaacctctttcactccgacctgaggcttgtagacctgcagccgggggtgccgtccacacacggggactcgacttcgcttgtgatatatatatttgggcgcccctggccggcacttgtggagttcttttgctctctcttgttatcacattgtactgcaagcgaggtaggaagaaattgctttacatttttaagcagccgttcatgcgaccagtacagactactcaagaagaagatgggtgctcttgtcggttcccggaagaagaagagggtggttgcgagttgagggtgaagttctcccgctctgccgacgcaccggcatatcagcagggacaaaaccagctctacaacgaattgaacctgggtcggcgggaagaatatgacgtgctcgataagcggcggggtcgcgacccagaaatgggaggcaaaccgcgcaggaaaaatccacaggagggactttataacgaacttcaaaaggataagatggcagaggcatacagcgaaatcgggatgaaaggcgagagaagaagggggaaagggcacgatggtctttaccaggggctttctaccgcgacgaaggatacctacgatgctctccatatgcaagcacttcctcctagacgggcaaagcggggctcaggggcgactaacttttcactgttgaagcaggccggggatgtggaggagaatcctggtcctagagctaagcgagtagacatgcaaataccacaagcgccgtggcccgtcgtctgggctgttcttcagcttggctggagacctggctggtttctcgattctccagataggccctggaacccaccgacgttcagtccggcacttctcgtggtcacagagggggacaacgccacttttacgtgctcctttagcaacacctccgagtccttcgtactgaattggtatcgcatgagtccgtccaatcagacggacaagttggccgcgtttcctgaagataggtcacaacctggccaagactgtcggttccgggtcacccagttgccgaatgggagggactttcatatgagcgtcgttcgggcaagaaggaacgattctggaacgtatttgtgcggggccattagccttgcgccaaaagcgcagataaaggagtcccttcgggcagaacttcgcgtgacagagcgacgcgctgaagttccgactgcccatccctctccgagcccacgaccagccggacaatttcagactcttgtggtgggtgtggtaggcggcctgctcggaagcttggtcttgctggtgtgggtcctggctgtgatttgcagtcgagcagcccgcggcacc

SEQ ID NO: 106 - protein, 721 aa, synthetic construct
  REGION 1..721: note = source = /note="Description of Artificial Sequence: Synthetic polypeptide"
MLLLVTSLLLCELPHPAFLLIPDIQMTQTTSSLSASLGDRVTISCRASQDISKYLNWYQQKPDGTVKLLIYHTSRLHSGVPSRFSGSGSGTDYSLTISNLEQEDIATYFCQQGNTLPYTFGGGTKLEITGGGGSGGGGSGGGGSEVKLQESGPGLVAPSQSLSVTCTVSGVSLPDYGVSWIRQPPRKGLEWLGVIWGSETTYYNSALKSRLTIIKDNSKSQVFLKMNSLQTDDTAIYYCAKHYYYGGSYAMDYWGQGTSVTVSSAAATTTPAPRPPTPAPTIASQPLSLRPEACRPAAGGAVHTRGLDFACDIYIWAPLAGTCGVLLLSLVITLYCKRGRKKLLYIFKQPFMRPVQTTQEEDGCSCRFPEEEEGGCELRVKFSRSADAPAYQQGQNQLYNELNLGRREEYDVLDKRRGRDPEMGGKPRRKNPQEGLYNELQKDKMAEAYSEIGMKGERRRGKGHDGLYQGLSTATKDTYDALHMQALPPRRAKRGSGATNFSLLKQAGDVEENPGPRAKRVDMQIPQAPWPVVWAVLQLGWRPGWFLDSPDRPWNPPTFSPALLVVTEGDNATFTCSFSNTSESFVLNWYRMSPSNQTDKLAAFPEDRSQPGQDCRFRVTQLPNGRDFHMSVVRARRNDSGTYLCGAISLAPKAQIKESLRAELRVTERRAEVPTAHPSPSPRPAGQFQTLVVGVVGGLLGSLVLLVWVLAVICSRAARGT

SEQ ID NO: 107 - DNA, 3050 bp, synthetic construct
  misc_feature 1..3050: note = source = /note="Description of Artificial Sequence: Synthetic polynucleotide"
  source 1..3050: mol_type = other DNA
tgagctctgagtcagtgactcagtgagtcagtgactcagtgagtcagtgactcagctcgaggatctcgctagcgggaatttccggggactttccgggaatttccggggactttccgggaatttccagatctggcctcggcggccaagcttagacactagagggtatataatggaagctcgacttccagcttggcaatccggtactgttggtaaaggcgcgccccaccatgctgctgctggtcaccagcctgctgctgtgcgagctccctcaccccgcctttctgcttatcccggacattcagatgacacagaccacctcgagcttgtccgcgtcgctgggcgatcgcgtgaccatctcctgccgggcctcccaagacatttcaaagtatctcaactggtaccagcagaagccggacggaaccgtgaaactgctgatctaccataccagccgcctgcactccggcgtgccgtcccgcttctccggatcgggttccggaactgactactcactgactatctccaacttggaacaagaggacatcgccacttacttctgtcaacaaggaaatacccttccctacaccttcggggggggtaccaagctggagatcactgggggcggaggctccggtggaggcggatccggcggtggagggagcgaagtcaagctgcaggaatcaggaccaggactcgtggcgccatcccagtccctgtcggtgacctgtactgtctccggagtcagcctccccgattacggagtgtcatggattaggcaacccccaagaaaagggctggaatggctcggagtgatctggggctccgaaaccacctactacaactcggcgctgaagtcccggctgaccatcatcaaggacaactccaagagccaagtgttcttgaagatgaacagcttgcagaccgacgataccgcaatctactactgtgccaagcactattactacggggggtcttacgccatggactactggggacagggcacctccgtgactgtgtcgtccgcggccgctaccacaacccctgcgccccggcctcctacccccgcacccacgattgcttctcaacctctttcactccgacctgaggcttgtagacctgcagccgggggtgccgtccacacacggggactcgacttcgcttgtgatatatatatttgggcgcccctggccggcacttgtggagttcttttgctctctcttgttatcacattgtactgcaagcgaggtaggaagaaattgctttacatttttaagcagccgttcatgcgaccagtacagactactcaagaagaagatgggtgctcttgtcggttcccggaagaagaagagggtggttgcgagttgagggtgaagttctcccgctctgccgacgcaccggcatatcagcagggacaaaaccagctctacaacgaattgaacctgggtcggcgggaagaatatgacgtgctcgataagcggcggggtcgcgacccagaaatgggaggcaaaccgcgcaggaaaaatccacaggagggactttataacgaacttcaaaaggataagatggcagaggcatacagcgaaatcgggatgaaaggcgagagaagaagggggaaagggcacgatggtctttaccaggggctttctaccgcgacgaaggatacctacgatgctctccatatgcaagcacttcctcctagacgggcaaagcggggctcaggggcgactaacttttcactgttgaagcaggccggggatgtggaggagaatcctggtcctagagctaagcgagtagacatgcaaataccacaagcgccgtggcccgtcgtctgggctgttcttcagcttggctggagacctggctggtttctcgattctccagataggccctggaacccaccgacgttcagtccggcacttctcgtggtcacagagggggacaacgccacttttacgtgctcctttagcaacacctccgagtccttcgtactgaattggtatcgcatgagtccgtccaatcagacggacaagttggccgcgtttcctgaagataggtcacaacctggccaagactgtcggttccgggtcacccagttgccgaatgggagggactttcatatgagcgtcgttcgggcaagaaggaacgattctggaacgtatttgtgcggggccattagccttgcgccaaaagcgcagataaaggagtcccttcgggcagaacttcgcgtgacagagcgacgcgctgaagttccgactgcccatccctctccgagcccacgaccagccggacaatttcagactcttgtggtgggtgtggtaggcggcctgctcggaagcttggtcttgctggtgtgggtcctggctgtgatttgcagtcgagcagcccgcggcacccgggctaaacggagcggctccggggcaaccaactttagtctgctgaaacaggcaggagatgtggaggaaaacccaggaccagctagcatgggaagagggctgctccgaggcttgtggccgttgcatattgtattgtggacgcggatagcgagtacaatcccgcctcacgtgcaaaaatcagttaataacgacatgatcgttactgacaacaatggcgcagttaaatttccgcagctttgtaaattctgtgatgtaagattttcaacgtgcgataaccagaaaagctgtatgtccaactgcagcatcacatcaatctgtgaaaaaccccaagaggtatgtgtggccgtctggcgaaagaatgacgaaaatatcacactggagaccgtttgtcacgatcctaaactcccttatcatgactttattctggaagacgcagcgtcaccgaagtgtataatgaaagagaagaagaagcctggagagacgtttttcatgtgcagttgctcctcagatgagtgtaatgacaacatcattttttccgaggagtacaatacgagtaacccagacctcctgctggttattttccaggtaaccggcatcagtttgttgcccccactgggtgttgcaatcagtgtaataatcatattttattgttaccgggtg

SEQ ID NO: 108 - protein, 941 aa, synthetic construct
  REGION 1..941: note = source = /note="Description of Artificial Sequence: Synthetic polypeptide"
MLLLVTSLLLCELPHPAFLLIPDIQMTQTTSSLSASLGDRVTISCRASQDISKYLNWYQQKPDGTVKLLIYHTSRLHSGVPSRFSGSGSGTDYSLTISNLEQEDIATYFCQQGNTLPYTFGGGTKLEITGGGGSGGGGSGGGGSEVKLQESGPGLVAPSQSLSVTCTVSGVSLPDYGVSWIRQPPRKGLEWLGVIWGSETTYYNSALKSRLTIIKDNSKSQVFLKMNSLQTDDTAIYYCAKHYYYGGSYAMDYWGQGTSVTVSSAAATTTPAPRPPTPAPTIASQPLSLRPEACRPAAGGAVHTRGLDFACDIYIWAPLAGTCGVLLLSLVITLYCKRGRKKLLYIFKQPFMRPVQTTQEEDGCSCRFPEEEEGGCELRVKFSRSADAPAYQQGQNQLYNELNLGRREEYDVLDKRRGRDPEMGGKPRRKNPQEGLYNELQKDKMAEAYSEIGMKGERRRGKGHDGLYQGLSTATKDTYDALHMQALPPRRAKRGSGATNFSLLKQAGDVEENPGPRAKRVDMQIPQAPWPVVWAVLQLGWRPGWFLDSPDRPWNPPTFSPALLVVTEGDNATFTCSFSNTSESFVLNWYRMSPSNQTDKLAAFPEDRSQPGQDCRFRVTQLPNGRDFHMSVVRARRNDSGTYLCGAISLAPKAQIKESLRAELRVTERRAEVPTAHPSPSPRPAGQFQTLVVGVVGGLLGSLVLLVWVLAVICSRAARGTRAKRSGSGATNFSLLKQAGDVEENPGPASMGRGLLRGLWPLHIVLWTRIASTIPPHVQKSVNNDMIVTDNNGAVKFPQLCKFCDVRFSTCDNQKSCMSNCSITSICEKPQEVCVAVWRKNDENITLETVCHDPKLPYHDFILEDAASPKCIMKEKKKPGETFFMCSCSSDECNDNIIFSEEYNTSNPDLLLVIFQVTGISLLPPLGVAISVIIIFYCYRV

SEQ ID NO: 109 - DNA, 2342 bp, synthetic construct
  misc_feature 1..2342: note = source = /note="Description of Artificial Sequence: Synthetic polynucleotide"
  source 1..2342: mol_type = other DNA
ggtacctgagctcagttctgagaaaagtagttctgagaaaagtagttctgagaaaagtagttctgagaaaagtagttctgagaaaagtctcgaggatatcaagatctggcctcggcggccaagcttagacactagagggtatataatggaagctcgacttccagcttggcaatccggtactgttggtaaaggcgcgccccaccatgctgctgctggtcaccagcctgctgctgtgcgagctccctcaccccgcctttctgcttatcccggacattcagatgacacagaccacctcgagcttgtccgcgtcgctgggcgatcgcgtgaccatctcctgccgggcctcccaagacatttcaaagtatctcaactggtaccagcagaagccggacggaaccgtgaaactgctgatctaccataccagccgcctgcactccggcgtgccgtcccgcttctccggatcgggttccggaactgactactcactgactatctccaacttggaacaagaggacatcgccacttacttctgtcaacaaggaaatacccttccctacaccttcggggggggtaccaagctggagatcactgggggcggaggctccggtggaggcggatccggcggtggagggagcgaagtcaagctgcaggaatcaggaccaggactcgtggcgccatcccagtccctgtcggtgacctgtactgtctccggagtcagcctccccgattacggagtgtcatggattaggcaacccccaagaaaagggctggaatggctcggagtgatctggggctccgaaaccacctactacaactcggcgctgaagtcccggctgaccatcatcaaggacaactccaagagccaagtgttcttgaagatgaacagcttgcagaccgacgataccgcaatctactactgtgccaagcactattactacggggggtcttacgccatggactactggggacagggcacctccgtgactgtgtcgtccgcggccgctaccacaacccctgcgccccggcctcctacccccgcacccacgattgcttctcaacctctttcactccgacctgaggcttgtagacctgcagccgggggtgccgtccacacacggggactcgacttcgcttgtgatatatatatttgggcgcccctggccggcacttgtggagttcttttgctctctcttgttatcacattgtactgcaagcgaggtaggaagaaattgctttacatttttaagcagccgttcatgcgaccagtacagactactcaagaagaagatgggtgctcttgtcggttcccggaagaagaagagggtggttgcgagttgagggtgaagttctcccgctctgccgacgcaccggcatatcagcagggacaaaaccagctctacaacgaattgaacctgggtcggcgggaagaatatgacgtgctcgataagcggcggggtcgcgacccagaaatgggaggcaaaccgcgcaggaaaaatccacaggagggactttataacgaacttcaaaaggataagatggcagaggcatacagcgaaatcgggatgaaaggcgagagaagaagggggaaagggcacgatggtctttaccaggggctttctaccgcgacgaaggatacctacgatgctctccatatgcaagcacttcctcctagacgggcaaagcggggctcaggggcgactaacttttcactgttgaagcaggccggggatgtggaggagaatcctggtcctagagctaagcgagtagacatgggaagagggctgctccgaggcttgtggccgttgcatattgtattgtggacgcggatagcgagtacaatcccgcctcacgtgcaaaaatcagttaataacgacatgatcgttactgacaacaatggcgcagttaaatttccgcagctttgtaaattctgtgatgtaagattttcaacgtgcgataaccagaaaagctgtatgtccaactgcagcatcacatcaatctgtgaaaaaccccaagaggtatgtgtggccgtctggcgaaagaatgacgaaaatatcacactggagaccgtttgtcacgatcctaaactcccttatcatgactttattctggaagacgcagcgtcaccgaagtgtataatgaaagagaagaagaagcctggagagacgtttttcatgtgcagttgctcctcagatgagtgtaatgacaacatcattttttccgaggagtacaatacgagtaacccagacctcctgctggttattttccaggtaaccggcatcagtttgttgcccccactgggtgttgcaatcagtgtaataatcatattttattgttaccgggtg

SEQ ID NO: 110 - DNA, 2366 bp, synthetic construct
  misc_feature 1..2366: note = source = /note="Description of Artificial Sequence: Synthetic polynucleotide"
  source 1..2366: mol_type = other DNA
ggtacctgagctcagttctgagaaaagtagttctgagaaaagtagttctgagaaaagtagttctgagaaaagtagttctgagaaaagtctcgaggatatcaagatctggcctcggcggccaagcttagacactagagggtatataatggaagctcgacttccagcttggcaatccggtactgttggtaaaggcgcgccccaccatgctgctgctggtcaccagcctgctgctgtgcgagctccctcaccccgcctttctgcttatcccggacattcagatgacacagaccacctcgagcttgtccgcgtcgctgggcgatcgcgtgaccatctcctgccgggcctcccaagacatttcaaagtatctcaactggtaccagcagaagccggacggaaccgtgaaactgctgatctaccataccagccgcctgcactccggcgtgccgtcccgcttctccggatcgggttccggaactgactactcactgactatctccaacttggaacaagaggacatcgccacttacttctgtcaacaaggaaatacccttccctacaccttcggggggggtaccaagctggagatcactgggggcggaggctccggtggaggcggatccggcggtggagggagcgaagtcaagctgcaggaatcaggaccaggactcgtggcgccatcccagtccctgtcggtgacctgtactgtctccggagtcagcctccccgattacggagtgtcatggattaggcaacccccaagaaaagggctggaatggctcggagtgatctggggctccgaaaccacctactacaactcggcgctgaagtcccggctgaccatcatcaaggacaactccaagagccaagtgttcttgaagatgaacagcttgcagaccgacgataccgcaatctactactgtgccaagcactattactacggggggtcttacgccatggactactggggacagggcacctccgtgactgtgtcgtccgcggccgctaccacaacccctgcgccccggcctcctacccccgcacccacgattgcttctcaacctctttcactccgacctgaggcttgtagacctgcagccgggggtgccgtccacacacggggactcgacttcgcttgtgatatatatatttgggcgcccctggccggcacttgtggagttcttttgctctctcttgttatcacattgtactgcaagcgaggtaggaagaaattgctttacatttttaagcagccgttcatgcgaccagtacagactactcaagaagaagatgggtgctcttgtcggttcccggaagaagaagagggtggttgcgagttgagggtgaagttctcccgctctgccgacgcaccggcatatcagcagggacaaaaccagctctacaacgaattgaacctgggtcggcgggaagaatatgacgtgctcgataagcggcggggtcgcgacccagaaatgggaggcaaaccgcgcaggaaaaatccacaggagggactttataacgaacttcaaaaggataagatggcagaggcatacagcgaaatcgggatgaaaggcgagagaagaagggggaaagggcacgatggtctttaccaggggctttctaccgcgacgaaggatacctacgatgctctccatatgcaagcacttcctcctagacgggcaaagcggggctcaggggcgactaacttttcactgttgaagcaggccggggatgtggaggagaatcctggtcctagagctaagcgagtagacatgcaaataccacaagcgccgtggcccgtcgtctgggctgttcttcagcttggctggagacctggctggtttctcgattctccagataggccctggaacccaccgacgttcagtccggcacttctcgtggtcacagagggggacaacgccacttttacgtgctcctttagcaacacctccgagtccttcgtactgaattggtatcgcatgagtccgtccaatcagacggacaagttggccgcgtttcctgaagataggtcacaacctggccaagactgtcggttccgggtcacccagttgccgaatgggagggactttcatatgagcgtcgttcgggcaagaaggaacgattctggaacgtatttgtgcggggccattagccttgcgccaaaagcgcagataaaggagtcccttcgggcagaacttcgcgtgacagagcgacgcgctgaagttccgactgcccatccctctccgagcccacgaccagccggacaatttcagactcttgtggtgggtgtggtaggcggcctgctcggaagcttggtcttgctggtgtgggtcctggctgtgatttgcagtcgagcagcccgcggcacc

SEQ ID NO: 111 - DNA, 3026 bp, synthetic construct
  misc_feature 1..3026: note = source = /note="Description of Artificial Sequence: Synthetic polynucleotide"
  source 1..3026: mol_type = other DNA
ggtacctgagctcagttctgagaaaagtagttctgagaaaagtagttctgagaaaagtagttctgagaaaagtagttctgagaaaagtctcgaggatatcaagatctggcctcggcggccaagcttagacactagagggtatataatggaagctcgacttccagcttggcaatccggtactgttggtaaaggcgcgccccaccatgctgctgctggtcaccagcctgctgctgtgcgagctccctcaccccgcctttctgcttatcccggacattcagatgacacagaccacctcgagcttgtccgcgtcgctgggcgatcgcgtgaccatctcctgccgggcctcccaagacatttcaaagtatctcaactggtaccagcagaagccggacggaaccgtgaaactgctgatctaccataccagccgcctgcactccggcgtgccgtcccgcttctccggatcgggttccggaactgactactcactgactatctccaacttggaacaagaggacatcgccacttacttctgtcaacaaggaaatacccttccctacaccttcggggggggtaccaagctggagatcactgggggcggaggctccggtggaggcggatccggcggtggagggagcgaagtcaagctgcaggaatcaggaccaggactcgtggcgccatcccagtccctgtcggtgacctgtactgtctccggagtcagcctccccgattacggagtgtcatggattaggcaacccccaagaaaagggctggaatggctcggagtgatctggggctccgaaaccacctactacaactcggcgctgaagtcccggctgaccatcatcaaggacaactccaagagccaagtgttcttgaagatgaacagcttgcagaccgacgataccgcaatctactactgtgccaagcactattactacggggggtcttacgccatggactactggggacagggcacctccgtgactgtgtcgtccgcggccgctaccacaacccctgcgccccggcctcctacccccgcacccacgattgcttctcaacctctttcactccgacctgaggcttgtagacctgcagccgggggtgccgtccacacacggggactcgacttcgcttgtgatatatatatttgggcgcccctggccggcacttgtggagttcttttgctctctcttgttatcacattgtactgcaagcgaggtaggaagaaattgctttacatttttaagcagccgttcatgcgaccagtacagactactcaagaagaagatgggtgctcttgtcggttcccggaagaagaagagggtggttgcgagttgagggtgaagttctcccgctctgccgacgcaccggcatatcagcagggacaaaaccagctctacaacgaattgaacctgggtcggcgggaagaatatgacgtgctcgataagcggcggggtcgcgacccagaaatgggaggcaaaccgcgcaggaaaaatccacaggagggactttataacgaacttcaaaaggataagatggcagaggcatacagcgaaatcgggatgaaaggcgagagaagaagggggaaagggcacgatggtctttaccaggggctttctaccgcgacgaaggatacctacgatgctctccatatgcaagcacttcctcctagacgggcaaagcggggctcaggggcgactaacttttcactgttgaagcaggccggggatgtggaggagaatcctggtcctagagctaagcgagtagacatgcaaataccacaagcgccgtggcccgtcgtctgggctgttcttcagcttggctggagacctggctggtttctcgattctccagataggccctggaacccaccgacgttcagtccggcacttctcgtggtcacagagggggacaacgccacttttacgtgctcctttagcaacacctccgagtccttcgtactgaattggtatcgcatgagtccgtccaatcagacggacaagttggccgcgtttcctgaagataggtcacaacctggccaagactgtcggttccgggtcacccagttgccgaatgggagggactttcatatgagcgtcgttcgggcaagaaggaacgattctggaacgtatttgtgcggggccattagccttgcgccaaaagcgcagataaaggagtcccttcgggcagaacttcgcgtgacagagcgacgcgctgaagttccgactgcccatccctctccgagcccacgaccagccggacaatttcagactcttgtggtgggtgtggtaggcggcctgctcggaagcttggtcttgctggtgtgggtcctggctgtgatttgcagtcgagcagcccgcggcacccgggctaaacggagcggctccggggcaaccaactttagtctgctgaaacaggcaggagatgtggaggaaaacccaggaccagctagcatgggaagagggctgctccgaggcttgtggccgttgcatattgtattgtggacgcggatagcgagtacaatcccgcctcacgtgcaaaaatcagttaataacgacatgatcgttactgacaacaatggcgcagttaaatttccgcagctttgtaaattctgtgatgtaagattttcaacgtgcgataaccagaaaagctgtatgtccaactgcagcatcacatcaatctgtgaaaaaccccaagaggtatgtgtggccgtctggcgaaagaatgacgaaaatatcacactggagaccgtttgtcacgatcctaaactcccttatcatgactttattctggaagacgcagcgtcaccgaagtgtataatgaaagagaagaagaagcctggagagacgtttttcatgtgcagttgctcctcagatgagtgtaatgacaacatcattttttccgaggagtacaatacgagtaacccagacctcctgctggttattttccaggtaaccggcatcagtttgttgcccccactgggtgttgcaatcagtgtaataatcatattttattgttaccgggtg

SEQ ID NO: 112 - protein, 245 aa, synthetic construct
  REGION 1..245: note = source = /note="Description of Artificial Sequence: Synthetic polypeptide"
DIQMTQTTSSLSASLGDRVTISCRASQDISKYLNWYQQKPDGTVKLLIYHTSRLHSGVPSRFSGSGSGTDYSLTISNLEQEDIATYFCQQGNTLPYTFGGGTKLEITGSTSGSGKPGSGEGSTKGEVKLQESGPGLVAPSQSLSVTCTVSGVSLPDYGVSWIRQPPRKGLEWLGVIWGSETTYYNSALKSRLTIIKDNSKSQVFLKMNSLQTDDTAIYYCAKHYYYGGSYAMDYWGQGTSVTVSS

SEQ ID NO: 113 - DNA, 729 bp, synthetic construct
  misc_feature 1..729: note = source = /note="Description of Artificial Sequence: Synthetic polynucleotide"
  source 1..729: mol_type = other DNA
gaggtgcagttgcaacagtcaggagctgaactggtcaagccaggagccagcgtgaagatgagctgcaaggcctccggttacaccttcacctcctacaacatgcactgggtgaaacagaccccgggacaagggctcgaatggattggcgccatctaccccgggaatggcgatacttcgtacaaccagaagttcaagggaaaggccaccctgaccgccgacaagagctcctccaccgcgtatatgcagttgagctccctgacctccgaggactccgccgactactactgcgcacggtccaactactatggaagctcgtactggttcttcgatgtctggggggccggcaccactgtgaccgtcagctccgggggcggaggatccggtggaggcggaagcgggggtggaggatccgacattgtgctgactcagtccccggcaatcctgtcggcctcaccgggcgaaaaggtcacgatgacttgtagagcgtcgtccagcgtgaactacatggattggtaccaaaagaagcctggatcgtcacccaagccttggatctacgctacatctaacctggcctccggcgtgccagcgcggttcagcgggtccggctcgggcacctcatactcgctgaccatctcccgcgtggaggctgaggacgccgcgacctactactgccagcagtggtccttcaacccgccgacttttggaggcggtactaagctggagatcaaa

SEQ ID NO: 114 - protein, 243 aa, synthetic construct
  REGION 1..243: note = source = /note="Description of Artificial Sequence: Synthetic polypeptide"
EVQLQQSGAELVKPGASVKMSCKASGYTFTSYNMHWVKQTPGQGLEWIGAIYPGNGDTSYNQKFKGKATLTADKSSSTAYMQLSSLTSEDSADYYCARSNYYGSSYWFFDVWGAGTTVTVSSGGGGSGGGGSGGGGSDIVLTQSPAILSASPGEKVTMTCRASSSVNYMDWYQKKPGSSPKPWIYATSNLASGVPARFSGSGSGTSYSLTISRVEAEDAATYYCQQWSFNPPTFGGGTKLEIK

SEQ ID NO: 115 - DNA, 1491 bp, synthetic construct
  misc_feature 1..1491: note = source = /note="Description of Artificial Sequence: Synthetic polynucleotide"
  source 1..1491: mol_type = other DNA
atgctgctgctggtgaccagcctgctgctgtgcgaactgccgcatccggcgtttctgctgattccgcaagtgcaactcgtccaatccggtgccgaagtcaagaagcctggttcctccgtgaaagtgtcgtgcaaagccagcggcgggacttttagctcctacgcgatcagctgggtcagacaggcccctggacaaggcctcgagtggatgggcggcatcattccgattttcggtaccgccaactacgcccagaagttccagggacgcgtgaccattactaccgacgagagcacctcaaccgcatacatggaactgtccagcctgcgctccgaggacacggctgtgtactattgcgccagacggggatggggaggattctcctccggctccgcattcgacatctggggacagggcactatggtcactgtgtcatccgggggaggaggatcaggcggtggaggatccggtggtggcggatccaacttcatgctgacccagccccactcagtgtcggaatcgcccggcaacaccgtgactatcagctgcaccggatccagcgggaccatcggctctaatttcgtgcagtggtaccagcagtccccagggagagctccgaccctgttgatctacgaggacacaaagcggccaagcggagtgccgcctagattcgccggctccgtggattcctcgtccaactcggcgtcgctgaccatcagcggactcaagactgaagatgaagccgactactactgtcagtcctacgactcgagcaactgggtgtttgggggcgggactaagctgaccgtgcttggagcggccgcaactaccacccctgcccctcggccgccgactccggccccaaccatcgcaagccaacccctctccttgcgccccgaagcttgccgcccggccgcgggtggagccgtgcatacccgggggctggactttgcctgcgatatctacatttgggccccgctggccggcacttgcggcgtgctcctgctgtcgctggtcatcaccctttactgcaagaggggccggaagaagctgctttacatcttcaagcagccgttcatgcggcccgtgcagacgactcaggaagaggacggatgctcgtgcagattccctgaggaggaagaggggggatgcgaactgcgcgtcaagttctcacggtccgccgacgcccccgcatatcaacagggccagaatcagctctacaacgagctgaacctgggaaggagagaggagtacgacgtgctggacaagcgacgcggacgcgacccggagatgggggggaaaccacggcggaaaaaccctcaggaaggactgtacaacgaactccagaaagacaagatggcggaagcctactcagaaatcgggatgaagggagagcggaggaggggaaagggtcacgacgggctgtaccagggactgagcaccgccactaaggatacctacgatgccttgcatatgcaagcactcccaccccgg

SEQ ID NO: 116 - protein, 497 aa, synthetic construct
  REGION 1..497: note = source = /note="Description of Artificial Sequence: Synthetic polypeptide"
MLLLVTSLLLCELPHPAFLLIPQVQLVQSGAEVKKPGSSVKVSCKASGGTFSSYAISWVRQAPGQGLEWMGGIIPIFGTANYAQKFQGRVTITTDESTSTAYMELSSLRSEDTAVYYCARRGWGGFSSGSAFDIWGQGTMVTVSSGGGGSGGGGSGGGGSNFMLTQPHSVSESPGNTVTISCTGSSGTIGSNFVQWYQQSPGRAPTLLIYEDTKRPSGVPPRFAGSVDSSSNSASLTISGLKTEDEADYYCQSYDSSNWVFGGGTKLTVLGAAATTTPAPRPPTPAPTIASQPLSLRPEACRPAAGGAVHTRGLDFACDIYIWAPLAGTCGVLLLSLVITLYCKRGRKKLLYIFKQPFMRPVQTTQEEDGCSCRFPEEEEGGCELRVKFSRSADAPAYQQGQNQLYNELNLGRREEYDVLDKRRGRDPEMGGKPRRKNPQEGLYNELQKDKMAEAYSEIGMKGERRRGKGHDGLYQGLSTATKDTYDALHMQALPPR

SEQ ID NO: 117 - DNA, 1479 bp, synthetic construct
  misc_feature 1..1479: note = source = /note="Description of Artificial Sequence: Synthetic polynucleotide"
  source 1..1479: mol_type = other DNA
atgctgctgctggtgaccagcctgctgctgtgcgaactgccgcatccggcgtttctgctgattccggaagtccaattggtgcagagcggatccgaacttaagaaacctggcgcgagcgtgaaagtgtcctgcaaggcctccggagggactttctcgtcgtacgccattagctgggtccgccaagctcctggccaaggcctggagtggatgggcgggattatccccatcttcgggactgcgaactacgcccagaagtttcagggccgggtcactatcaccgccgacgaatcaacctcgaccgcctacatggaactgtcctcgcttcggtccgaggatactgccgtgtactattgtgcctcaacggccagacgcggatgggacaccgctggtccgctcgattactggggccagggaaccctcgtgaccgtcagctccggaggaggaggctccggtggtggaggatccgggggtggtggatccgacatccaaatgacccagtccccctcgtccctgagcgcctctgtgggcgacagagtgacaattgcatgcagggcctcacagactatctcccgctacctgaactggtaccagcagaagccaggaaaggcccctaagctgctcatctacgctgcgtcctcgctccaatccggggtgtcctcacggttttccggatcgggttccggcaccgagttcaccctgaccatcagcagcctgcagcccgaggacttcgcaacctacttctgccagcaaacctactccccgccgattacgttcggacaggggactcggctggaaatcaaggcggccgcaactaccacccctgcccctcggccgccgactccggccccaaccatcgcaagccaacccctctccttgcgccccgaagcttgccgcccggccgcgggtggagccgtgcatacccgggggctggactttgcctgcgatatctacatttgggccccgctggccggcacttgcggcgtgctcctgctgtcgctggtcatcaccctttactgcaagaggggccggaagaagctgctttacatcttcaagcagccgttcatgcggcccgtgcagacgactcaggaagaggacggatgctcgtgcagattccctgaggaggaagaggggggatgcgaactgcgcgtcaagttctcacggtccgccgacgcccccgcatatcaacagggccagaatcagctctacaacgagctgaacctgggaaggagagaggagtacgacgtgctggacaagcgacgcggacgcgacccggagatgggggggaaaccacggcggaaaaaccctcaggaaggactgtacaacgaactccagaaagacaagatggcggaagcctactcagaaatcgggatgaagggagagcggaggaggggaaagggtcacgacgggctgtaccagggactgagcaccgccactaaggatacctacgatgccttgcatatgcaagcactcccaccccgg

SEQ ID NO: 118 - protein, 493 aa, synthetic construct
  REGION 1..493: note = source = /note="Description of Artificial Sequence: Synthetic polypeptide"
MLLLVTSLLLCELPHPAFLLIPEVQLVQSGSELKKPGASVKVSCKASGGTFSSYAISWVRQAPGQGLEWMGGIIPIFGTANYAQKFQGRVTITADESTSTAYMELSSLRSEDTAVYYCASTARRGWDTAGPLDYWGQGTLVTVSSGGGGSGGGGSGGGGSDIQMTQSPSSLSASVGDRVTIACRASQTISRYLNWYQQKPGKAPKLLIYAASSLQSGVSSRFSGSGSGTEFTLTISSLQPEDFATYFCQQTYSPPITFGQGTRLEIKAAATTTPAPRPPTPAPTIASQPLSLRPEACRPAAGGAVHTRGLDFACDIYIWAPLAGTCGVLLLSLVITLYCKRGRKKLLYIFKQPFMRPVQTTQEEDGCSCRFPEEEEGGCELRVKFSRSADAPAYQQGQNQLYNELNLGRREEYDVLDKRRGRDPEMGGKPRRKNPQEGLYNELQKDKMAEAYSEIGMKGERRRGKGHDGLYQGLSTATKDTYDALHMQALPPR

SEQ ID NO: 119 - DNA, 1473 bp, synthetic construct
  misc_feature 1..1473: note = source = /note="Description of Artificial Sequence: Synthetic polynucleotide"
  source 1..1473: mol_type = other DNA
atgctgctgctggtgaccagcctgctgctgtgcgaactgccgcatccggcgtttctgctgattccggaagtgcaactcgtcgaaacaggggcagaagtgaaaaacccaggctcaagcgtgaaagtgtcgtgcaaggcttcgggcggaactctgtccaactacgccatctcctgggtccgccaagctccgggaaagggcctcgagtggatgggcggaatcattcccattttcgggaccgccaactacgcgcaaaagttccagggccgggtcactatcaccgcggacgaaagcaccagcaccgcctacatggaactgtcctccctgcgctccgaggacactgccgtgtactattgcgcccggaggtcatcgtggtaccccgagggctgcttccagcactggggacagggcactctcgtgaccgtgtcgtcgggtggtggtggatcaggagggggaggatccggaggaggcggaagcgatattcagctgacccagtcaccgagctccctgtccgcctccaccggagacagagtgaccatcacgtgtcgggcctcccaagggatctcctcctacctggcctggtaccagcagaagcctggaaaggcaccgaagttgctgatctacgccgcgagcacccttcagtccggagtgcctagccgcttctcgggttccggctctggcactgacttcactctgaccattagctgcctgcagtccgaggattttgccacctactactgccagcagtactatagctaccccctgaccttcgggggcggaaccaagctcgacatcaaggcggccgcaactaccacccctgcccctcggccgccgactccggccccaaccatcgcaagccaacccctctccttgcgccccgaagcttgccgcccggccgcgggtggagccgtgcatacccgggggctggactttgcctgcgatatctacatttgggccccgctggccggcacttgcggcgtgctcctgctgtcgctggtcatcaccctttactgcaagaggggccggaagaagctgctttacatcttcaagcagccgttcatgcggcccgtgcagacgactcaggaagaggacggatgctcgtgcagattccctgaggaggaagaggggggatgcgaactgcgcgtcaagttctcacggtccgccgacgcccccgcatatcaacagggccagaatcagctctacaacgagctgaacctgggaaggagagaggagtacgacgtgctggacaagcgacgcggacgcgacccggagatgggggggaaaccacggcggaaaaaccctcaggaaggactgtacaacgaactccagaaagacaagatggcggaagcctactcagaaatcgggatgaagggagagcggaggaggggaaagggtcacgacgggctgtaccagggactgagcaccgccactaaggatacctacgatgccttgcatatgcaagcactcccaccccgg

SEQ ID NO: 120 - protein, 491 aa, synthetic construct
  REGION 1..491: note = source = /note="Description of Artificial Sequence: Synthetic polypeptide"
MLLLVTSLLLCELPHPAFLLIPEVQLVETGAEVKNPGSSVKVSCKASGGTLSNYAISWVRQAPGKGLEWMGGIIPIFGTANYAQKFQGRVTITADESTSTAYMELSSLRSEDTAVYYCARRSSWYPEGCFQHWGQGTLVTVSSGGGGSGGGGSGGGGSDIQLTQSPSSLSASTGDRVTITCRASQGISSYLAWYQQKPGKAPKLLIYAASTLQSGVPSRFSGSGSGTDFTLTISCLQSEDFATYYCQQYYSYPLTFGGGTKLDIKAAATTTPAPRPPTPAPTIASQPLSLRPEACRPAAGGAVHTRGLDFACDIYIWAPLAGTCGVLLLSLVITLYCKRGRKKLLYIFKQPFMRPVQTTQEEDGCSCRFPEEEEGGCELRVKFSRSADAPAYQQGQNQLYNELNLGRREEYDVLDKRRGRDPEMGGKPRRKNPQEGLYNELQKDKMAEAYSEIGMKGERRRGKGHDGLYQGLSTATKDTYDALHMQALPPR

SEQ ID NO: 121 - DNA, 1476 bp, synthetic construct
  misc_feature 1..1476: note = source = /note="Description of Artificial Sequence: Synthetic polynucleotide"
  source 1..1476: mol_type = other DNA
atgctgctgctggtgaccagcctgctgctgtgcgaactgccgcatccggcgtttctgctgattccggaagtgcaactcgtccaatctggtgccgaagtcaagaagcctggctcaagcgtgaaagtgtcctgcaaagcgtcgggagggaccttcagctcctacgccatttcctgggtccgccaagcaccaggacagggcctggagtggatgggcggcatcatcccgatcttcgggactgccaactacgcccagaagttccaggggagagtgaccattaccgccgacgagtcgaccagcacggcctacatggaactgtccagcctgcgctccgaggacactgccgtgtactactgcgcgagggccagactcggtggagcgttcgacatctggggacagggcaccatggtcaccgtgtcatccggtggcggaggatccggtggtggcggatcaggagggggaggatcccagtccgtgctgactcagcctccctccgtgagcgctgcaccgggacagaaggtcaccatctcatgctcggggggaagctccaacatcgggaaccactacgtgtcctggtaccaacagttgcctggtgccgctccaaagctgctgatctatgacgataacaagcggccgtccggaatccccgaccggttctcggggtctagatccggaaccagcgcaactctcggcattaccggactgcagagcggcgatgaggccgactactactgtggcacatgggactcgtcgctggctgcccacgtgtttggcactggcaccaaggtcaccgtgcttggagcggccgcaactaccacccctgcccctcggccgccgactccggccccaaccatcgcaagccaacccctctccttgcgccccgaagcttgccgcccggccgcgggtggagccgtgcatacccgggggctggactttgcctgcgatatctacatttgggccccgctggccggcacttgcggcgtgctcctgctgtcgctggtcatcaccctttactgcaagaggggccggaagaagctgctttacatcttcaagcagccgttcatgcggcccgtgcagacgactcaggaagaggacggatgctcgtgcagattccctgaggaggaagaggggggatgcgaactgcgcgtcaagttctcacggtccgccgacgcccccgcatatcaacagggccagaatcagctctacaacgagctgaacctgggaaggagagaggagtacgacgtgctggacaagcgacgcggacgcgacccggagatgggggggaaaccacggcggaaaaaccctcaggaaggactgtacaacgaactccagaaagacaagatggcggaagcctactcagaaatcgggatgaagggagagcggaggaggggaaagggtcacgacgggctgtaccagggactgagcaccgccactaaggatacctacgatgccttgcatatgcaagcactcccaccccgg

SEQ ID NO: 122 - protein, 492 aa, synthetic construct
  REGION 1..492: note = source = /note="Description of Artificial Sequence: Synthetic polypeptide"
MLLLVTSLLLCELPHPAFLLIPEVQLVQSGAEVKKPGSSVKVSCKASGGTFSSYAISWVRQAPGQGLEWMGGIIPIFGTANYAQKFQGRVTITADESTSTAYMELSSLRSEDTAVYYCARARLGGAFDIWGQGTMVTVSSGGGGSGGGGSGGGGSQSVLTQPPSVSAAPGQKVTISCSGGSSNIGNHYVSWYQQLPGAAPKLLIYDDNKRPSGIPDRFSGSRSGTSATLGITGLQSGDEADYYCGTWDSSLAAHVFGTGTKVTVLGAAATTTPAPRPPTPAPTIASQPLSLRPEACRPAAGGAVHTRGLDFACDIYIWAPLAGTCGVLLLSLVITLYCKRGRKKLLYIFKQPFMRPVQTTQEEDGCSCRFPEEEEGGCELRVKFSRSADAPAYQQGQNQLYNELNLGRREEYDVLDKRRGRDPEMGGKPRRKNPQEGLYNELQKDKMAEAYSEIGMKGERRRGKGHDGLYQGLSTATKDTYDALHMQALPPR

SEQ ID NO: 123 - DNA, 1491 bp, synthetic construct
  misc_feature 1..1491: note = source = /note="Description of Artificial Sequence: Synthetic polynucleotide"
  source 1..1491: mol_type = other DNA
atgctgctgctggtgaccagcctgctgctgtgcgaactgccgcatccggcgtttctgctgattccggaagtgcaacttgtccagagcggagccgaagtgaagaaacctggatcctccgtcaaagtgtcgtgcaaggcttcgggcggaaccttctcctcgtacgcgatctcatgggtcagacaggcacccggacagggactggagtggatgggcggcatcattcccatcttcggcaccgctaattacgcccagaagtttcaggggagagtgaccatcaccgccgacgagtccacctccactgcctacatggaactgtcctcactgaggtccgaggatactgccgtgtactactgcgcgtcgcaaaaggggggtggatggtccattgacgccttcgatatttggggacaggggacgatggtcacagtgtcatccggcggtggtggatccggtggtggcggatccggaggaggaggcagccagtccgtgctgacccagccgcctagcgtgtcggccgcatctgggcagcgcgtgaccatttcctgttccgggtcctcgtccaacatcggcaacaactacgcctcctggtaccaacagctcccgggaatggcccctaagctgctgatctacgaggacaacaagcggccatccgggatctcagaccggttcagcggatcccagtccggcacttccgcgagcctcgccatcaccggactgcaggctgaggacgaagccgactactactgccaatcatatgacagctcgctcagcggcgatgtggtgttcggcggtggcactaagctgaccgtgttgggagcggccgcaactaccacccctgcccctcggccgccgactccggccccaaccatcgcaagccaacccctctccttgcgccccgaagcttgccgcccggccgcgggtggagccgtgcatacccgggggctggactttgcctgcgatatctacatttgggccccgctggccggcacttgcggcgtgctcctgctgtcgctggtcatcaccctttactgcaagaggggccggaagaagctgctttacatcttcaagcagccgttcatgcggcccgtgcagacgactcaggaagaggacggatgctcgtgcagattccctgaggaggaagaggggggatgcgaactgcgcgtcaagttctcacggtccgccgacgcccccgcatatcaacagggccagaatcagctctacaacgagctgaacctgggaaggagagaggagtacgacgtgctggacaagcgacgcggacgcgacccggagatgggggggaaaccacggcggaaaaaccctcaggaaggactgtacaacgaactccagaaagacaagatggcggaagcctactcagaaatcgggatgaagggagagcggaggaggggaaagggtcacgacgggctgtaccagggactgagcaccgccactaaggatacctacgatgccttgcatatgcaagcactcccaccccgg

SEQ ID NO: 124 - protein, 497 aa, synthetic construct
  REGION 1..497: note = source = /note="Description of Artificial Sequence: Synthetic polypeptide"
MLLLVTSLLLCELPHPAFLLIPEVQLVQSGAEVKKPGSSVKVSCKASGGTFSSYAISWVRQAPGQGLEWMGGIIPIFGTANYAQKFQGRVTITADESTSTAYMELSSLRSEDTAVYYCASQKGGGWSIDAFDIWGQGTMVTVSSGGGGSGGGGSGGGGSQSVLTQPPSVSAASGQRVTISCSGSSSNIGNNYASWYQQLPGMAPKLLIYEDNKRPSGISDRFSGSQSGTSASLAITGLQAEDEADYYCQSYDSSLSGDVVFGGGTKLTVLGAAATTTPAPRPPTPAPTIASQPLSLRPEACRPAAGGAVHTRGLDFACDIYIWAPLAGTCGVLLLSLVITLYCKRGRKKLLYIFKQPFMRPVQTTQEEDGCSCRFPEEEEGGCELRVKFSRSADAPAYQQGQNQLYNELNLGRREEYDVLDKRRGRDPEMGGKPRRKNPQEGLYNELQKDKMAEAYSEIGMKGERRRGKGHDGLYQGLSTATKDTYDALHMQALPPR

SEQ ID NO: 125 - DNA, 1479 bp, synthetic construct
  misc_feature 1..1479: note = source = /note="Description of Artificial Sequence: Synthetic polynucleotide"
  source 1..1479: mol_type = other DNA
atgctgctgctggtgaccagcctgctgctgtgcgaactgccgcatccggcgtttctgctgattccgcaagtccagttgcaacaatggggagcaggccttctgaaaccgtccgagacactgagcctgacgtgcgccgtctatggcggatcgttctccggatactactggtcgtggatcagacagcctccgggaaagggtctggaatggatcggcgaaatcaaccacagcggcagcaccaattacaacccgtcactgaagtcaagggtcaccattagcgtggacacttccaagaaccagttctccctgaaactgtcgagcgtgaccgctgccgatactgccgtgtactactgtgcccgcggccaagtcaagtatagctcaagcctcggctactggggccagggaaccctcgtgaccgtgtcctcgggtggaggaggctccggtggtggaggatccggtggcggaggatcgcagtccgtgctgacccagcctccctccgtgtctgctgcccctgggcaaaaggtcaccatttcgtgctccggctcatcgtccaacatcgggaacaactttgtgtcctggtaccagcagctgcccggtactgccccaaagctgctgatctacgaggacaacaagcgcccatccgggattccggatcggttcagcggatcacggtccggaactagcgcgaccctggggatcaccgggctccagactggcgacgaagcggactactactgcggaacttgggactcctccttgggggcctgggtgttcggcggagggaccaagctcaccgtgcttggagcggccgcaactaccacccctgcccctcggccgccgactccggccccaaccatcgcaagccaacccctctccttgcgccccgaagcttgccgcccggccgcgggtggagccgtgcatacccgggggctggactttgcctgcgatatctacatttgggccccgctggccggcacttgcggcgtgctcctgctgtcgctggtcatcaccctttactgcaagaggggccggaagaagctgctttacatcttcaagcagccgttcatgcggcccgtgcagacgactcaggaagaggacggatgctcgtgcagattccctgaggaggaagaggggggatgcgaactgcgcgtcaagttctcacggtccgccgacgcccccgcatatcaacagggccagaatcagctctacaacgagctgaacctgggaaggagagaggagtacgacgtgctggacaagcgacgcggacgcgacccggagatgggggggaaaccacggcggaaaaaccctcaggaaggactgtacaacgaactccagaaagacaagatggcggaagcctactcagaaatcgggatgaagggagagcggaggaggggaaagggtcacgacgggctgtaccagggactgagcaccgccactaaggatacctacgatgccttgcatatgcaagcactcccaccccgg

SEQ ID NO: 126 - protein, 493 aa, synthetic construct
  REGION 1..493: note = source = /note="Description of Artificial Sequence: Synthetic polypeptide"
MLLLVTSLLLCELPHPAFLLIPQVQLQQWGAGLLKPSETLSLTCAVYGGSFSGYYWSWIRQPPGKGLEWIGEINHSGSTNYNPSLKSRVTISVDTSKNQFSLKLSSVTAADTAVYYCARGQVKYSSSLGYWGQGTLVTVSSGGGGSGGGGSGGGGSQSVLTQPPSVSAAPGQKVTISCSGSSSNIGNNFVSWYQQLPGTAPKLLIYEDNKRPSGIPDRFSGSRSGTSATLGITGLQTGDEADYYCGTWDSSLGAWVFGGGTKLTVLGAAATTTPAPRPPTPAPTIASQPLSLRPEACRPAAGGAVHTRGLDFACDIYIWAPLAGTCGVLLLSLVITLYCKRGRKKLLYIFKQPFMRPVQTTQEEDGCSCRFPEEEEGGCELRVKFSRSADAPAYQQGQNQLYNELNLGRREEYDVLDKRRGRDPEMGGKPRRKNPQEGLYNELQKDKMAEAYSEIGMKGERRRGKGHDGLYQGLSTATKDTYDALHMQALPPR

SEQ ID NO: 127 - DNA, 1467 bp, synthetic construct
  misc_feature 1..1467: note = source = /note="Description of Artificial Sequence: Synthetic polynucleotide"
  source 1..1467: mol_type = other DNA
atgctgctgctggtgaccagcctgctgctgtgcgaactgccgcatccggcgtttctgctgattccgcaagtccaactcgtcgaaactggtggtggcctcgtgaagcctggaggatccctgcgcctttcctgtgccgcttccggctttactttctcgtcgtactccatgaactgggtcagacaggctcccggaaagggcctggaatgggtgtcctccatctcgtcctcatcctcctacatctattacgcggactccgtgaagggcagattcaccatttcccgggacaacgccaagaacagcttgtacctccaaatgaactccctgcgggcagaggacaccgccgtgtactactgcgcgagggatggggatttctggagcggagccatcgactactggggccagggaactctcgtgaccgtcagctccggtggtggtggaagcggaggcggaggttctggggggggaggatcagacattcagctgacccagtcgccatcctccctgagcgcctcagtgggggaccgcgtgactattacatgccaggcctcccaagatatctcgaactacctgaactggtatcagcagaagcctggaaaggccccgaagctgttgatctacgatgccagcaacctggagactggggtgccttcccggttctcgggatcaggctcgggcaccgatttcaccttcacgatcagcagcctgcagcccgaggacattgcaacctactactgccagcagtacgacaatctgccgctttttgggggaggcaccaagctggaaatcaaagcggccgcaactaccacccctgcccctcggccgccgactccggccccaaccatcgcaagccaacccctctccttgcgccccgaagcttgccgcccggccgcgggtggagccgtgcatacccgggggctggactttgcctgcgatatctacatttgggccccgctggccggcacttgcggcgtgctcctgctgtcgctggtcatcaccctttactgcaagaggggccggaagaagctgctttacatcttcaagcagccgttcatgcggcccgtgcagacgactcaggaagaggacggatgctcgtgcagattccctgaggaggaagaggggggatgcgaactgcgcgtcaagttctcacggtccgccgacgcccccgcatatcaacagggccagaatcagctctacaacgagctgaacctgggaaggagagaggagtacgacgtgctggacaagcgacgcggacgcgacccggagatgggggggaaaccacggcggaaaaaccctcaggaaggactgtacaacgaactccagaaagacaagatggcggaagcctactcagaaatcgggatgaagggagagcggaggaggggaaagggtcacgacgggctgtaccagggactgagcaccgccactaaggatacctacgatgccttgcatatgcaagcactcccaccccgg

SEQ ID NO: 128 - protein, 489 aa, synthetic construct
  REGION 1..489: note = source = /note="Description of Artificial Sequence: Synthetic polypeptide"
MLLLVTSLLLCELPHPAFLLIPQVQLVETGGGLVKPGGSLRLSCAASGFTFSSYSMNWVRQAPGKGLEWVSSISSSSSYIYYADSVKGRFTISRDNAKNSLYLQMNSLRAEDTAVYYCARDGDFWSGAIDYWGQGTLVTVSSGGGGSGGGGSGGGGSDIQLTQSPSSLSASVGDRVTITCQASQDISNYLNWYQQKPGKAPKLLIYDASNLETGVPSRFSGSGSGTDFTFTISSLQPEDIATYYCQQYDNLPLFGGGTKLEIKAAATTTPAPRPPTPAPTIASQPLSLRPEACRPAAGGAVHTRGLDFACDIYIWAPLAGTCGVLLLSLVITLYCKRGRKKLLYIFKQPFMRPVQTTQEEDGCSCRFPEEEEGGCELRVKFSRSADAPAYQQGQNQLYNELNLGRREEYDVLDKRRGRDPEMGGKPRRKNPQEGLYNELQKDKMAEAYSEIGMKGERRRGKGHDGLYQGLSTATKDTYDALHMQALPPR

SEQ ID NO: 129 - DNA, 1467 bp, synthetic construct
  misc_feature 1..1467: note = source = /note="Description of Artificial Sequence: Synthetic polynucleotide"
  source 1..1467: mol_type = other DNA
atgctgctgctggtgaccagcctgctgctgtgcgaactgccgcatccggcgtttctgctgattccggaggtgcaattggtgcagtcaggtggtggagtggtgcagccaggaagatcccttagactctcgtgtgcggcgtcaggctttaccttctcctcgtactccatgaactgggtcagacaggcaccgggaaagggactggaatgggtgtcctccatctcgtcctcctcctcctacatctactacgccgatagcgtgaagggccggttcaccatttcgcgcgacaacgccaagaacaccctgtacctccaaatgaattcgctgcgggccgaagataccgctgtctattactgcgcccgcgacaactggggctcgctggactattggggccagggaaccctcgtcaccgtgtcaagcggagggggtggatccggaggcggaggatccggtggagggggaagcgacattcagatgactcagagcccgtcctccctgtctgcctccgtgggggatcgcgtgaccatcacatgccaggcctcacaagacatcagcaattacctgaactggtaccagcagaagcctggaaaggcccccaagctgctgatctacgatgccagcaacctggagactggggtgccttcaaggttctccggttccggaagcggcactgacttcaccttcactatctcgagcctgcaacccgaggacattgccacctactactgccagcagtacgacaaccttccgcacatgtacacgttcggccagggcaccaagctcgaaatcaaagcggccgcaactaccacccctgcccctcggccgccgactccggccccaaccatcgcaagccaacccctctccttgcgccccgaagcttgccgcccggccgcgggtggagccgtgcatacccgggggctggactttgcctgcgatatctacatttgggccccgctggccggcacttgcggcgtgctcctgctgtcgctggtcatcaccctttactgcaagaggggccggaagaagctgctttacatcttcaagcagccgttcatgcggcccgtgcagacgactcaggaagaggacggatgctcgtgcagattccctgaggaggaagaggggggatgcgaactgcgcgtcaagttctcacggtccgccgacgcccccgcatatcaacagggccagaatcagctctacaacgagctgaacctgggaaggagagaggagtacgacgtgctggacaagcgacgcggacgcgacccggagatgggggggaaaccacggcggaaaaaccctcaggaaggactgtacaacgaactccagaaagacaagatggcggaagcctactcagaaatcgggatgaagggagagcggaggaggggaaagggtcacgacgggctgtaccagggactgagcaccgccactaaggatacctacgatgccttgcatatgcaagcactcccaccccgg

SEQ ID NO: 130 - protein, 489 aa, synthetic construct
  REGION 1..489: note = source = /note="Description of Artificial Sequence: Synthetic polypeptide"
MLLLVTSLLLCELPHPAFLLIPEVQLVQSGGGVVQPGRSLRLSCAASGFTFSSYSMNWVRQAPGKGLEWVSSISSSSSYIYYADSVKGRFTISRDNAKNTLYLQMNSLRAEDTAVYYCARDNWGSLDYWGQGTLVTVSSGGGGSGGGGSGGGGSDIQMTQSPSSLSASVGDRVTITCQASQDISNYLNWYQQKPGKAPKLLIYDASNLETGVPSRFSGSGSGTDFTFTISSLQPEDIATYYCQQYDNLPHMYTFGQGTKLEIKAAATTTPAPRPPTPAPTIASQPLSLRPEACRPAAGGAVHTRGLDFACDIYIWAPLAGTCGVLLLSLVITLYCKRGRKKLLYIFKQPFMRPVQTTQEEDGCSCRFPEEEEGGCELRVKFSRSADAPAYQQGQNQLYNELNLGRREEYDVLDKRRGRDPEMGGKPRRKNPQEGLYNELQKDKMAEAYSEIGMKGERRRGKGHDGLYQGLSTATKDTYDALHMQALPPR

SEQ ID NO: 131 - DNA, 2293 bp, synthetic construct
  misc_feature 1..2293: note = source = /note="Description of Artificial Sequence: Synthetic polynucleotide"
  source 1..2293: mol_type = other DNA
atgctcttgctcgtgacttctttgcttttgtgcgaacttccgcacccagccttccttttgatacctcaggtacagcttcaacaaagcggaccgggacttgttaagcattcccaaaccctttctctcacgtgtgcaattagcggcgatagtgtatcctctaattctgcggcctggaactggatacgacaatcaccaagccggggactcgagtggttgggccgaacctactatcggtccaaatggtataatgactacgcagtatccgtgaaatctcgcattacgatcaatccagacacctccaaaaatcaattttctctgcagttgaatagcgtgactcccgaggacacggccgtttactattgcgcccaggaagttgaaccccacgatgcatttgatatttggggccagggaaccatggtgacagtgagtagtgggggtggaggatctggaggaggcggtagcggcgggggcggcagtgatatccagatgacgcagtcaccttccagcgtgtatgcgagtgtgggggacaaggtcaccataacctgtcgcgctagccaagatgtcagcgggtggctggcttggtaccagcagaaaccaggtttggctcctcagcttttgatctcaggagcgagcacgcttcagggtgaggtcccaagtcgctttagtggctctggctccgggacagacttcacgttgacgatcagcagtttgcagcctgaggatttcgcgacctactactgccagcaagcgaaatattttccgtacactttcggtcaggggaccaaattggagatcaaaggtgggggtggttcaggcggcggaggctcaggcggcggcggtagcggaggaggcggaagcgggggtggcggatcagaagtgcaactcgttcagagtggcgcggaggttaagaaacccggtgcatctgtaaaggttagctgtaaggcatcaggatacacttttaccagctattacatgcattgggtgagacaggctcccggtcaggggctcgaatggatggggttgatcaacccgagtggtggttcaacatcttacgcccagaagtttcagggccgagtaacaatgactcgggacacgtctacctcaactgtgtatatggagctttccagcctgcgctcagaggatacagcagtctattactgcgcacggtcagacagaggtataacggccactgatgcgttcgatatctggggacaagggactatggtaactgtgtcttccggaggaggaggtagtggagggggaggaagcggtggggggggctcacagtccgttttgactcagccaccaagcgtctcagtcgcaccggggcgaatggcgaaaattacttgcggcgggagcgacataggcaacaagaatgtgcattggtaccaacagaaaccaggtcaagcacctgttctcgtggtgtatgatgactacgatcgcccaagcgggatcccggagcggttctctggatcaaattctggtgatgcagccactctgacaatatcaacggtggaagtcggtgacgaggctgattacttctgccaagtatgggatggcagcggagatccctactggatgtttggaggaggtactcaactgacagttctgggcgcggccgcaacgaccactcctgcaccccgccctccgactccggccccaaccattgccagccagcccctgtccctgcggccggaagcctgcagaccggctgccggcggagccgtccatacccggggactggatttcgcctgcgatatctatatctgggcaccactcgccggaacctgtggagtgctgctgctgtcccttgtgatcaccctgtactgcaagcgcggacggaagaaactcttgtacatcttcaagcagccgttcatgcgccctgtgcaaaccacccaagaagaggacgggtgctcctgccggttcccggaagaggaagagggcggctgcgaactgcgcgtgaagttttcccggtccgccgacgctccggcgtaccagcaggggcaaaaccagctgtacaacgaacttaacctcggtcgccgggaagaatatgacgtgctggacaagcggcggggaagagatcccgagatgggtggaaagccgcggcggaagaaccctcaggagggcttgtacaacgagctgcaaaaggacaaaatggccgaagcctactccgagattggcatgaagggagagcgcagacgcgggaagggacacgatggactgtaccagggactgtcaaccgcgactaaggacacttacgacgccctgcacatgcaggccctgcccccgcgct

SEQ ID NO: 132 - protein, 764 aa, synthetic construct
  REGION 1..764: note = source = /note="Description of Artificial Sequence: Synthetic polypeptide"
MLLLVTSLLLCELPHPAFLLIPQVQLQQSGPGLVKHSQTLSLTCAISGDSVSSNSAAWNWIRQSPSRGLEWLGRTYYRSKWYNDYAVSVKSRITINPDTSKNQFSLQLNSVTPEDTAVYYCAQEVEPHDAFDIWGQGTMVTVSSGGGGSGGGGSGGGGSDIQMTQSPSSVYASVGDKVTITCRASQDVSGWLAWYQQKPGLAPQLLISGASTLQGEVPSRFSGSGSGTDFTLTISSLQPEDFATYYCQQAKYFPYTFGQGTKLEIKGGGGSGGGGSGGGGSGGGGSGGGGSEVQLVQSGAEVKKPGASVKVSCKASGYTFTSYYMHWVRQAPGQGLEWMGLINPSGGSTSYAQKFQGRVTMTRDTSTSTVYMELSSLRSEDTAVYYCARSDRGITATDAFDIWGQGTMVTVSSGGGGSGGGGSGGGGSQSVLTQPPSVSVAPGRMAKITCGGSDIGNKNVHWYQQKPGQAPVLVVYDDYDRPSGIPERFSGSNSGDAATLTISTVEVGDEADYFCQVWDGSGDPYWMFGGGTQLTVLGAAATTTPAPRPPTPAPTIASQPLSLRPEACRPAAGGAVHTRGLDFACDIYIWAPLAGTCGVLLLSLVITLYCKRGRKKLLYIFKQPFMRPVQTTQEEDGCSCRFPEEEEGGCELRVKFSRSADAPAYQQGQNQLYNELNLGRREEYDVLDKRRGRDPEMGGKPRRKNPQEGLYNELQKDKMAEAYSEIGMKGERRRGKGHDGLYQGLSTATKDTYDALHMQALPPR

SEQ ID NO: 133 - DNA, 1476 bp, synthetic construct
  misc_feature 1..1476: note = source = /note="Description of Artificial Sequence: Synthetic polynucleotide"
  source 1..1476: mol_type = other DNA
atgcttcttttggtgacttcccttttgctgtgcgagttgccacaccccgccttcctgcttattccccaggtacagcttcaacagagtgggccgggactggtgaaacactcccaaacactttctctgacgtgcgctatatcaggtgactctgtttcatctaattctgctgcgtggaactggattcgacaatctcccagtcgcgggttggaatggctgggacgaacatattatcggtctaagtggtataacgattatgctgtatctgttaaatctcgaattacgattaatcctgacacctccaagaaccagttctccctccagttgaactcagtcacaccggaagacactgcggtctactattgcgctcaagaagtcgagccacatgatgcattcgacatctggggccagggaacgatggtcaccgtcagcagtggcggcggcggatctgggggtggcggttctggcggtggaggatcagacatacaaatgacgcagagtccctcaagtgtgtacgcgagtgtgggggataaggtaactattacgtgcagagcgtcacaggatgttagtggatggcttgcctggtatcagcagaagccaggccttgctccacagctccttatcagtggtgcttctacacttcagggcgaggttccgagtagattctctggttctggatctggtactgacttcactcttacaatttcttctttgcaaccagaagactttgcgacttattactgccaacaggccaaatacttcccttatacatttggccaaggtaccaagttggagataaaggcggccgcaactaccacccctgcccctcggccgccgactccggccccaaccatcgcaagccaacccctctccttgcgccccgaagcttgccgcccggccgcgggtggagccgtgcatacccgggggctggactttgcctgcgatatctacatttgggccccgctggccggcacttgcggcgtgctcctgctgtcgctggtcatcaccctttactgcaagaggggccggaagaagctgctttacatcttcaagcagccgttcatgcggcccgtgcagacgactcaggaagaggacggatgctcgtgcagattccctgaggaggaagaggggggatgcgaactgcgcgtcaagttctcacggtccgccgacgcccccgcatatcaacagggccagaatcagctctacaacgagctgaacctgggaaggagagaggagtacgacgtgctggacaagcgacgcggacgcgacccggagatgggggggaaaccacggcggaaaaaccctcaggaaggactgtacaacgaactccagaaagacaagatggcggaagcctactcagaaatcgggatgaagggagagcggaggaggggaaagggtcacgacgggctgtaccagggactgagcaccgccactaaggatacctacgatgccttgcatatgcaagcactcccaccccgg

SEQ ID NO: 134 - protein, 492 aa, synthetic construct
  REGION 1..492: note = source = /note="Description of Artificial Sequence: Synthetic polypeptide"
MLLLVTSLLLCELPHPAFLLIPQVQLQQSGPGLVKHSQTLSLTCAISGDSVSSNSAAWNWIRQSPSRGLEWLGRTYYRSKWYNDYAVSVKSRITINPDTSKNQFSLQLNSVTPEDTAVYYCAQEVEPHDAFDIWGQGTMVTVSSGGGGSGGGGSGGGGSDIQMTQSPSSVYASVGDKVTITCRASQDVSGWLAWYQQKPGLAPQLLISGASTLQGEVPSRFSGSGSGTDFTLTISSLQPEDFATYYCQQAKYFPYTFGQGTKLEIKAAATTTPAPRPPTPAPTIASQPLSLRPEACRPAAGGAVHTRGLDFACDIYIWAPLAGTCGVLLLSLVITLYCKRGRKKLLYIFKQPFMRPVQTTQEEDGCSCRFPEEEEGGCELRVKFSRSADAPAYQQGQNQLYNELNLGRREEYDVLDKRRGRDPEMGGKPRRKNPQEGLYNELQKDKMAEAYSEIGMKGERRRGKGHDGLYQGLSTATKDTYDALHMQALPPR

SEQ ID NO: 135 - DNA, 1476 bp, synthetic construct
  misc_feature 1..1476: note = source = /note="Description of Artificial Sequence: Synthetic polynucleotide"
  source 1..1476: mol_type = other DNA
atgttgctgctcgtgacctcgctccttctgtgcgagctgccccatccggcttttctgctcatccctcaagtgcagctgcagcagtccggtcctggactggtcaagccgtcccagactctgagcctgacttgcgccattagcgggaactcagtctcgtccaattcggcggcctggaactggatccggcagtcaccatcaaggggcctggaatggctcgggcgcacttactaccggtccaaatggtataacgactacgccgtgtccgtgaagtcccggatcaccattaaccccgacacctcgaagaaccagttctcactccaactgaacagcgtgacccccgaggataccgcggtgtactactgcgcacaagaagtggaaccgcaggacgccttcgacatttggggacagggaacgatggtcacagtgtcgtccggtggaggaggttccggaggcggtggatctggaggcggaggttcggatatccagatgacccagagcccctcctcggtgtccgcatccgtgggcgataaggtcaccattacctgtagagcgtcccaggacgtgtccggatggctggcctggtaccagcagaagccaggcttggctcctcaactgctgatctttggcgccagcactcttcagggggaggtgccatcacgcttctccggaggtggttccggcaccgacttcaccctgaccatcagcagcctccagcctgaggacttcgccacttactactgccaacaggccaagtacttcccctataccttcggacaaggcactaagctggaaatcaaggcggccgcaactaccacccctgcccctcggccgccgactccggccccaaccatcgcaagccaacccctctccttgcgccccgaagcttgccgcccggccgcgggtggagccgtgcatacccgggggctggactttgcctgcgatatctacatttgggccccgctggccggcacttgcggcgtgctcctgctgtcgctggtcatcaccctttactgcaagaggggccggaagaagctgctttacatcttcaagcagccgttcatgcggcccgtgcagacgactcaggaagaggacggatgctcgtgcagattccctgaggaggaagaggggggatgcgaactgcgcgtcaagttctcacggtccgccgacgcccccgcatatcaacagggccagaatcagctctacaacgagctgaacctgggaaggagagaggagtacgacgtgctggacaagcgacgcggacgcgacccggagatgggggggaaaccacggcggaaaaaccctcaggaaggactgtacaacgaactccagaaagacaagatggcggaagcctactcagaaatcgggatgaagggagagcggaggaggggaaagggtcacgacgggctgtaccagggactgagcaccgccactaaggatacctacgatgccttgcatatgcaagcactcccaccccgg

SEQ ID NO: 136 - protein, 492 aa, synthetic construct
  REGION 1..492: note = source = /note="Description of Artificial Sequence: Synthetic polypeptide"
MLLLVTSLLLCELPHPAFLLIPQVQLQQSGPGLVKPSQTLSLTCAISGNSVSSNSAAWNWIRQSPSRGLEWLGRTYYRSKWYNDYAVSVKSRITINPDTSKNQFSLQLNSVTPEDTAVYYCAQEVEPQDAFDIWGQGTMVTVSSGGGGSGGGGSGGGGSDIQMTQSPSSVSASVGDKVTITCRASQDVSGWLAWYQQKPGLAPQLLIFGASTLQGEVPSRFSGGGSGTDFTLTISSLQPEDFATYYCQQAKYFPYTFGQGTKLEIKAAATTTPAPRPPTPAPTIASQPLSLRPEACRPAAGGAVHTRGLDFACDIYIWAPLAGTCGVLLLSLVITLYCKRGRKKLLYIFKQPFMRPVQTTQEEDGCSCRFPEEEEGGCELRVKFSRSADAPAYQQGQNQLYNELNLGRREEYDVLDKRRGRDPEMGGKPRRKNPQEGLYNELQKDKMAEAYSEIGMKGERRRGKGHDGLYQGLSTATKDTYDALHMQALPPR

SEQ ID NO: 137 - DNA, 190 bp, synthetic construct
  misc_feature 1..190: note = source = /note="Description of Artificial Sequence: Synthetic polynucleotide"
  source 1..190: mol_type = other DNA
ggtacctgagctcagttctgagaaaagtagttctgagaaaagtagttctgagaaaagtagttctgagaaaagtagttctgagaaaagtctcgaggatatcaagatctggcctcggcggccaagcttagacactagagggtatataatggaagctcgacttccagcttggcaatccggtactgttggtaaa

SEQ ID NO: 138 - DNA, 214 bp, synthetic construct
  misc_feature 1..214: note = source = /note="Description of Artificial Sequence: Synthetic polynucleotide"
  source 1..214: mol_type = other DNA
tgagctctgagtcagtgactcagtgagtcagtgactcagtgagtcagtgactcagctcgaggatctcgctagcgggaatttccggggactttccgggaatttccggggactttccgggaatttccagatctggcctcggcggccaagcttagacactagagggtatataatggaagctcgacttccagcttggcaatccggtactgttggtaaa

SEQ ID NO: 139 - DNA, 1670 bp, synthetic construct
  misc_feature 1..1670: note = source = /note="Description of Artificial Sequence: Synthetic polynucleotide"
  source 1..1670: mol_type = other DNA
ggtacctgagctcagttctgagaaaagtagttctgagaaaagtagttctgagaaaagtagttctgagaaaagtagttctgagaaaagtctcgaggatatcaagatctggcctcggcggccaagcttagacactagagggtatataatggaagctcgacttccagcttggcaatccggtactgttggtaaaggcgcgccccaccatgctgctgctggtcaccagcctgctgctgtgcgagctccctcaccccgcctttctgcttatcccggacattcagatgacacagaccacctcgagcttgtccgcgtcgctgggcgatcgcgtgaccatctcctgccgggcctcccaagacatttcaaagtatctcaactggtaccagcagaagccggacggaaccgtgaaactgctgatctaccataccagccgcctgcactccggcgtgccgtcccgcttctccggatcgggttccggaactgactactcactgactatctccaacttggaacaagaggacatcgccacttacttctgtcaacaaggaaatacccttccctacaccttcggggggggtaccaagctggagatcactgggggcggaggctccggtggaggcggatccggcggtggagggagcgaagtcaagctgcaggaatcaggaccaggactcgtggcgccatcccagtccctgtcggtgacctgtactgtctccggagtcagcctccccgattacggagtgtcatggattaggcaacccccaagaaaagggctggaatggctcggagtgatctggggctccgaaaccacctactacaactcggcgctgaagtcccggctgaccatcatcaaggacaactccaagagccaagtgttcttgaagatgaacagcttgcagaccgacgataccgcaatctactactgtgccaagcactattactacggggggtcttacgccatggactactggggacagggcacctccgtgactgtgtcgtccgcggccgcgcccgcccctcggcccccgactcctgccccgacgatcgcttcccaacctctctcgctgcgcccggaagcatgccggcccgccgccggtggcgctgtccacactcgcggactggactttgataccgcactggcggccgtgatctgtagcgccctggccaccgtgctgctggcgctgctcatcctttgcgtgatctactgcaagcggcagcctaggcgaaagaagctcctctacattttcaagcaacccttcatgcgccccgtgcaaaccacccaggaggaggatggatgctcatgccggttccctgaggaagaagagggcggttgcgagctcagagtgaaattcagccggtcggctgacgccccggcgtaccagcagggccagaaccagctgtacaatgagctcaacctggggcgccgcgaagagtacgacgtgctggacaagaggagaggcagagatccggaaatgggcggaaagccaaggcggaagaacccgcaggaaggtctttacaacgaactgcagaaggacaagatggccgaggcctactccgagattgggatgaagggagaaagacggaggggaaagggacatgacggactttaccagggcctgagcactgccacgaaggacacctatgatgccctgcacatgcaggcgctgccgcctcgg

SEQ ID NO: 140 - DNA, 1694 bp, synthetic construct
  misc_feature 1..1694: note = source = /note="Description of Artificial Sequence: Synthetic polynucleotide"
  source 1..1694: mol_type = other DNA
tgagctctgagtcagtgactcagtgagtcagtgactcagtgagtcagtgactcagctcgaggatctcgctagcgggaatttccggggactttccgggaatttccggggactttccgggaatttccagatctggcctcggcggccaagcttagacactagagggtatataatggaagctcgacttccagcttggcaatccggtactgttggtaaaggcgcgccccaccatgctgctgctggtcaccagcctgctgctgtgcgagctccctcaccccgcctttctgcttatcccggacattcagatgacacagaccacctcgagcttgtccgcgtcgctgggcgatcgcgtgaccatctcctgccgggcctcccaagacatttcaaagtatctcaactggtaccagcagaagccggacggaaccgtgaaactgctgatctaccataccagccgcctgcactccggcgtgccgtcccgcttctccggatcgggttccggaactgactactcactgactatctccaacttggaacaagaggacatcgccacttacttctgtcaacaaggaaatacccttccctacaccttcggggggggtaccaagctggagatcactgggggcggaggctccggtggaggcggatccggcggtggagggagcgaagtcaagctgcaggaatcaggaccaggactcgtggcgccatcccagtccctgtcggtgacctgtactgtctccggagtcagcctccccgattacggagtgtcatggattaggcaacccccaagaaaagggctggaatggctcggagtgatctggggctccgaaaccacctactacaactcggcgctgaagtcccggctgaccatcatcaaggacaactccaagagccaagtgttcttgaagatgaacagcttgcagaccgacgataccgcaatctactactgtgccaagcactattactacggggggtcttacgccatggactactggggacagggcacctccgtgactgtgtcgtccgcggccgcgcccgcccctcggcccccgactcctgccccgacgatcgcttcccaacctctctcgctgcgcccggaagcatgccggcccgccgccggtggcgctgtccacactcgcggactggactttgataccgcactggcggccgtgatctgtagcgccctggccaccgtgctgctggcgctgctcatcctttgcgtgatctactgcaagcggcagcctaggcgaaagaagctcctctacattttcaagcaacccttcatgcgccccgtgcaaaccacccaggaggaggatggatgctcatgccggttccctgaggaagaagagggcggttgcgagctcagagtgaaattcagccggtcggctgacgccccggcgtaccagcagggccagaaccagctgtacaatgagctcaacctggggcgccgcgaagagtacgacgtgctggacaagaggagaggcagagatccggaaatgggcggaaagccaaggcggaagaacccgcaggaaggtctttacaacgaactgcagaaggacaagatggccgaggcctactccgagattgggatgaagggagaaagacggaggggaaagggacatgacggactttaccagggcctgagcactgccacgaaggacacctatgatgccctgcacatgcaggcgctgccgcctcgg

SEQ ID NO: 141 - DNA, 735 bp, synthetic construct
  misc_feature 1..735: note = source = /note="Description of Artificial Sequence: Synthetic polynucleotide"
  source 1..735: mol_type = other DNA
gacattcagatgactcagaccacctcctccctgtccgcctccctgggcgaccgcgtgaccatctcatgccgcgccagccaggacatctcgaagtacctcaactggtaccagcagaagcccgacggaaccgtgaagctcctgatctaccacacctcccggctgcacagcggagtgccgtctagattctcgggttcggggtcgggaactgactactcccttactatttccaacctggagcaggaggatattgccacctacttctgccaacaaggaaacaccctgccgtacacttttggcgggggaaccaagctggaaatcactggcagcacatccggttccgggaagcccggctccggagagggcagcaccaagggggaagtcaagctgcaggaatcaggacctggcctggtggccccgagccagtcactgtccgtgacttgtactgtgtccggagtgtcgctcccggattacggagtgtcctggatcaggcagccacctcggaaaggattggaatggctcggagtcatctggggttccgaaaccacctattacaactcggcactgaaatccaggctcaccattatcaaggataactccaagtcacaagtgttcctgaagatgaatagcctgcagactgacgacacggcgatctactattgcgccaagcactactactacggcggatcctacgctatggactactggggccaggggaccagcgtgaccgtgtcatcc

SEQ ID NO: 142 - DNA, 1473 bp, synthetic construct
  misc_feature 1..1473: note = source = /note="Description of Artificial Sequence: Synthetic polynucleotide"
  source 1..1473: mol_type = other DNA
atgctccttctcgtgacctccctgcttctctgcgaactgccccatcctgccttcctgctgattcccgaggtgcagttgcaacagtcaggagctgaactggtcaagccaggagccagcgtgaagatgagctgcaaggcctccggttacaccttcacctcctacaacatgcactgggtgaaacagaccccgggacaagggctcgaatggattggcgccatctaccccgggaatggcgatacttcgtacaaccagaagttcaagggaaaggccaccctgaccgccgacaagagctcctccaccgcgtatatgcagttgagctccctgacctccgaggactccgccgactactactgcgcacggtccaactactatggaagctcgtactggttcttcgatgtctggggggccggcaccactgtgaccgtcagctccgggggcggaggatccggtggaggcggaagcgggggtggaggatccgacattgtgctgactcagtccccggcaatcctgtcggcctcaccgggcgaaaaggtcacgatgacttgtagagcgtcgtccagcgtgaactacatggattggtaccaaaagaagcctggatcgtcacccaagccttggatctacgctacatctaacctggcctccggcgtgccagcgcggttcagcgggtccggctcgggcacctcatactcgctgaccatctcccgcgtggaggctgaggacgccgcgacctactactgccagcagtggtccttcaacccgccgacttttggaggcggtactaagctggagatcaaagcggccgcaactaccacccctgcccctcggccgccgactccggccccaaccatcgcaagccaacccctctccttgcgccccgaagcttgccgcccggccgcgggtggagccgtgcatacccgggggctggactttgcctgcgatatctacatttgggccccgctggccggcacttgcggcgtgctcctgctgtcgctggtcatcaccctttactgcaagaggggccggaagaagctgctttacatcttcaagcagccgttcatgcggcccgtgcagacgactcaggaagaggacggatgctcgtgcagattccctgaggaggaagaggggggatgcgaactgcgcgtcaagttctcacggtccgccgacgcccccgcatatcaacagggccagaatcagctctacaacgagctgaacctgggaaggagagaggagtacgacgtgctggacaagcgacgcggacgcgacccggagatgggggggaaaccacggcggaaaaaccctcaggaaggactgtacaacgaactccagaaagacaagatggcggaagcctactcagaaatcgggatgaagggagagcggaggaggggaaagggtcacgacgggctgtaccagggactgagcaccgccactaaggatacctacgatgccttgcatatgcaagcactcccaccccgg

SEQ ID NO: 143 - protein, 491 aa, synthetic construct
  REGION 1..491: note = source = /note="Description of Artificial Sequence: Synthetic polypeptide"
MLLLVTSLLLCELPHPAFLLIPEVQLQQSGAELVKPGASVKMSCKASGYTFTSYNMHWVKQTPGQGLEWIGAIYPGNGDTSYNQKFKGKATLTADKSSSTAYMQLSSLTSEDSADYYCARSNYYGSSYWFFDVWGAGTTVTVSSGGGGSGGGGSGGGGSDIVLTQSPAILSASPGEKVTMTCRASSSVNYMDWYQKKPGSSPKPWIYATSNLASGVPARFSGSGSGTSYSLTISRVEAEDAATYYCQQWSFNPPTFGGGTKLEIKAAATTTPAPRPPTPAPTIASQPLSLRPEACRPAAGGAVHTRGLDFACDIYIWAPLAGTCGVLLLSLVITLYCKRGRKKLLYIFKQPFMRPVQTTQEEDGCSCRFPEEEEGGCELRVKFSRSADAPAYQQGQNQLYNELNLGRREEYDVLDKRRGRDPEMGGKPRRKNPQEGLYNELQKDKMAEAYSEIGMKGERRRGKGHDGLYQGLSTATKDTYDALHMQALPPR

SEQ ID NO: 144 - DNA, 750 bp, synthetic construct
  misc_feature 1..750: note = source = /note="Description of Artificial Sequence: Synthetic polynucleotide"
  source 1..750: mol_type = other DNA
gaagtgcaattggtgcagagcggtggaggacttgtgaaacctggtggatccctgagactttcctgtgccgcttcgggcttcaccttctcggactactacatgtcctggattcgccaggcccctggaaagggactggaatgggtgtcatacatcagctcctccggttccaccatctactatgccgattccgtgaagggcagattcaccatctcgcgcgacaacgccaagaacactctctatctgcaaatgaactcactgcgggctgaggacaccgcggtctactactgcgcccgggacctcagcggaaagtccagcggatggtcccattacttcgattactggggacagggaaccctggtcaccgtgtccagcggcggggggggctcgggtggcggcggctccggcggcggcgggagcaacttcatgctgactcagccccactccgtgtccgagagcccgggaaagaccgtgactatttcgtgcacacggtcctccgggagcattgcgaacaactacgtgcagtggtaccagcagcggcccgatagggccccaaccactgtgatctacgaagatgaccagcggccgtctggagtcccggaccgcttctcggggtccatcgactcatcatccaattccgcatcgctgacgatcagcggactgaagatcgaggacgaagccgattactactgccagtcctacgacggcaccaactgggtctttgggggtggaaccaagctgactgtgctcgga

SEQ ID NO: 145 - protein, 250 aa, synthetic construct
  REGION 1..250: note = source = /note="Description of Artificial Sequence: Synthetic polypeptide"
EVQLVQSGGGLVKPGGSLRLSCAASGFTFSDYYMSWIRQAPGKGLEWVSYISSSGSTIYYADSVKGRFTISRDNAKNTLYLQMNSLRAEDTAVYYCARDLSGKSSGWSHYFDYWGQGTLVTVSSGGGGSGGGGSGGGGSNFMLTQPHSVSESPGKTVTISCTRSSGSIANNYVQWYQQRPDRAPTTVIYEDDQRPSGVPDRFSGSIDSSSNSASLTISGLKIEDEADYYCQSYDGTNWVFGGGTKLTVLG

SEQ ID NO: 146 - DNA, 729 bp, synthetic construct
  misc_feature 1..729: note = source = /note="Description of Artificial Sequence: Synthetic polynucleotide"
  source 1..729: mol_type = other DNA
gaagtgcaacttgtcgaaagcggtggaggtcttgtccaacctggtcgctccctgaggctctcgtgtgccgcgagcggattcaccttctcatcgtacgctatgtcctgggtcagacaggctcctggaaagggcctggaatgggtggccgtgatctcctacgacggcagcaacaagtattacgccgactcagtgaagggccggttcaccatttcccgggacaacagcaagaacaccctgtacttgcaaatgaactccctgcgggccgaggataccgcggtgtactactgcgcccacctccgctttggatacggaatggatgtctggggacagggaactaccgtgaccgtgtcgtccgggggggggggaagcggcggcgggggatcgggtggcggcggatcccagactgtggtcacccaagagccttcactgaccgtgtccccgggtggcaccgtgacgctgacttgcgcgtcatctaccggggccgtgacctcggaccactacccctgctggttccagcagaaacccggacatccaccgagagccctggtgtactccactgacaccatccactcctggactccggcccggttctccggaagcctcctgggcgggaaggccgcactgacagtgtccggagtgcagcccgaggatgaagccgactactactgtctgctctactatgggggagcacgcgtgttcggtggcggcactcagctgaccgtgctggga

SEQ ID NO: 147 - protein, 243 aa, synthetic construct
  REGION 1..243: note = source = /note="Description of Artificial Sequence: Synthetic polypeptide"
EVQLVESGGGLVQPGRSLRLSCAASGFTFSSYAMSWVRQAPGKGLEWVAVISYDGSNKYYADSVKGRFTISRDNSKNTLYLQMNSLRAEDTAVYYCAHLRFGYGMDVWGQGTTVTVSSGGGGSGGGGSGGGGSQTVVTQEPSLTVSPGGTVTLTCASSTGAVTSDHYPCWFQQKPGHPPRALVYSTDTIHSWTPARFSGSLLGGKAALTVSGVQPEDEADYYCLLYYGGARVFGGGTQLTVLG

SEQ ID NO: 148 - DNA, 723 bp, synthetic construct
  misc_feature 1..723: note = source = /note="Description of Artificial Sequence: Synthetic polynucleotide"
  source 1..723: mol_type = other DNA
caagtccaactcgtccagtccggtgccgaagtcaagaagcctggctcatccgtgaaagtgtcctgcaaagcatcgggcggaaccttctcctcctatgccatttcctgggtccgccaggcaccgggccagggtctggagtggatgggcgggattatccctatcttcggaactgccaaccacgcccaaaagttccagggacgcgtgaccattaccgccgatgaatcaacctcaaccgcctacatggaactgtccagcttgaggtccgaggacaccgccgtgtactactgcgcgttcatgatggtgccggagtactactttgactactggggccagggaacccttgtgaccgtgtcgtccggtggtggcggatccgggggggggggatctgggggcggcggaagcgatatccagatgacccagtcgccatcgagcctgtccgcttccgtgggcgacagagtgacgatcacttgccgggcttcacaaggcatcagaaatgacctgggctggtatcagcagaagcccggagaagcgcccaagcggctgatctacgcggccagcaccctgcaaaacggagtgccttcgcggttctccgggagcggctccggaactgacttcactctgactattaacagcctccagcccgaggatttcgccacatactactgtcagcagtacaacagctacccgtacaccttcggacagggaactaagctcgaaatcaag

SEQ ID NO: 149 - protein, 241 aa, synthetic construct
  REGION 1..241: note = source = /note="Description of Artificial Sequence: Synthetic polypeptide"
QVQLVQSGAEVKKPGSSVKVSCKASGGTFSSYAISWVRQAPGQGLEWMGGIIPIFGTANHAQKFQGRVTITADESTSTAYMELSSLRSEDTAVYYCAFMMVPEYYFDYWGQGTLVTVSSGGGGSGGGGSGGGGSDIQMTQSPSSLSASVGDRVTITCRASQGIRNDLGWYQQKPGEAPKRLIYAASTLQNGVPSRFSGSGSGTDFTLTINSLQPEDFATYYCQQYNSYPYTFGQGTKLEIK

SEQ ID NO: 150 - DNA, 756 bp, synthetic construct
  misc_feature 1..756: note = source = /note="Description of Artificial Sequence: Synthetic polynucleotide"
  source 1..756: mol_type = other DNA
caactccaactccaagaatctggaccaggcctcgtgaagccctcccaaactctgtccctgacctgtaccgtgtcgggtggaagcatttcgagcggtggatactactggtcctggatcaggcagcatcctggaaagggactggagtggattgggtacatctactactccggctcaacctactacaacccgtccttgaaatcgcgcgtgacgatctccgtggacacttcaaagaaccagttcagcctgaagctttcctccgtgaccgcggccgatacagcggtgtactactgcgctcgggatcagagcgtggccgaccctggtggcggctactactactacggaatggatgtctggggacagggaaccaccgtgactgtgtccagcgggggcggcggatccgggggggggggatcgggcggcggcggttcgcagtccgtgctgacccagccacctagcgtgtcagtggcaccgggacagaccgcctccatttcctgcgggggaaatgacttcggtagccgctccgtgtcatggtatcaccagaagccgggacaggccccggtgctggtcatctatgacgacaacgacagaccctcgggcatccccgaacggttttcgggaagcacctccggagacactgccaccctgaccatctcccgggtcgaggtcggcgatgaagccgattactactgccaagtctgggacgacgactccgaccactgggtgttcggcggcggaactaagctgactgtgctgggg

SEQ ID NO: 151 - protein, 252 aa, synthetic construct
  REGION 1..252: note = source = /note="Description of Artificial Sequence: Synthetic polypeptide"
QLQLQESGPGLVKPSQTLSLTCTVSGGSISSGGYYWSWIRQHPGKGLEWIGYIYYSGSTYYNPSLKSRVTISVDTSKNQFSLKLSSVTAADTAVYYCARDQSVADPGGGYYYYGMDVWGQGTTVTVSSGGGGSGGGGSGGGGSQSVLTQPPSVSVAPGQTASISCGGNDFGSRSVSWYHQKPGQAPVLVIYDDNDRPSGIPERFSGSTSGDTATLTISRVEVGDEADYYCQVWDDDSDHWVFGGGTKLTVLG

SEQ ID NO: 152 - DNA, 723 bp, synthetic construct
  misc_feature 1..723: note = source = /note="Description of Artificial Sequence: Synthetic polynucleotide"
  source 1..723: mol_type = other DNA
caggtgcagctgcaggagtccggcccaggactggtgaagccttcggagaccctgtccctcacctgcactgtctctggtggctccatcagcagtagtagttactactggggctggatccgccagcccccagggaaggggctggagtggattgggagtatctattatagtgggagcacctactacaacccgtccctcaagagtcgagtcaccatacccgtagacacgtccaagaaccagttctccctgaagctgagctctgtgaccgccgcagacacggctgtgtattactgtgcgagacacctggggggtgatgcttttgatatctggggccaagggaccacggtcaccgtctcctcaggaggtggcgggtctggtggtggcggtagcggtggaggcggatccctgcctgtgctgactcagcccccctcggtgtcagtggccccaggacagacggccaggattacctgtggggggaacaacattggaagtaaaagtgtgcactggtaccagcagaagccaggccaggcccctgtgctggtcgtctatgatgatagcgaccggccctcagggatccctgagcgattctctggctccaactctgggaacacagccactctgaccatcagcgggacccaggctatggatgaggctgactacttctgtcagtcttatgatagcagcaatcccgtggtattcggcggagggacccagctcaccgtttta

SEQ ID NO: 153 - protein, 241 aa, synthetic construct
  REGION 1..241: note = source = /note="Description of Artificial Sequence: Synthetic polypeptide"
QVQLQESGPGLVKPSETLSLTCTVSGGSISSSSYYWGWIRQPPGKGLEWIGSIYYSGSTYYNPSLKSRVTIPVDTSKNQFSLKLSSVTAADTAVYYCARHLGGDAFDIWGQGTTVTVSSGGGGSGGGGSGGGGSLPVLTQPPSVSVAPGQTARITCGGNNIGSKSVHWYQQKPGQAPVLVVYDDSDRPSGIPERFSGSNSGNTATLTISGTQAMDEADYFCQSYDSSNPVVFGGGTQLTVL

SEQ ID NO: 154 - DNA, 732 bp, synthetic construct
  misc_feature 1..732: note = source = /note="Description of Artificial Sequence: Synthetic polynucleotide"
  source 1..732: mol_type = other DNA
caggcggcccaggtacagctgcagcagtcaggggctgaggtgaagaagcctgggtcctcggtgaaggtctcctgcaaggcttctggaggcaccttcagcagctatgctatcagctgggtgcgacaggcccctggacaagggcttgagtggatgggatggatcaaccctaacagtggtggcacaaactatgcacagaggtttcagggcagggtcaccatgaccagggacacgtccatcagcacagcctacatggagctgagcaggctgagatctgacgacacggccgtgtattactgtgcgagttataatgatgcttttgatatctggggccaaggcaccctggtcaccgtctcctcaggaggtggcgggtctggtggtggcggtagcggtggtggcggatccaattttatgctgactcagccccactctgtgtcggagtctccggggaagacggtaaccatctcctgcacccgcagcagtggcagcattgccagcaactatgtgcagtggtaccagcagcgcccgggcagtgcccccaccattgtgatctatgaggatgatcaaagaccctctggggtccctgatcggttctctggctccatcgacacctcctccaactctgcctccctcaccatctctggactgcagagtgaggacgaggctgactactactgtcagtcttatgagcccggcaatggggtattcggcggagggaccaaggtcaccgtccta

SEQ ID NO: 155 - protein, 244 aa, synthetic construct
  REGION 1..244: note = source = /note="Description of Artificial Sequence: Synthetic polypeptide"
QAAQVQLQQSGAEVKKPGSSVKVSCKASGGTFSSYAISWVRQAPGQGLEWMGWINPNSGGTNYAQRFQGRVTMTRDTSISTAYMELSRLRSDDTAVYYCASYNDAFDIWGQGTLVTVSSGGGGSGGGGSGGGGSNFMLTQPHSVSESPGKTVTISCTRSSGSIASNYVQWYQQRPGSAPTIVIYEDDQRPSGVPDRFSGSIDTSSNSASLTISGLQSEDEADYYCQSYEPGNGVFGGGTKVTVL

SEQ ID NO: 156 - DNA, 744 bp, synthetic construct
  misc_feature 1..744: note = source = /note="Description of Artificial Sequence: Synthetic polynucleotide"
  source 1..744: mol_type = other DNA
caagaacagcttgtagagtccggcggtagattggtgacaccgggggggagccttaccctgtcttgtaaggcatctgggttcgatttcagtgcgtattatatgagctgggttcggcaggcgcccgggaaggggctggaatggatagccactatatacccgtcatccggcaagacttactacgcgacttgggtaaacgggaggtttacgataagctcagataacgcccaaaacacggttgatctccaaatgaatagcttgaccgccgctgatagggcgacctatttctgtgcgcgggactcttacgctgatgacggggccctcttcaatatatggggaccgggaacgctcgtaaccatatcatctggaggaggtgggagcggaggcggagggtcaggtgggggcgggagcgaactcgtacttacacaatctccaagcgtaagcgcagcgttggggagtccagcaaagatcacctgcactttgtcaagcgcccacaaaacggatacgatagattggtatcagcaactccaaggtgaagcgccacgatatctcatgcaggtacagagcgacgggagttatactaagaggcccggggtcccagacagattcagtggcagcagttcaggtgccgacagatacctgataataccctcagttcaagccgatgatgaagccgattactactgtggggctgactacataggtgggtatgttttcgggggcggcactcaattgacagttacaggg

SEQ ID NO: 157 - protein, 248 aa, synthetic construct
  REGION 1..248: note = source = /note="Description of Artificial Sequence: Synthetic polypeptide"
QEQLVESGGRLVTPGGSLTLSCKASGFDFSAYYMSWVRQAPGKGLEWIATIYPSSGKTYYATWVNGRFTISSDNAQNTVDLQMNSLTAADRATYFCARDSYADDGALFNIWGPGTLVTISSGGGGSGGGGSGGGGSELVLTQSPSVSAALGSPAKITCTLSSAHKTDTIDWYQQLQGEAPRYLMQVQSDGSYTKRPGVPDRFSGSSSGADRYLIIPSVQADDEADYYCGADYIGGYVFGGGTQLTVTG

SEQ ID NO: 158 - DNA, 720 bp, synthetic construct
  misc_feature 1..720: note = source = /note="Description of Artificial Sequence: Synthetic polynucleotide"
  source 1..720: mol_type = other DNA
gaagtgcaactcgtcgaaactggagccgaagtgaaaaagcctggagcgtccgtcaaagtgtcgtgcaaggcctccggctacaccttcacgacctactacgtgcactgggtcagacaggctccgggtcaagggctggagtggatgggcatcattaacccctccggtggaagcacctcctatgcgcaaaagttccagggtcgcgtcaccatgactcgcgatacctccacttccactgtgtacatggaactgagctccctgaggtccgaggacaccgccgtgtactactgcgcacgggatggaggcttgggcggctacgaggcttggggacagggcaccctcgtgactgtgtcaagcggagggggtggatccggagggggaggatcaggcggtggtggaagcgatatccagcttacccagtcgccttccgcgctgtctgcatcggccggcgacagagtgacaattacctgtcaagccagccaggacatctccaactatctgaactggtaccagcagaagcccggaaaggctccgaagctgctgatctacgacgccagcaacctggaacggggcgtgccatcacggttctcgggatcagggtcgggcactgagttcaccttcaccatctcctccctccaacccgaggacattgccacctactactgccagcagtacgacaacctcccgatcacctttggacaggggactcgcctggaaatcaag

SEQ ID NO: 159 - protein, 240 aa, synthetic construct
  REGION 1..240: note = source = /note="Description of Artificial Sequence: Synthetic polypeptide"
EVQLVETGAEVKKPGASVKVSCKASGYTFTTYYVHWVRQAPGQGLEWMGIINPSGGSTSYAQKFQGRVTMTRDTSTSTVYMELSSLRSEDTAVYYCARDGGLGGYEAWGQGTLVTVSSGGGGSGGGGSGGGGSDIQLTQSPSALSASAGDRVTITCQASQDISNYLNWYQQKPGKAPKLLIYDASNLERGVPSRFSGSGSGTEFTFTISSLQPEDIATYYCQQYDNLPITFGQGTRLEIK

SEQ ID NO: 160 - DNA, 759 bp, synthetic construct
  misc_feature 1..759: note = source = /note="Description of Artificial Sequence: Synthetic polynucleotide"
  source 1..759: mol_type = other DNA
gaagtgcaattggtccagagcggaggaggacttgtgaagccaggcggatccctgagattgtcatgcgccgcatcggggttcaccttttcctcctactccatgaactgggtcagacaggcgcccggaaagggacttgaatgggtgtcgtccatttcctcctcctcgtcctacatctactacgccgactccgtgaagggccgcttcaccatctcccgggacaacgccaagaacagcctgtatctccaaatgaactccctgcgggccgaagatactgctgtgtattactgcgctcgggacttcccgtacgactcatcgggctattactcggacgcgttcgatatctggggccagggaactatggtcaccgtcagctctggtggcggtggttccggagggggtggatccggtggcggaggatcagagattgtgctgacccagtccccgctgtcactgcccgtgactccgggagagcctgcctcgatctcgtgtcggtccagccagtccctgctgcactcgaatgggtacaactacctcgattggtacctccaaaagcctgggcagtcaccccaactgctgatctacctcgggagcaacagagccagcggagtgcctgaccgctttagcggttccggatccggcaccgacttcaccctgaaaatcagccgggtggaagccgaggatgtcggcgtgtactactgcatgcaggcactgcagactctggggtacaccttcggccagggcacgaagctcgagatcaag

SEQ ID NO: 161 - protein, 253 aa, synthetic construct
  REGION 1..253: note = source = /note="Description of Artificial Sequence: Synthetic polypeptide"
EVQLVQSGGGLVKPGGSLRLSCAASGFTFSSYSMNWVRQAPGKGLEWVSSISSSSSYIYYADSVKGRFTISRDNAKNSLYLQMNSLRAEDTAVYYCARDFPYDSSGYYSDAFDIWGQGTMVTVSSGGGGSGGGGSGGGGSEIVLTQSPLSLPVTPGEPASISCRSSQSLLHSNGYNYLDWYLQKPGQSPQLLIYLGSNRASGVPDRFSGSGSGTDFTLKISRVEAEDVGVYYCMQALQTLGYTFGQGTKLEIK

SEQ ID NO: 162 - DNA, 747 bp, synthetic construct
  misc_feature 1..747: note = source = /note="Description of Artificial Sequence: Synthetic polynucleotide"
  source 1..747: mol_type = other DNA
caagtgcaactcgtccaatccggtgccgaagtcaagaagcctggttcctccgtgaaagtgtcgtgcaaagccagcggcgggacttttagctcctacgcgatcagctgggtcagacaggcccctggacaaggcctcgagtggatgggcggcatcattccgattttcggtaccgccaactacgcccagaagttccagggacgcgtgaccattactaccgacgagagcacctcaaccgcatacatggaactgtccagcctgcgctccgaggacacggctgtgtactattgcgccagacggggatggggaggattctcctccggctccgcattcgacatctggggacagggcactatggtcactgtgtcatccgggggaggaggatcaggcggtggaggatccggtggtggcggatccaacttcatgctgacccagccccactcagtgtcggaatcgcccggcaacaccgtgactatcagctgcaccggatccagcgggaccatcggctctaatttcgtgcagtggtaccagcagtccccagggagagctccgaccctgttgatctacgaggacacaaagcggccaagcggagtgccgcctagattcgccggctccgtggattcctcgtccaactcggcgtcgctgaccatcagcggactcaagactgaagatgaagccgactactactgtcagtcctacgactcgagcaactgggtgtttgggggcgggactaagctgaccgtgcttgga

SEQ ID NO: 163 - protein, 249 aa, synthetic construct
  REGION 1..249: note = source = /note="Description of Artificial Sequence: Synthetic polypeptide"
QVQLVQSGAEVKKPGSSVKVSCKASGGTFSSYAISWVRQAPGQGLEWMGGIIPIFGTANYAQKFQGRVTITTDESTSTAYMELSSLRSEDTAVYYCARRGWGGFSSGSAFDIWGQGTMVTVSSGGGGSGGGGSGGGGSNFMLTQPHSVSESPGNTVTISCTGSSGTIGSNFVQWYQQSPGRAPTLLIYEDTKRPSGVPPRFAGSVDSSSNSASLTISGLKTEDEADYYCQSYDSSNWVFGGGTKLTVLG

SEQ ID NO: 164 - DNA, 735 bp, synthetic construct
  misc_feature 1..735: note = source = /note="Description of Artificial Sequence: Synthetic polynucleotide"
  source 1..735: mol_type = other DNA
gaagtccaattggtgcagagcggatccgaacttaagaaacctggcgcgagcgtgaaagtgtcctgcaaggcctccggagggactttctcgtcgtacgccattagctgggtccgccaagctcctggccaaggcctggagtggatgggcgggattatccccatcttcgggactgcgaactacgcccagaagtttcagggccgggtcactatcaccgccgacgaatcaacctcgaccgcctacatggaactgtcctcgcttcggtccgaggatactgccgtgtactattgtgcctcaacggccagacgcggatgggacaccgctggtccgctcgattactggggccagggaaccctcgtgaccgtcagctccggaggaggaggctccggtggtggaggatccgggggtggtggatccgacatccaaatgacccagtccccctcgtccctgagcgcctctgtgggcgacagagtgacaattgcatgcagggcctcacagactatctcccgctacctgaactggtaccagcagaagccaggaaaggcccctaagctgctcatctacgctgcgtcctcgctccaatccggggtgtcctcacggttttccggatcgggttccggcaccgagttcaccctgaccatcagcagcctgcagcccgaggacttcgcaacctacttctgccagcaaacctactccccgccgattacgttcggacaggggactcggctggaaatcaag

SEQ ID NO: 165 - protein, 245 aa, synthetic construct
  REGION 1..245: note = source = /note="Description of Artificial Sequence: Synthetic polypeptide"
EVQLVQSGSELKKPGASVKVSCKASGGTFSSYAISWVRQAPGQGLEWMGGIIPIFGTANYAQKFQGRVTITADESTSTAYMELSSLRSEDTAVYYCASTARRGWDTAGPLDYWGQGTLVTVSSGGGGSGGGGSGGGGSDIQMTQSPSSLSASVGDRVTIACRASQTISRYLNWYQQKPGKAPKLLIYAASSLQSGVSSRFSGSGSGTEFTLTISSLQPEDFATYFCQQTYSPPITFGQGTRLEIK

SEQ ID NO: 166 - DNA, 729 bp, synthetic construct
  misc_feature 1..729: note = source = /note="Description of Artificial Sequence: Synthetic polynucleotide"
  source 1..729: mol_type = other DNA
gaagtgcaactcgtcgaaacaggggcagaagtgaaaaacccaggctcaagcgtgaaagtgtcgtgcaaggcttcgggcggaactctgtccaactacgccatctcctgggtccgccaagctccgggaaagggcctcgagtggatgggcggaatcattcccattttcgggaccgccaactacgcgcaaaagttccagggccgggtcactatcaccgcggacgaaagcaccagcaccgcctacatggaactgtcctccctgcgctccgaggacactgccgtgtactattgcgcccggaggtcatcgtggtaccccgagggctgcttccagcactggggacagggcactctcgtgaccgtgtcgtcgggtggtggtggatcaggagggggaggatccggaggaggcggaagcgatattcagctgacccagtcaccgagctccctgtccgcctccaccggagacagagtgaccatcacgtgtcgggcctcccaagggatctcctcctacctggcctggtaccagcagaagcctggaaaggcaccgaagttgctgatctacgccgcgagcacccttcagtccggagtgcctagccgcttctcgggttccggctctggcactgacttcactctgaccattagctgcctgcagtccgaggattttgccacctactactgccagcagtactatagctaccccctgaccttcgggggcggaaccaagctcgacatcaag

SEQ ID NO: 167 - protein, 243 aa, synthetic construct
  REGION 1..243: note = source = /note="Description of Artificial Sequence: Synthetic polypeptide"
EVQLVETGAEVKNPGSSVKVSCKASGGTLSNYAISWVRQAPGKGLEWMGGIIPIFGTANYAQKFQGRVTITADESTSTAYMELSSLRSEDTAVYYCARRSSWYPEGCFQHWGQGTLVTVSSGGGGSGGGGSGGGGSDIQLTQSPSSLSASTGDRVTITCRASQGISSYLAWYQQKPGKAPKLLIYAASTLQSGVPSRFSGSGSGTDFTLTISCLQSEDFATYYCQQYYSYPLTFGGGTKLDIK

SEQ ID NO: 168 - DNA, 732 bp, synthetic construct
  misc_feature 1..732: note = source = /note="Description of Artificial Sequence: Synthetic polynucleotide"
  source 1..732: mol_type = other DNA
gaagtgcaactcgtccaatctggtgccgaagtcaagaagcctggctcaagcgtgaaagtgtcctgcaaagcgtcgggagggaccttcagctcctacgccatttcctgggtccgccaagcaccaggacagggcctggagtggatgggcggcatcatcccgatcttcgggactgccaactacgcccagaagttccaggggagagtgaccattaccgccgacgagtcgaccagcacggcctacatggaactgtccagcctgcgctccgaggacactgccgtgtactactgcgcgagggccagactcggtggagcgttcgacatctggggacagggcaccatggtcaccgtgtcatccggtggcggaggatccggtggtggcggatcaggagggggaggatcccagtccgtgctgactcagcctccctccgtgagcgctgcaccgggacagaaggtcaccatctcatgctcggggggaagctccaacatcgggaaccactacgtgtcctggtaccaacagttgcctggtgccgctccaaagctgctgatctatgacgataacaagcggccgtccggaatccccgaccggttctcggggtctagatccggaaccagcgcaactctcggcattaccggactgcagagcggcgatgaggccgactactactgtggcacatgggactcgtcgctggctgcccacgtgtttggcactggcaccaaggtcaccgtgcttgga

SEQ ID NO: 169 - protein, 244 aa, synthetic construct
  REGION 1..244: note = source = /note="Description of Artificial Sequence: Synthetic polypeptide"
EVQLVQSGAEVKKPGSSVKVSCKASGGTFSSYAISWVRQAPGQGLEWMGGIIPIFGTANYAQKFQGRVTITADESTSTAYMELSSLRSEDTAVYYCARARLGGAFDIWGQGTMVTVSSGGGGSGGGGSGGGGSQSVLTQPPSVSAAPGQKVTISCSGGSSNIGNHYVSWYQQLPGAAPKLLIYDDNKRPSGIPDRFSGSRSGTSATLGITGLQSGDEADYYCGTWDSSLAAHVFGTGTKVTVLG

SEQ ID NO: 170 - DNA, 747 bp, synthetic construct
  misc_feature 1..747: note = source = /note="Description of Artificial Sequence: Synthetic polynucleotide"
  source 1..747: mol_type = other DNA
gaagtgcaacttgtccagagcggagccgaagtgaagaaacctggatcctccgtcaaagtgtcgtgcaaggcttcgggcggaaccttctcctcgtacgcgatctcatgggtcagacaggcacccggacagggactggagtggatgggcggcatcattcccatcttcggcaccgctaattacgcccagaagtttcaggggagagtgaccatcaccgccgacgagtccacctccactgcctacatggaactgtcctcactgaggtccgaggatactgccgtgtactactgcgcgtcgcaaaaggggggtggatggtccattgacgccttcgatatttggggacaggggacgatggtcacagtgtcatccggcggtggtggatccggtggtggcggatccggaggaggaggcagccagtccgtgctgacccagccgcctagcgtgtcggccgcatctgggcagcgcgtgaccatttcctgttccgggtcctcgtccaacatcggcaacaactacgcctcctggtaccaacagctcccgggaatggcccctaagctgctgatctacgaggacaacaagcggccatccgggatctcagaccggttcagcggatcccagtccggcacttccgcgagcctcgccatcaccggactgcaggctgaggacgaagccgactactactgccaatcatatgacagctcgctcagcggcgatgtggtgttcggcggtggcactaagctgaccgtgttggga

SEQ ID NO: 171 - protein, 249 aa, synthetic construct
  REGION 1..249: note = source = /note="Description of Artificial Sequence: Synthetic polypeptide"
EVQLVQSGAEVKKPGSSVKVSCKASGGTFSSYAISWVRQAPGQGLEWMGGIIPIFGTANYAQKFQGRVTITADESTSTAYMELSSLRSEDTAVYYCASQKGGGWSIDAFDIWGQGTMVTVSSGGGGSGGGGSGGGGSQSVLTQPPSVSAASGQRVTISCSGSSSNIGNNYASWYQQLPGMAPKLLIYEDNKRPSGISDRFSGSQSGTSASLAITGLQAEDEADYYCQSYDSSLSGDVVFGGGTKLTVLG

SEQ ID NO: 172 - DNA, 735 bp, synthetic construct
  misc_feature 1..735: note = source = /note="Description of Artificial Sequence: Synthetic polynucleotide"
  source 1..735: mol_type = other DNA
caagtccagttgcaacaatggggagcaggccttctgaaaccgtccgagacactgagcctgacgtgcgccgtctatggcggatcgttctccggatactactggtcgtggatcagacagcctccgggaaagggtctggaatggatcggcgaaatcaaccacagcggcagcaccaattacaacccgtcactgaagtcaagggtcaccattagcgtggacacttccaagaaccagttctccctgaaactgtcgagcgtgaccgctgccgatactgccgtgtactactgtgcccgcggccaagtcaagtatagctcaagcctcggctactggggccagggaaccctcgtgaccgtgtcctcgggtggaggaggctccggtggtggaggatccggtggcggaggatcgcagtccgtgctgacccagcctccctccgtgtctgctgcccctgggcaaaaggtcaccatttcgtgctccggctcatcgtccaacatcgggaacaactttgtgtcctggtaccagcagctgcccggtactgccccaaagctgctgatctacgaggacaacaagcgcccatccgggattccggatcggttcagcggatcacggtccggaactagcgcgaccctggggatcaccgggctccagactggcgacgaagcggactactactgcggaacttgggactcctccttgggggcctgggtgttcggcggagggaccaagctcaccgtgcttgga

SEQ ID NO: 173 - protein, 245 aa, synthetic construct
  REGION 1..245: note = source = /note="Description of Artificial Sequence: Synthetic polypeptide"
QVQLQQWGAGLLKPSETLSLTCAVYGGSFSGYYWSWIRQPPGKGLEWIGEINHSGSTNYNPSLKSRVTISVDTSKNQFSLKLSSVTAADTAVYYCARGQVKYSSSLGYWGQGTLVTVSSGGGGSGGGGSGGGGSQSVLTQPPSVSAAPGQKVTISCSGSSSNIGNNFVSWYQQLPGTAPKLLIYEDNKRPSGIPDRFSGSRSGTSATLGITGLQTGDEADYYCGTWDSSLGAWVFGGGTKLTVLG

SEQ ID NO: 174 - DNA, 723 bp, synthetic construct
  misc_feature 1..723: note = source = /note="Description of Artificial Sequence: Synthetic polynucleotide"
  source 1..723: mol_type = other DNA
caagtccaactcgtcgaaactggtggtggcctcgtgaagcctggaggatccctgcgcctttcctgtgccgcttccggctttactttctcgtcgtactccatgaactgggtcagacaggctcccggaaagggcctggaatgggtgtcctccatctcgtcctcatcctcctacatctattacgcggactccgtgaagggcagattcaccatttcccgggacaacgccaagaacagcttgtacctccaaatgaactccctgcgggcagaggacaccgccgtgtactactgcgcgagggatggggatttctggagcggagccatcgactactggggccagggaactctcgtgaccgtcagctccggtggtggtggaagcggaggcggaggttctggggggggaggatcagacattcagctgacccagtcgccatcctccctgagcgcctcagtgggggaccgcgtgactattacatgccaggcctcccaagatatctcgaactacctgaactggtatcagcagaagcctggaaaggccccgaagctgttgatctacgatgccagcaacctggagactggggtgccttcccggttctcgggatcaggctcgggcaccgatttcaccttcacgatcagcagcctgcagcccgaggacattgcaacctactactgccagcagtacgacaatctgccgctttttgggggaggcaccaagctggaaatcaaa

SEQ ID NO: 175 - protein, 241 aa, synthetic construct
  REGION 1..241: note = source = /note="Description of Artificial Sequence: Synthetic polypeptide"
QVQLVETGGGLVKPGGSLRLSCAASGFTFSSYSMNWVRQAPGKGLEWVSSISSSSSYIYYADSVKGRFTISRDNAKNSLYLQMNSLRAEDTAVYYCARDGDFWSGAIDYWGQGTLVTVSSGGGGSGGGGSGGGGSDIQLTQSPSSLSASVGDRVTITCQASQDISNYLNWYQQKPGKAPKLLIYDASNLETGVPSRFSGSGSGTDFTFTISSLQPEDIATYYCQQYDNLPLFGGGTKLEIK

SEQ ID NO: 176 - DNA, 723 bp, synthetic construct
  misc_feature 1..723: note = source = /note="Description of Artificial Sequence: Synthetic polynucleotide"
  source 1..723: mol_type = other DNA
gaggtgcaattggtgcagtcaggtggtggagtggtgcagccaggaagatcccttagactctcgtgtgcggcgtcaggctttaccttctcctcgtactccatgaactgggtcagacaggcaccgggaaagggactggaatgggtgtcctccatctcgtcctcctcctcctacatctactacgccgatagcgtgaagggccggttcaccatttcgcgcgacaacgccaagaacaccctgtacctccaaatgaattcgctgcgggccgaagataccgctgtctattactgcgcccgcgacaactggggctcgctggactattggggccagggaaccctcgtcaccgtgtcaagcggagggggtggatccggaggcggaggatccggtggagggggaagcgacattcagatgactcagagcccgtcctccctgtctgcctccgtgggggatcgcgtgaccatcacatgccaggcctcacaagacatcagcaattacctgaactggtaccagcagaagcctggaaaggcccccaagctgctgatctacgatgccagcaacctggagactggggtgccttcaaggttctccggttccggaagcggcactgacttcaccttcactatctcgagcctgcaacccgaggacattgccacctactactgccagcagtacgacaaccttccgcacatgtacacgttcggccagggcaccaagctcgaaatcaaa

SEQ ID NO: 177 - protein, 241 aa, synthetic construct
  REGION 1..241: note = source = /note="Description of Artificial Sequence: Synthetic polypeptide"
EVQLVQSGGGVVQPGRSLRLSCAASGFTFSSYSMNWVRQAPGKGLEWVSSISSSSSYIYYADSVKGRFTISRDNAKNTLYLQMNSLRAEDTAVYYCARDNWGSLDYWGQGTLVTVSSGGGGSGGGGSGGGGSDIQMTQSPSSLSASVGDRVTITCQASQDISNYLNWYQQKPGKAPKLLIYDASNLETGVPSRFSGSGSGTDFTFTISSLQPEDIATYYCQQYDNLPHMYTFGQGTKLEIK

SEQ ID NO: 178 - DNA, 1548 bp, synthetic construct
  misc_feature 1..1548: note = source = /note="Description of Artificial Sequence: Synthetic polynucleotide"
  source 1..1548: mol_type = other DNA
caggtacagcttcaacaaagcggaccgggacttgttaagcattcccaaaccctttctctcacgtgtgcaattagcggcgatagtgtatcctctaattctgcggcctggaactggatacgacaatcaccaagccggggactcgagtggttgggccgaacctactatcggtccaaatggtataatgactacgcagtatccgtgaaatctcgcattacgatcaatccagacacctccaaaaatcaattttctctgcagttgaatagcgtgactcccgaggacacggccgtttactattgcgcccaggaagttgaaccccacgatgcatttgatatttggggccagggaaccatggtgacagtgagtagtgggggtggaggatctggaggaggcggtagcggcgggggcggcagtgatatccagatgacgcagtcaccttccagcgtgtatgcgagtgtgggggacaaggtcaccataacctgtcgcgctagccaagatgtcagcgggtggctggcttggtaccagcagaaaccaggtttggctcctcagcttttgatctcaggagcgagcacgcttcagggtgaggtcccaagtcgctttagtggctctggctccgggacagacttcacgttgacgatcagcagtttgcagcctgaggatttcgcgacctactactgccagcaagcgaaatattttccgtacactttcggtcaggggaccaaattggagatcaaaggtgggggtggttcaggcggcggaggctcaggcggcggcggtagcggaggaggcggaagcgggggtggcggatcagaagtgcaactcgttcagagtggcgcggaggttaagaaacccggtgcatctgtaaaggttagctgtaaggcatcaggatacacttttaccagctattacatgcattgggtgagacaggctcccggtcaggggctcgaatggatggggttgatcaacccgagtggtggttcaacatcttacgcccagaagtttcagggccgagtaacaatgactcgggacacgtctacctcaactgtgtatatggagctttccagcctgcgctcagaggatacagcagtctattactgcgcacggtcagacagaggtataacggccactgatgcgttcgatatctggggacaagggactatggtaactgtgtcttccggaggaggaggtagtggagggggaggaagcggtggggggggctcacagtccgttttgactcagccaccaagcgtctcagtcgcaccggggcgaatggcgaaaattacttgcggcgggagcgacataggcaacaagaatgtgcattggtaccaacagaaaccaggtcaagcacctgttctcgtggtgtatgatgactacgatcgcccaagcgggatcccggagcggttctctggatcaaattctggtgatgcagccactctgacaatatcaacggtggaagtcggtgacgaggctgattacttctgccaagtatgggatggcagcggagatccctactggatgtttggaggaggtactcaactgacagttctgggc

SEQ ID NO: 179 - protein, 516 aa, synthetic construct
  REGION 1..516: note = source = /note="Description of Artificial Sequence: Synthetic polypeptide"
QVQLQQSGPGLVKHSQTLSLTCAISGDSVSSNSAAWNWIRQSPSRGLEWLGRTYYRSKWYNDYAVSVKSRITINPDTSKNQFSLQLNSVTPEDTAVYYCAQEVEPHDAFDIWGQGTMVTVSSGGGGSGGGGSGGGGSDIQMTQSPSSVYASVGDKVTITCRASQDVSGWLAWYQQKPGLAPQLLISGASTLQGEVPSRFSGSGSGTDFTLTISSLQPEDFATYYCQQAKYFPYTFGQGTKLEIKGGGGSGGGGSGGGGSGGGGSGGGGSEVQLVQSGAEVKKPGASVKVSCKASGYTFTSYYMHWVRQAPGQGLEWMGLINPSGGSTSYAQKFQGRVTMTRDTSTSTVYMELSSLRSEDTAVYYCARSDRGITATDAFDIWGQGTMVTVSSGGGGSGGGGSGGGGSQSVLTQPPSVSVAPGRMAKITCGGSDIGNKNVHWYQQKPGQAPVLVVYDDYDRPSGIPERFSGSNSGDAATLTISTVEVGDEADYFCQVWDGSGDPYWMFGGGTQLTVLG

SEQ ID NO: 180 - DNA, 732 bp, synthetic construct
  misc_feature 1..732: note = source = /note="Description of Artificial Sequence: Synthetic polynucleotide"
  source 1..732: mol_type = other DNA
caggtacagctgcagcagtcaggtccaggactggtgaagcactcgcagaccctctcactcacctgtgccatctccggggacagtgtctctagcaacagtgctgcttggaactggatcaggcagtccccatcgagaggccttgagtggctgggaaggacatactacaggtccaagtggtataatgattatgcagtatctgtgaaaagtcgaataaccatcaacccagacacatccaagaaccagttctccctgcagttgaactctgtgactcccgaggacacggctgtgtattactgtgcccaagaggtagaacctcatgatgcttttgatatctggggccaagggacaatggtcaccgtctcttcaggaggtggcgggtctggcggtggaggtagcggtggtggcggatccgacatccagatgacccagtctccatcttccgtgtatgcatctgtaggagacaaagtcaccatcacttgtcgggcgagtcaggatgttagcggctggttagcctggtatcagcagaaaccagggctagcccctcagctcctgatctctggtgcatccactttgcaaggtgaagtcccatcaaggttcagcggcagtggatctgggacagattttactctcaccatcagcagcctgcagcctgaagattttgccacttattattgtcaacaggctaaatatttcccttacacttttggccaggggaccaagctggaaatcaaa

SEQ ID NO: 181 - protein, 244 aa, synthetic construct
  REGION 1..244: note = source = /note="Description of Artificial Sequence: Synthetic polypeptide"
QVQLQQSGPGLVKHSQTLSLTCAISGDSVSSNSAAWNWIRQSPSRGLEWLGRTYYRSKWYNDYAVSVKSRITINPDTSKNQFSLQLNSVTPEDTAVYYCAQEVEPHDAFDIWGQGTMVTVSSGGGGSGGGGSGGGGSDIQMTQSPSSVYASVGDKVTITCRASQDVSGWLAWYQQKPGLAPQLLISGASTLQGEVPSRFSGSGSGTDFTLTISSLQPEDFATYYCQQAKYFPYTFGQGTKLEIK

SEQ ID NO: 182 - DNA, 732 bp, synthetic construct
  misc_feature 1..732: note = source = /note="Description of Artificial Sequence: Synthetic polynucleotide"
  source 1..732: mol_type = other DNA
caggtacagctgcagcagtcaggtccaggactggtgaagccctcgcagaccctctcactcacctgtgccatctcagggaacagtgtctctagcaacagtgctgcttggaactggatcaggcagtccccatcgagaggccttgagtggctgggaaggacatactacaggtccaagtggtataatgattatgcagtatctgtgaaaagtcgaataaccatcaacccagacacatccaagaaccagttctccctgcagctgaactctgtgactcccgaggacacggctgtgtattactgtgcccaagaggtagaacctcaagatgcttttgatatctggggccaagggacaatggtcaccgtctcttcaggaggtggcgggtctggcggtggaggtagcggtggtggcggatccgacatccagatgacccagtctccatcttccgtgtctgcatctgtaggagacaaagtcaccatcacttgtcgggcgagtcaggatgttagcggctggttagcctggtatcagcagaaaccagggctagcccctcagctcctgatctttggtgcatccactttgcaaggtgaagtcccatcaagattcagcggcggtggatctgggacagattttactctcaccatcagcagcctgcagcctgaagattttgccacttattattgtcaacaggctaaatatttcccttacacttttggccaggggaccaagctggaaatcaaa

SEQ ID NO: 183 - protein, 244 aa, synthetic construct
  REGION 1..244: note = source = /note="Description of Artificial Sequence: Synthetic polypeptide"
QVQLQQSGPGLVKPSQTLSLTCAISGNSVSSNSAAWNWIRQSPSRGLEWLGRTYYRSKWYNDYAVSVKSRITINPDTSKNQFSLQLNSVTPEDTAVYYCAQEVEPQDAFDIWGQGTMVTVSSGGGGSGGGGSGGGGSDIQMTQSPSSVSASVGDKVTITCRASQDVSGWLAWYQQKPGLAPQLLIFGASTLQGEVPSRFSGGGSGTDFTLTISSLQPEDFATYYCQQAKYFPYTFGQGTKLEIK

SEQ ID NO: 184 - protein, 18 aa, synthetic construct
  REGION 1..18: note = source = /note="Description of Artificial Sequence: Synthetic peptide"
GSTSGSGKPGSGEGSTKG

SEQ ID NO: 185 - protein, 5 aa, synthetic construct
  REGION 1..5: note = source = /note="Description of Artificial Sequence: Synthetic peptide"
GGGGS

SEQ ID NO: 186 - protein, 4 aa, synthetic construct
  REGION 1..4: note = source = /note="Description of Artificial Sequence: Synthetic peptide"
GFLG

SEQ ID NO: 187 - protein, 15 aa, synthetic construct
  REGION 1..15: note = source = /note="Description of Artificial Sequence: Synthetic peptide"
GGGGSGGGGSGGGGS

SEQ ID NO: 188 - protein, 4 aa, synthetic construct
  REGION 1..4: note = source = /note="Description of Artificial Sequence: Synthetic peptide"
RAKR

SEQ ID NO: 189 - protein, 25 aa, synthetic construct
  REGION 1..25: note = source = /note="Description of Artificial Sequence: Synthetic peptide"
GGGGSGGGGSGGGGSGGGGSGGGGS